European Patent Specification EP 3 720 965 B1, published August 12, 2026. Title: Eucalyptus promoters and genes. Applicant: SweTree Technologies AB. The sequence listing filed with the application follows.

SEQUENCE LISTING (131 sequences)

SEQ ID NO: 1 - protein, 144 aa, Arabidopsis thaliana
MDYRESTGESQSKYKGIRRRKWGKWVSEIRVPGTRDRLWLGSFSTAEGAAVAHDVAFFCLHQPDSLESLNFPHLLNPSLVSRTSPRSIQQAASNAGMAIDAGIVHSTSVNSGCGDTTTYYENGADQVEPLNISVYDYLGGHDHV

SEQ ID NO: 2 - protein, 361 aa, Populus tremula x tremuloides
MAVELMMGYSGDSFATKMQENDVREAATAGIQSVEEVIKLLKQNQLEQQQKQQYYQELSAASSSSNLGTDNIMAVTDMAVNNFKKVISLLGRTTRTGHARFRRAPVACPPQQRMQEPEPEPQQQKQQVQEPVPYVRAINSQPTEQGSAFRVYQPTPIHRLPPLPHNQQQKTLVVTKNGLSDRNEMATTINFSNSPTISAPTSFLSSVTGETDSFQRSTLSGFQFTQPSAGKPPLSSSSLKRKCNSMDDAALKCGSSSSRCHCSKKRKSRIKRVVRVPAISSKMADIPPDDYSWRKYGQKPIKGSPHPRGYYKCSSVRGCPARKHVERALDDSMMLVVTYEGEHNHSHPIDEAPGALVLESS

SEQ ID NO: 3 - protein, 568 aa, Populus tremula x tremuloides
MERDKLFVSEGANTAATIWNSCSFGMEIQANELSCGPEKLVNCFLNPNWDNSLDQSDPFESALSSIVSSPVASGANANANAVPNAGVGGDGFMIRELIGRLGNICNSGDISPQSFVNNNNNSTNTSCYSTPLNSPPKLNLSMMDSQMRGNLPIPGNSVVKHPGLAPFPADFVERAARFSCFGSNNLGGLNKQFGLNESELINRLMPRVEPGKLSRVSSNNSMKVTVSQANVQESNKSSPQDGSLNSDKKFSRQSRPSTSENGDSREESSVSEQVPGGKLSMKSQNDANSRKRKSIPRGKAKETPSSSPSASDVKVAAENDDSKAKRSKSDETNGSDKDTAKEKEEENGNQKQNKNNSKPPEPPKDYIHVRARRGQATDSHSLAERVRREKISERMKFLQDLVPGCNKVTGKAVMLDEIINYVQSLQRQVEFLSMKLSSVNPRMEFNMETLLSKDIFQSRGSMPHSLYPSDASTPAFPYGYQSQQGLALQNGMPSNAETQFSMNPLNAALRRNPSMHLPPLDGFGDPAVLQASAMWEDDLQSVVQMGYGQNHQESFQGSVPSTHMKIEL

SEQ ID NO: 4 - protein, 347 aa, Populus tremula x tremuloides
MEGVEEANRAAVESCHRVITLLSQPQDQVQYRNLMVETGEAVFRFKKVVSLLNTGLGHARVRKLKKLPTPLSQSILLDNPLSSTGHPSKTSQFLQSSSYLESQSIQELGSIAKNCLSLGTPSLELSSNGKNPLQLGQPTPAAPYQFLQQQQLHRLQLQQQQQMKQQAEIMFRKNNSGMSLNFDSSSCTPTMSSTRSFISSLSIDGNVANLEGTAFHLTGAARSSDQSSQQHKRKCSGRGEDGSMKCGSSVRCHCSKKRKHRVKRSIKVPAISNKLADIPPDDYSWRKYGQKPIKGSPHPRGYYKCSSMRGCPARKHVERCLEDPSMLIVTYEGEHNHPRIPAQSTNT

SEQ ID NO: 5 - protein, 301 aa, Populus tremula x tremuloides
MAVDLVRYSKMEDQMAIQEAASAGLESMEHLIFALSNQTRQSHQLDCGEITNFTVAKFKQVISMLNRTGHARFRRGPTSSPSSYPVPVRPVPQEPQKLNLDFVNSKSPPKAESKNDLSLGSQYSKDSLSSGTTTSSFVSSVTADGSVSNGKQGGSSLFGTQARSTGKPPLSSTHRKKCHDHALSARKISSGGSCHCSKRRKSRVKRTIRVPAVSSKLADIPADEYSWRKYGQKPIKGSPYPRGYYKCSSVRGCPAKKHVERAVDDSAMLIVTYEGEHRHSHTPLPEDVTASAAMRHVFHST

SEQ ID NO: 6 - DNA, 1084 bp, Eucalyptus grandis
cagaagcccttgcgttgactacagtctgcatttcagggcagttaagaaagagggaaaggaggagagggagagatgtagaaagatggagagtccatcagaaacagaaactgactacagccatttatttataggaagatgaggactctcgagactcgtggcgaagaacgagtcatcaagcacggggcccttcgatgcggaatttttttggaggtcctgaagatgattattcatttccccaccatgtctataaattcttcgaatttgtggcaattcaagttggggaacaaaacacggccagacccaaagaggaaaatgagtttacaacataattcaaccgacatgaaaaattagttcttgcaaatatgatgccatatagatcattcttcatagttaagctactatgtggttgttaacatgatattcgtgttgatacttataaagagaccaatcaaaatcgatccttatccttaaaaagtcaatatattttcggggaggcctattggaatactaataatcatgctgcctaattttgtcataagaatgtgagatctcgatataatcaaaggtcgtgagatcatgacagatgtagataggtaggtttcttaggagcaaagcaaaatatcggggacactgctggccagtaaagcccatgatgcagataaaggaacgaatccctccctccatctttggaagcccaacccacctcagaggccaaaagctacgttgacaggagaatgggagcagagagtcgcatcgttcaacgacgtgtggttggaccgacgaaaacttcaaaagccagggaaaaagaaagagcgcctgtgatcctttacgtaaatacgcgggggggagttctgtggtgcgtttcggttttttttcaacaccgaccctcccagttgtcttccttcctgcctaagatcggttttacttttagacgatcgattagacgatcgatcgctctctctctctctctctctctgtggcctcacgcgcatttccataggcaaccaacaacagcagcagaaagtagagttcctgcggcgatatcgcgcgatccgagtcgcgagctgaggccccgaccccgacg

SEQ ID NO: 7 - DNA, 2000 bp, Eucalyptus grandis
aaaaacacggatatgatacaaaatagagagagagagggatctattattctcacttggatgtattgtaagaaatcacaataaatctttcattcttgctagaaggggaagttgatacccccaatctaaacttgttctttttagtccatctattttggtcaattgagtagctttccctctaccaaactctgaaatgttctaaaataatttctcaaaaaaagatttttttatcaaaagaatagaccttgaatatatattaagccatgtcaaaattgcaaatcacagcaattacaattaataatcctaaaacgaaaaatcaagcttgtaacgatgattgctacaaaaaaaattatgaattgcaatttttttggggagttcactaaattatgtaaccttcaagaactgagtaaatctaaaaaaatgttccaaaactctagtagaattacgatagtaacttacacttgctaaataatctaaagaccccaaaagaaataaagttattttagtaagtgaaacgcttcggattctgatagtggaattcccagctataaaatctcaagcacatcccaaacctatagtattaaaaaaattgccaaatcttcgaacttggagaacttttttttctagaaaccgatcaaatttaattttagtaggcacatgcagacatgtgccatttcaccagtaaactaaaaaccaagaaaagattaacacggaatgacaacattctataataaatttgagaaaatcgcagaaaatgtgcaacaaaatcgagagatccaatccattcactagaaaaatgtaatatcgagcgcaattaccaaaaacatcgagttcccatacgcgcgatcacacaagacatatagcaaaaataaagaaaagagattatttccaaaaaaaataaattggatttatacacggcatctagaaagaggccgactcttggatacattaccaaagaagaaattcactcgcaagaccatccatattctgtagaagattctagaaccaggagctcgcgaaaggtagttgccaacttgctcatgtcttgtctgtccgccatcaacctttcatcggcttttgacttttcctcctgaccaaaaaaaccctaattcaattcaaaattctcctccggctgctgggtttaggtactcctaaattcggcgggcaatgccttaagggccacaagtttttcttcagtctcgcacaatttttttttttttttaacaacacataaaataatagtaatttttgcgggcgtctaatataataaagaatagatcaaaattgcttgatcaaaatttactttgcgctggcgcaatatgctcagtcttttgttcttgaattaatcacttcttcgatatgactgtcgctaaaagcgacatacgcgaaacaaattttggtacgtaagatcgatacaaattgttcacaatttcttagaatttctaatatttcttttattttttgcaaagggggaggcaaaaaattaaatgagaaggaaataatgttagacaagcggaaccattgaaaacctcctcctacccaagcccaccggctctcagatatgctccgaatattcccgcttctcgttttccccacgctcgcttcacgcgcgtggctcacaatcctaccctccgcgccggcctccctttcgaattccccgagctcggcgcgtgcccgtgatgggcacgacattcccgaaccagcgggctcccaacagagtcccgctttcaactaaatcagcggctcgaagcatcgttcttctcgctatcatctttagggatttcgtttcgcccaaggcagagagaaaaaagagagaggctgactcgtcgactcacgtgacccggcccgagcggactcaccgttctgactcgcttatttaaagcgtcttactgtccctcaccctgttgtctcaaaccactctcaactcactctcatctctacactgctttttctcgtcttctctcgctagccatttccagaaccctcgtcgcgcgtcgcttgcc

SEQ ID NO: 8 - DNA, 2000 bp, Eucalyptus grandis
aaatggatatgactacacaattattttcgagtgcatactttgtccatcaaacaaaaatgcctgaaaatttctttattaatgggctcgacaaggatgctaattgctagtgaaattcggtgatttgctgctgctgctagagacatgttagactcttgtccatgttcgtgcctcttgggcaattttgttgtctaattcgagagagatcacaaaaaaacatggaagtgtgaatctcttctcgtctacttgatatgtagccaaatcacatgaccttaagagcctatctttttcatcaattcgccaatcatacgagggaggttagatgctgattcgcgagccgtaaaaagcccattcatcgtctaactagccatgcctaggtgaatgcaaccgcacaattagctccaaaagcatatatcgttcgtcgaacggaaatgtctaagaatttatcgacactacaaaaaggatcctgattggatgtgttggactcgtgtctatgcgtgtcccctttggacaacttggttgtctaattcgagagaaaatacaagaagccatgaaagtgcagatctcttgcttttccttttagagtacttgatatatggccaaatcacatgatcctagaggccatatctttcatcgtttcgccaattatatgaaggaggttaggcactaattcacaagctgtaaaagcaccagcatgttaaacaagtaaacgaaaaacgtcatacattcaaaaatgtatacacataacgagtatcttggaatagaatactatgttattatccagtttcgatacgacggagaatcgccaagtcatgatcttctcgcgattccattgatcggaacaaggttcgcctatgctccgacagtaaatcctagggagggccacccccacatttctaaatgctaacaagaatcaagaacgagctcgagacaaaaaagatgtcctgtaataaccttagaagtcctgcattgattcgcacacgtcaggcaatttttcattttggatggtaaccaatccatcgaagcttggctcaatgcatacagaatagaaacaagtatggggggcatcgagtattaaatttggaaatgatgagagatgggagaggccatggtgcgagaacgcagttaattcttgctctgcaacacacagtgaaagagagagaaataattcgtccttttcgacccctgaaatggatcgccatttacattttacccccatctctgcaagaaaacagctcccccccagcaagaaccgagaagcgaaagcgacccattattcattacggcgtatgtaaccaagcatcccaacattcaagaaagagagagagaaacggtagtagtggggtggggaggagggggggaaatgtagagagagaaatttcaccacccagagtgtcatagcgcgcagagagagagagagtatagcgttgcaggcgttgttgcagaaccgtggcagatggtcttttaaccttttctctcgaaataattcgctccctctctctctctacccacgtctatctctctcctcattacggttctattctggggtggctctttgcctgggagcagtgagcattatatgctcatcgaaggaggagaaaaaaatgagaacggaaaagcaaaatgcagtgtaccccatctttctctgcaggcagagagagccctgtgtgtgccagagcgatgtgatggaacgagtaaaagtaagctaatctcagacttgaggctgtcataacatctcagagggagaagaagaagaagaagaaagcccaagaatttacttcttggttttttcaaaatgactatcaaagacccaacgaacatgcgcttctctttcttcagctcctccttcctatctctgcaggcatcgtgtcggtgagctcggagtgggctccgaccgggcaagctttgcttccgaagcattcgttcgtaacagagtccaaagttggctcctttgccgcgaattctggagtttgaaaagtgtgtggttggctgggggaacggcc

SEQ ID NO: 9 - DNA, 2500 bp, Eucalyptus grandis
ctcacaatccatatgcatcgcgggccattatatcttaaccgaattttagtgcgccctaaaatgaaatcatgcagatattcattcgttaaatcgcacgtcttttcgcaagagcacgtcataaataatgctctagcggatgcaaaagcgtgtgctgttaatgtcgaatcaaaagctgtaaaccacgttcgaggggctaaggcaatgtttttcgcaggaagtcgcagacaggagaagaagagatctaaaattagatactcaagctgtaaatagggtagagagagggggagggagtactgtacgtaggaagtgactggagggtgcacagtgtccctcccggtcatatctatcttaggccctgcgcctctgaaaaaaaagctacccagttttggttatcttctttgctgtcgccttgggaaaactcgttattttattattttacaaaaaaaataaagtatttttttggtacgtaccatctgtttgatatatactgtgctggatttttttttttttctgggtgtggcggtcgatactttggtggatatcgtatgatttctgttttttttttttgtttattcattttctggtccattttcttttgagttgcttttattataacagaactagtgataatgatttctctgatttcattcctgaaactacattgtaaaatcatgtagaacttattagcagacaacattaacatttaaatctggaaaaaaaaatcataacttgtttcttaaaattagaaacaagctggaaggggccatacccgcgtggattatctctccggacattatcataagagttgtatgcccgccaacattgttcattttgaactagccaattgttattgcctcatcataatgttagcaaaaatggaatcggagttatcctgaatgacaacatgatcaaacctacactttggatacacattcctgaaattctaccctctcaaacttgtcacaacataaccatttaaaggagatgctccaaaagcttaattcctcctattttaaaaaaaaagatcgtgctttacatgagattcatcttgaaaatttatgtacaataaacaaaaagaccacccaaaaaagttagaatagaagattcatccacaacgagaagtatgacaagtgtacgagtcattgattttgcttaggttgggtaagaatcgggaattgaatttcttggcaaaacaaagattctcaatgcaattcaaacaatgatcgcaaaagtctgtacgtatatatagagtttgtaaacgtcgatgatttcaatattaaacaaatctcaaatggcaaaaagatgaaagtcgctctaaattagccctatgtgagcaatatttgtggatgatcatttgccccgtgacattaatatgtggcctttttcctactagacgctcaaaatctaataaatatagacttttgaggccacatcaatagtcttcataatttactaacataacagtttttgggctaccgtgagaataataatttgatgcgagtcacaaattattacgaggtacaaattatcgaaagaatggacctcataataatctacaattatttgttatttagttttttatgatctaaaacaaactattattaaagaacatcatccaattattactcattttcttttttattggaaagagtccataatttcccaaataattataatgtaatgtttactgtgacggaaaaatcaaatgctacttattttttggttggctgagagctggaccagaaagaggcagacgctgtaccaatatatgaatgtcattaatgtaaaatagtgcgttgggattctatggagggagggaaggggaggatgtttgtagtttccattaaataaatatagtgtggaactttaatggtatcaggacgacaacgagccaaagaatgtccggaggtcgctgtaggagcacgttttctgggcttatataatgcgcgcgtccgggatttgtgtgcttgtgttaagtgtcgagttttgttggctgttgtctcattaagccaaaaggccaatccataagagaaaggaggaaaaaaaaaggagaaaagcagagagagagagagagagagagagagggagtagggggatttctcgcacattgccttacacagatccccatggcttttttatgcagggatactacccagcattcgcttggagctgagctctttttattctctttgttttagattgaagtgaagggaccatttctctctctctctccccccctatatatgagagcttgagaggctgtgggtgtgaagttgttgggttatattctcggaactagacaacaacaacagggaaaaaaaaaaaaaaaaacccaagtgtgtgtgggtgtgtgttttctctctcagatgcaagaagatttcgaaatgattacttcccttcttgccaatgattgaagcctcgagctcgtgcttgcctcgcaccacaatgagacatgcttaacgaagtaccgactttttaactgaacgaggaggaggagaag

SEQ ID NO: 10 - DNA, 2700 bp, Eucalyptus grandis
aatgcaaaatggccgaaaaagagaggagagaaaagaaaaaactcagtcccgtctctcctccgcacgatccccatccccatccgacgcgcctgatctctccccagcgagatcagaagacgctttttacaccgaaacggatcgttctgatacgggggacggggggcaggaccgagcccaagtccccggcacggcaaaagcgaatcgcgagcaaagctcggtgcgtactgcagagaattcggggcacggagcggtgtaaaatatgcaggggagaaatcgcgaaataataaccggaagcaggggagcttacgatatcaaattccctcgtacacgtcagccgccgtggggaccacctccttcttttgtcctcttgctcctgctgccctcgcatgctcctgctctctactctctctctctctctatactctccatccgtgctttgctctctcttgtcacttcctgtcaaagttgcttgctttctctctctagcttagcttggagcttacctactgtactctgcttttcccccccctctctctctctctctcgctctgaacgtttttcagtcatcgagccgagctgaactcctctctctctctctctctgggtgacccttcttcccttttctctgcgcttccgtcgaagtgaaagagggcgccgaggttgtcgtccgagatgcgtcggagaaggacctctctcctgatttcatgagaccgaccagtgagtaagctcgctccgatgactggagcttcctctgacctccctttctttctttttcgggtgctgagcttgtccagcgtcttggccgtcgtcaattttacgctttcgtgtgagctttgcttgctgtctttgtgggtgccgtgcgggactcgattcgtctggtaatcgcgaatgcaggatcgatgctgacttttgagctcccgaaggacggacccttttatctttactagcagaagaccttaaaaagtggaggttctgatttctttttcatatttttctttggctcacggtctcaaatgagtgatcggtttcggttcttggaaagatggcatttctttttcttgaaagaacagcatctggtgaatattttattgttatctcatgcctagaaaggttccttttatttttattttctttttggttctgggaaagggttccagattccattatatctcatcactcggttgcatattcaattgggctctttggtttccctcgggttgcatctgtcttgtaccctgaagaatttggcatccgccgttcttaatgcagattcgttcactttttggagcttctgtttggtctctctttctgcatgacattcttgcattggttggtccccgtggactactcacaattggaaggttcagatgcttttctgggtgcataatttctatcagatgtttgtagagatggactcctttggggggtcatcctcctacatctactttgggggctctagtatgctgtattctgtatggttttaagctttactggaattttaacatcctttcctcttgtggtgtttggttgatgagatgcggatgatagaattccgaactcatcatttagactttcatttgtcgatttaaagactgataatcagaaaggagaattcaacgcaatttcacgttcaattaacttcttgctccacttaaattgcgggtgcagttcaggggccggtttggattctctccttcaatagatttagatgggtaatctctttataatgttttggagattctggaacaagcatctaggagtcaatgcacaaattgcaacactcagcagcatcaatcatagtgttcaccatttgtttggaactgtagatttgacgatagattattgatagggggttttctggattttctgtatagttagatttgcttggaagggacttgtggatgatctagggcggaataaattggtattagatttcaatctctttttgtctgagctcaaattccttgtttcaatgcattttaactatagttatggtactagatttctttctttccttggctgaatgtatgtgaatattgcttccttcatgaaaattgttgaaccagagaaatgcatggaaacatagtgctgcttgcttcgggaattgaacaatatagctggaccagtttggtcgtgtagtgactggaagtttgcctagggtaatatcattttgcttacaaaaccttaacaaaagaatgtgggactcttcattctgttcttggtgattgttctttcagacatagatttcgcttttcagttgttatatttcttggattaggtataattagagaatttgaacatcagcctgctcatgtcctttccttgaaaatgacatatccacccagataccctatgaatttatggaggataagtgacgacctcggctgtaaatgttgttacacaactgttttctctttatgatgctagggagagattgccgcttgttttttcttgcttgcctcactaattggccattgtcttttatagtttcccctaggtctgctttcatttccttggataaacctgtctcctccttgggattcttttcttttctcagaccagttaactcagctaaaatgttgtgtattatattgtgatgtgagaaattacttctaatttgtattatcaccatcttcttctgtagccacactatgaaagatctaagtttgaggcaatgggaagtggtgtctacacctggca

SEQ ID NO: 11 - DNA, 2500 bp, Eucalyptus grandis
ataaaaaactcctaagcataggtgcttcgagcatcctaaatgcgagttctcttattgcaagagattgaaaactctcaagcatgagaaattgagattcccaaacaagattcaatgaaaactctcataaaagtaagagcaatcgaagaaagccaaccataattgtatagtttttacctaaattttaggttgaagaagagcgcaatttgagtcgatgtggaaaattgatctccaaaagatgtcttcttggatttggaatatgagataaaactggacatgccacattactaagtgcaactttagatggagtgataacggaatgagaatcaagtaaaaattagtggtgttttatgagacaaaaaaagtttaggttagaataaggacttgacataaagtttaaggtaggattgtgattagaccaaaagttgagcatttttaatgaaaaaaagaaaagattagggtagaattggaacttaactgaaatttgaggaatttttagggtattagggtcacataaaacacatgataattatatcctagaaaaagtacttcaatttttagcttgcatatcatcttttatttagccaattagtgatgtaataagtaaattatcactcgtatgccaaaaaatatcaattataatatatcatcttcacagagaaaatgtaataatgattttatttctctttaataggatcagattagtaataaactcagtcattaaatgcggcatgtatataaaattttgtagttatagtggtcctataaagatatgcaattttttttttctcatttataacgcagttgatttgataaactcgtgataatatgaagcttagattatatattagtaatgtctaatttctgttgcgtattttttcatccctcatcccacatcataaaatttcagtcttctatgttaccaacaaagggtgtaaaagaactcatcgacatcgagttaaaaggttgtttactaacgtttgcatagcaatttctttttatttttgaaagcaaacaaaaacaattattgaaaaacattgtttgggtggttacaaaaaaaaattaattatgtaaaaataaaagaaaaaaaatgacacaaatggttactcttgccaagcctcgatcttttgaccttaaacaatgcaaagcctttactactgggctactatgttaggtggtgcattttagatagaaggatatcacaagatatttgttattccatgtccttcagacagcaattcacacttactgatttgagattttttgtatgcacaacgttcttatgttctgtgaccatatttactattgtcatagtgttgtaactagattatacaattcacttggttttcttcttttatgtcgagcgtgctaatacacaagttcccttacttgattaaaagagcatacataagatcttgaagactgcggagacataaagattttaactttgagggtggttaaagagattacatggaatattttaaatttaaataactatcgatactcacatggtaggttaggaaagacaaataactttctaaataagatagtggcaagcgattttattcaacaagtatcaaatgcaaagtcctcaccgaatctggggtttataatagttgagtcatcttggtttgtccatataaggattctagtcctttacctaataggttttttcaaggtttatgtgatgtgatgggcttgcccatcttgttgaaaacatcaagatttttgctagtaagcgagacagactttacaatagtctctatataactggatcgattaagacccgactaaactaaatgatatataaacgatatatcggaaacctaaagtccaactcaacaattgacgtagatatcaacgtatgatctactccattaatctgatcgtctctagacaagtgactgggtagtatgtgaaaagagatattatccaatcgatgcactttggattaagggttttaaacttacacattgattaaaatattaagaaaatttcgtgaatttgatttataatatgatacgatagactctttattaaatactaacatgacacatttactctccactcatgatttatatcatgctattttgtaagtcaattatataaaatctagagaggccatgcctcagctcttgcctttggtctaacccagccttgaccccacaaaaaaaaaagagcaaaaatctttccgaggaaaaattgcacaaattctacattaaacttttttgcagatatgaacaaatattttttttttctcgaaaatcttccaagacaaaaggcgaggccccttcatctccttcctcacgcaatcgcttggagcgccctctctccctcactccctccctcctctctctctctctctctctctctctctctctccatcccacattcttgaaagagacacatcagaagcgcaggcatgaatctgggcaccggctcgttctctttcctgctccatctataatgagcaaagccttcgctctcttctccgcagaagggc

SEQ ID NO: 12 - DNA, 2101 bp, Eucalyptus grandis
caacctcgtggtaatgcaacgaaactagcccaaatatatgttgatagccaatttggagtaactctaattttgtttgcgttggtataagatgcaacaaggtacataaaatccaattccattgaccctgaattgtgtgaggtcttctcatgctggaaagcactgaaaattacaaattcacccccacccagagtcaatacgtagacatacatatgattttacgcaatcattgaagatcaaagtggaataaaataatatttggagggtgatagtgccactgccatggtggtgcggtgctttaaccctggagctctctacacaattctctctctctctctctttcggattatgaaaatgaaagtggggttacgtattgctggttttgaactgtttgggaaattgaagcaagctgttcccaaagaaaaaagcacgccatttattggcaaaataatattaaacatatatctggggcattcagatagagttttctcaacactttgcctattttaaatatttattattttccaattgtatattccacttccattgcctaaagacgacggcattcagttttccccccttctttattcatttatttccccccccccccccttttcccgtcattggactgcgtagaaaagaggcaatttcgagtatagggattggagggatctttctttcgtttttttctttttttttgcttgaattatttttactattttttttaattatttgcttcattccctcgcacctcttcaactttatggaagaaaaaggttgatagaggccaccgaaaagcatggacaccttatcatgaaagcgagaaaaacacgacccgatttgacgggccaacacacacccacaacacaaaataccaaaaaccactcgagcgcctcgcaaaaaattcacacgcttgttccatcatcacattcacatctccatctccaccttctattccctcttggctattctctccaccccctttttcctcggtctctgttgacgagcatgatggagaaatacagagagttttgtcatgtttttgaagaagagattggctccttctgctggcttgcaatgaagaagtggagagctgctgaatggctccatatccttccaatcttccaaaattccacttgattaggatggacaatagtctgtcaaaaagggaaaataaacttatcctgggaaaatcatcgtttcaatcttggccctttaaagttgaatatcaagattattcgcgttatttacaatttggagaagtaaactgagtcaatttgctccaactcgacatgattgtagtccataaacctttaaaggggaaaaatgacatattgcaattgttttgctggtgagaaatcatgatataaagaggataaaattgagttaggcaattgagagcataccaatccatgcaatcaaaagcactttattgaaaaaaaatcaaataaagatatgataataattcatttttctcaataatggaaaaataccttatcaatctcatgaatgagataaacatgagttaaggatctaggtggatgcatctatattaaactctttacggtaggtggtgtagaaaactatgatcccttttatgagcctaatccacacacaaatatgttttttaatcactagccaaactctacaaattaaataccataagaaaaattaaacaataagaaaggcataatttaaagtattataaatttccatgctagtgcatttaatgcaactgaaagagcacctcaaagcaaaatggcaatcataaacagtttctcctttttcctttttgctccagtgcaactttagctttttcatcgtgtgggtaatcaatctccaagtcaacctcgcctcatcatttggtcttgggttcttctgaacaacccaccatgcacctcatttcccactttcccactttcgctctctctctcgctctctctctctctttctctctctccctccctctctccctccctctttttcgttttgtttttgtttttaccttttcaacaggagtgtgtcattccctatataattgcctctctcttttagccggatcttcccctcatgggaagcagaagcatctcgtttcaggcaaagc

SEQ ID NO: 13 - DNA, 1487 bp, Populus tremula x tremuloides
tctgcttatgaatggcatggacaacaagctctgcattttcgcccatttgcaccacaaaatcgttgtgtgaagatttttgaagggcaccagcacaactttgaaaagaacttgtgaaaagatagctggtcaccagatggaagcaaggttactagtgcagatcgcatggcttatatatgaatctgtcaatgagtgtgtcttccacctactgaacctatctttggatcatgcagcagcgacaaacagatttatcttggggaaatctgattactattttgtcagtttgcttaaaacgagttgttagtaacagtgaggatattttggggcttgcttgtgagtacccaacagaaagattaaacaggttgtaatgatactatgttacattttacttaactttctcatatcctgctgacatgtttgcagttcttttttgcttgttggcgatccttttcaactgaagtatgtacgcatgaatcaattagctcaaaatgtatgttcgagcaatatgcctggtgaatgtttgttagatacgaaattaagttactgaacttgtactctttgattttgaaacaagtttccgactatgttcattgtcctagcacggtgatattggtacgtcgaattttcaactatttttgtcttgttttcaactatttctgtcttgattttcaaagtctttctgaaaataaaaaacccaaaaatatgttttcagtgtcttgttagctaaatctgttgtacaaccaagcctccccgacttgctttgtgaaaaagaaagatgggagctgggggttttgtgttgattatacaaaaccttacgagataactgatatacaagcaaaaacaccctcatattattgaatctgcgacttctacagttcatttctgaggaagaattaggtgactactttctggactagatatttccgtgttcaatgcgtcgcaacaattgatttgttggctggattatgaacatgataatcacactatagaaagacgacgattatatttcaagctatggacaatgatgttacctgctcgaagatcaatacgcttgaaggccaagatatgatcacaggtatgcaggcagtccagatggctcttgggatatgagcttcaagattgttcttgaaaagaaccaaataaattgtaaaattctctgggaatatttttttgtaaaattatcagcattgctattttttttttcaaattcatttaaatattgctattgggttagtagttcagcgcaattaacttagctggcagtctggcattagcttcaaatcatatcacaacgttaaaagtagccgttgcaactagtcagcccactagcatttgctggtgaccaatcagatcataaaaggaaaactagccgttggcaaaccctctttcaacggtcatctccctgcttcatgatatatatgcttagatatcccagtatccccttcaacaaattatctcaatcttcaaaacccagtccccagttacagcag

SEQ ID NO: 14 - DNA, 1780 bp, Populus tremula x tremuloides
gatgcaaaagctggaatgagaatgcgctaaatgcgaaaagacagagagagcgaataaatcgtgctaaaaaaggagtggggtgggtaacgggttgagctagaagaagaaaagagacaagtgcactttaggaggggggcaaccagagcgtagatgataatggttcatgtggaaacaacacacatgagcagttggtgagaacttgaatgaaccctaacagcccaaccaaacccggagccacccttaccgaaccaccacttctaaaagtacaccatgcctttttcttgagcttggttgcacagggtgccaggtggggttgtttcgttttgggtaatcatgcgatagtttaaatacctttgcgataatcatatcaatggtgacttttaagcacatgttaggtgctcggttcttatctaaacatggacatggcaacaagagttaatgctaaaataatatacgtacattacctgtgaatgaatcgtcgctgtcttctgatcatggcttcaaataatatgcagataaacaagtgtcgatttttcagtgaagattttatgaaagtgcccgttctccttaagattacctgtgaatgaatcatccctgtcaggctgatcctgggtggtttttccccatgatgttcggaagatataattatataaatgatggaatttacatgaaataagtttcagtacattcttagcagaaaagcaatatcgacgaagacaaatgatgctgtttaagacaaactggggtaatatcaatttactagtaagagatttgtctgcttttcttaattctcaagaaactttcactaaaatgcacagccatgttaaacaatttacattcaacttaaaaactaaaattgtaggatgggtagctatccaagaattacgctttttgtaaacttaattttgatgggcatgtagttaacaagtatttttcatcgatcaattcaagagccatgtctgcatcataattgtgggagtggaggaggcttttgttgctagggaaggaatgccttcttagttcatggctttggacttcggacaaggagcgcatagaatggggttaccatttttgaaaaaaattacatttgaaccctccaactattatcatgtatgtttaatctacaatcctcgtccgctagaagaagtttgggttcaaagtcatccgctcaatgtaaaccatggagagacagggactaattgaaaatagtatgttagttggagggtctgcatgtattatgtccaaacattctcttattattcctgtatcatctctgagaaattcatccgaaaataataaaacaaaatggccttttttaaaataagaagctgatgcataggataccaaaagcgccttgtccattaggagcgtcagactttgaaaataagaccaataattccctgtaagctatcatctcatcttttattttgtttgaacttgtagacgtaggctttaagcgttccatgatgttcagtcacatgttgctgtctacttgattatggaatttaattcattcggctcataagaagataaaaggattatgacgttgaagaactctggtcactccttacttacggtcacataaaaacgatgcatctttccccaccaaccatcttcaagtgaacccactttcccttgcattaggtaaggagtatgggttaagtcatcttcatgaaattagtcccctagtggagctaattctactcactccatatttactcattccactatataacgccctcaacgaccatcctcaaagcaacccaaacaccttcttctc

SEQ ID NO: 15 - DNA, 2001 bp, Eucalyptus grandis
tcaggctctgtggcgggccaacgaccaattctaggttggtcagttattgctctggacaatataataggcgcagatccatggttcatggtcagacatgtcgagcgcatccatgcacgacatgccgtccctatgtttagccaccgcaaagaacatcaataacaattcgtctcgtgactggtgaaggaactatccagctttcgtctctttgaatgcgaattgcgattgcgtgttgttaccccgtccttccttcacgtccttctagattaaactctccttggttcttcgtacgcaagttccgcatacaataataagaatcccccccaaacgaaaggagattcatgaaaaggtacgagcagcaaagtttctctctacccttttaaaaaaatcaggatgtagaagggtcacaactcatcattcctcatatagaccctttctagaaagcaagtgggtggtgtatgtacacacgtctttgagacagattcccacgtaaaagagcgagcgagcagttggccaaatcaaccggacccttcacacaattatgctctccaccaaaccccaagtcatcaccaacccccctctcctccatctctcgtccgatcccatcgaaagtgaccatcattattcatcagtgtgttctcactttctcagagcttggccatgtgggcgttaccccgttttgtcccgtaattccgcttctcggttcgatccccgcaccgccccattgcaggtaaaaatcgatgtccgtgacgacccctttttatctccttttaggtggatggttgcgatcgtggtttggtggaaaaaggggatcaaatcatgctacatgatcctgctgttgacatgtggtagtaatgtcttcccccatttgtctgaactctgatgtcaagatcgtgtaattctatgcttcaaactgaagcgatgagaccctgtgcgtctcccacttatcatgcctctccagaaggattgatccgcttgtcgccacttacctactttggttttgattttcagtttccaacttattggagcgtagcgcgtaattccccaagcaattgatgacaatttaagcaacttcctgaactttgaaaccatgcgagtactgcaagcatgtcattactgtagctcactaatcaaagatataagccaagaaaatctcggttaaaccactcgatctattgttaaggacggccatttccccgacattttaagatgtgggatatgttaaagagtactgtagttattaggacttatcgaaggtatttgtgtccaaaaatgaggaattcgtgtctacttttgagattggtagttctcttttaatgggcattgatatatccgggacataattagcatcggtttcattaacctcgatcagtaatggtgcaatgacatcgcatccctcttatgtgaggagtcccgtttccaagggctcaacagctcaccagtttaatcaatccaacattcccaaaaataatagtggtaattcaaacaaagaaaggtcaccaattcatttaccttgaatgttactttgaggctttgagtagaatttaagtactcgtacaacataacgactaggttgtaattggtgagctttactagcgtcaaattgctctcatggcaatgacgaatgggttggttcttatccgtcaagaaaattagtgacatgattaactttaaagctttgtgaacattctctggactatgatggttatcggtaaatcttttagccgatcgaaatggaccggacatcatcatacaaagggacaaaagaggctaaagaaagagatgagacctatctgttttttgggcctaggggcattactttcgaaaactgcgccatcatgatgtgattaagtagaccaaacattaccaactccggcggccccaattccttcgtaccatctttccttcgtaccatcttgttttatataagatcaaaaacccggacggcattccatcgaaactcaacgattactctctctctctctcaaaagacataaacataag

SEQ ID NO: 16 - DNA, 600 bp, Eucalyptus grandis
cgacgcaggtcagacgactgagtactgaaagcattggcctatccgtcctcattgaaccaaacaatcaactgatgggtcgggccgctccgagattaagactatttgtcagagaatttttcccaattggtggtccattttcgtcctttaccttattcaaatggaagtctcgagatattcatgtaaaatcaacgaaaaataattttctaaaatgaaaagaaacaagaggaaaatttcgtgtgacatataagcagacgggccccctgtcccctgtcgcactcaaaacacaagatgacaaactcttctcgattagcacccattctttagaggcggttttgtgtccaccgcgtctcttatccggataaaatggctcgagtgcttaatccgtctaagcccacaatttttttttcccattttctcatttaatttacaatttttttccttttttccctaattcgagtggaatttacattttagaatttagaggtcgagtggagctataaatagaggggcacggtttgcaatgtaccctcaagcaactaggagaaagtgataagccttgtgaggtgttgaagacagctttgccccaaggggagatcagtg

SEQ ID NO: 17 - DNA, 1800 bp, Eucalyptus grandis
atttgtcagaaagactaaattggtaaatcttcatagggtttaagactaaattggtcaaattgaaaagtttaaaactgaatcagtacccgtataataggcttaattattttttgataattatcttgtcatatcaatcccctaatatcttgaggcaattaaggctttactcacaagatcaaagacaactgaggctttctgaataggaaaattgttcaaaaaaccataaatttattgtgcaatggtcaatttaattctaaatatttcaattttgtaatttagttttaaaccttttgacaacatgataattcaatcataaactttttgattgtgccaatttaattataaacttttaacggattgtcaatttagtcattttggctaattttggctagatatcgttgatatgatggcctagtcaacgctaactgtcctatgtaacatagtagacgtttatgcatacattaatttttaaaaaataaatttaatttttctattttttttttatattttctttttccactttttcaaagggctaatggagttactagccattgaggaagggcagtgaagcccttgctagtggtaggtgagggccacaacctcgccattccttgttgtggtggcgatagcctaggcaagggctcatggcacccttgccagccatagtgagggcttacgagcccttgccatacctagccagccatgacaccctcgctagattcagcgagggccgtgaccttgtggtcgagaaggcttcgcaatccttgcctagggcccaacgagggtcgccgattcttggctagtgaccctttgtaaaaagaggggaaaaaagaaaaaagattactaaaaactttgaataattttttaaacattaaaaattgttcacgtcagtaacgtccaatcaaaattaattggaatgaccaaatagacaatccgttaaaggatttaggacttatttggcaaattattaaaattttaggataaaattggcataattaaatgggttaggattggattagtgaattatttaaaaatttaagattaaattgataaattttaaaaggtttagaattaaattgactgtcatataataaattaataattttttggatatcttttccctttcagatccataaagcgtggtcacaaattttgaactttttgcaatcgatgtcgatccaactcggatccgtttaaaaccgacgcaggtcagacgactgagtactgaaagcattggcctatccgtcctcattgaaccaaacaatcaactgatgggtcgggccgctccgagattaagactatttgtcagagaatttttcccaattggtggtccattttcgtcctttaccttattcaaatggaagtctcgagatattcatgtaaaatcaacgaaaaataattttctaaaatgaaaagaaacaagaggaaaatttcgtgtgacatataagcagacgggccccctgtcccctgtcgcactcaaaacacaagatgacaaactcttctcgattagcacccattctttagaggcggttttgtgtccaccgcgtctcttatccggataaaatggctcgagtgcttaatccgtctaagcccacaatttttttttcccattttctcatttaatttacaatttttttccttttttccctaattcgagtggaatttacattttagaatttagaggtcgagtggagctataaatagaggggcacggtttgcaatgtaccctcaagcaactaggagaaagtgataagccttgtgaggtgttgaagacagctttgccccaaggggagatcagtg

SEQ ID NO: 18 - DNA, 2000 bp, Eucalyptus grandis
ggtcacctcctcccgcttgggaggagacccttcatttccttgtaccacgcccttgtgtttcaaatgggaaggcgtcgcaaggatccaagcggggttaccccttgtggccaggcccctagtaggggatccatttttactgagggggatcccctccctctatcttgtctttccaagatgtcaaaaccttttaaggtcttgcttatgaccaaattgtcaccactcttatcccggtctagaggactaacttagatataacagaactgcaaacatgaattcaacgtagatattaatcaagcaagaggctgttccttacatttgaataatataagatacagctgtatttagatttgtgtgaaagaattataattaaaatatatcgagcgccggcaccacctacaatgtggcatgtgatggtcattgccgttcgcatcattcggcaaggatacttataaaaaaccagtgtttccaatcaggtgtttacacgccagtttttgtcctttatacgaaagagcatcgggcaacttgtgtgactagtgatgtaccgtaataacgatcgcgtcaacgaggacagagatcagcaaaaccaaggtgtgcgagagagagttaagcaatttcactgtattcacattcaagttcgcaaatgaaggtttgacttttatgggaatatgccgtggagatgctgaagctcacatggctcttctcggtgtcagtagactttaaatacaacccccgtccaacatttatctacgactctctctctctctctctctctctcttctctcggggtgagcagagtttaaatacaaccccatccatcccctcgttctctccatcccctctttctctccgtcccaacccaaggttggcgacattttcttacaactctccctctccatcccctctttctctccgtcccaacccaaggttggcgacattttcatacaactctctctctctctccatcccctatttctctccgtcccaacccaaggtcggcgacattttcatacaactctctctctctctctctctctctctctctctgccctccattgttgccgcgagagactgaggttagtgttcattgctcttttattgttgcactcgtttgtggtgtgtcttttgcatttgcagacgacgagaaggggcttaagaaatttggttcgtcacgcttgacagttgaaaaaagcaatcttgtatttagccatgttttggttacgtagaattttagcggactctcttgtctaaggagaatgataacccgcacactgtcatagatatagcaacgggattgaattactttgttgttaagcattattcttgtcctatattcagtagagctatgttggtacccgaaacaggaggtgacgtgacaatttcaaatggcgtctgaaattttgtagacaattacatcatctgtaaatgtctctattggtttctatggttgaagttcataatttgtttttctagaattgatgtcgttttaagaattcttatcaactttgatctctcttgaagataaaacgaagaatgatatgacgcctttatgaagtgagatacttaaaggagtaatgagtcgaccggttgccattgaagttgcatcatcaaacaataattggcataattagattaattgaccatctcgaaagaagtacaacagacagcctcacatcataaattaaaagttttgttctgtacccgccaatcgaaatacgatttatacatccaatgatgtggtgttagaatcttgacatgttcttgtgcttaaaaatctataaaatctaatgtaatatcataaactaaaaaatttgaactagggcacgtaaaaacaattttctttaccccgtatttttacttaagatcattgttggtttttattgtctctcttttccctagatatatatatacttccataatcacttaaatataatttgattatctctttcatgggcaggaaaattgttgaactagttggaaggcattgaactccagcttcgatc

SEQ ID NO: 19 - DNA, 2000 bp, Eucalyptus grandis
caccacaatgagcaaataaaaacaaaaaaaatgagagaaataagacaccaaatgaggtgaaaaaaatacttccaaattagatggagggaggaggagaaaagaaaaccaaagcccaaaaaagaaaagtaaagcaaagcaagcttttttgaagggatttttttgggagagagacggttaccaatagaaagattaggattttttgttagttagagagttcctcgttagttttgagataaataaacgaaaggaatcccaacgtgaataacaaacattcccctttttaggcagtgatagagcacgtagacagataaaatgcactctaatttttcgctactggctttgaatgtgagggataaaagtgcttaccacttgggatttatttgcacgaatctaactctcaaattccacaagttgagggagaaattgaagcggcccaacccgatggtagtcttctctctttcgtctcccttagaacggttgggctgcccatggagataaagcacagacacatcctcctcttctaggcctaactttttgatactcaccggcgatttaacagcagccatggatctctctctctcctccgacatgggagaaagcacggccgagccagctaacgaaaattccgaggccgtatctcgctaaaggctcgggctggccggaactagcactcggcctgaaagtccttgtccgatcatcctcatgcttaaaaatctttaggttttccatgtagaaccaaatgggcctagacggcccagtagataggttaggctcaaacaggaatcgctagcccaactcacccaactttgcccgatcggacttgggtaggcccaaacaagcgcgaggcatttgccggctgatcatgtttattcttcgctaatgaaaaatatttagctctcaagggaccgtcaattcaggatcgtgaagttacgtgcgctagtaaagttcatcgactagtagtagatgcggatgacaagtaaatctacacaagcgagacataggcaagtcgtttcaacctcctatcccattcataattaatgaaatgagatcttctaaaacgagtcatcgcagtctgttcttctatctactaaccatatgatgtttgctttaataggcaagtcattccctcactctgcatgactttcataaatttttcaccgtctctgtgttacatttctttatcatagagcattaagactagatactgagataggcaaactagataccttcattatgcccccgaagatgaagccgagataaagaaattaacttgacatgaatcgggatggcaaacctctaagaacagtgggggcaaggttgggcaactcgcccggcccgctctacttcattccattccattccattccattaccattccattaccattaccattaccattcccattccccatatcttcatgaaaggttggtggacaatagtggtgcttatctcgatcgtacctttccgctattttattcatgcaaatagcccttcggcgcgtccattctcatgtcacgaggaaaatgacataaggacatgattagggtcgatggtcctttgcttccgcgaattattccctctaaaaccgcatttaataatctcccggaagagcgacagggactcgcttgtctcgttgcacgtaaattactagttaagctggttgtccttatgcccataatcgcccattattacacatttaagaattcatcggcggttggtcggcgcccaaccaccgcgctccactgcatccccggtcccaatgggcggtgccggctgtgccctcctcgtccatctctagctaatatatactcgaattagcctgataaaagattaaggagatggattaaaataagaaagccactattcgaaaggatgcctttagggcgagtatatatgcgcgtcttgttcgccggacttgacgcacaagctcactgcgaagcatagctaagcgagttctctttctaaaagtggttgattctagttctttcgatcgagcaaac

SEQ ID NO: 20 - DNA, 942 bp, Cauliflower Mosaic Virus
gatctcctttgccccggagatcaccatggacgactttctctatctctacgatctaggaagaaagttcgacggagaaggtgacgataccatgttcaccaccgataatgagaagattagcctcttcaatttcagaaagaatgctgacccacagatggttagagaggcctacgcggcaggtctcatcaagacgatctacccgagtaataatctccaggagatcaaataccttcccaagaaggttaaagatgcagtcaaaagattcaggactaactgcatcaagaacacagagaaagatatatttctcaagatcagaagtactattccagtatggacgattcaaggcttgcttcataaaccaaggcaagtaatagagattggagtctctaagaaagtagttcctactgaatcaaaggccatggagtcaaaaattcagatcgaggatctaacagaactcgccgtgaagactggcgaacagttcatacagagtcttttacgactcaatgacaagaagaaaatcttcgtcaacatggtggagcacgacactctcgtctactccaagaatatcaaagatacagtctcagaagaccaaagggctattgagacttttcaacaaagggtaatatcgggaaacctcctcggattccattgcccagctatctgtcacttcatcaaaaggacagtagaaaaggaaggtggcacctacaaatgccatcattgcgataaaggaaaggctatcgttcaagatgcccctgccgacagtggtcccaaagatggacccccacccacgaggagcatcgtggaaaaagaagacgttccaaccacgtcttcaaagcaagtggattgatgtgatatctccactgacgtaagggatgacgcacaatcccactatccttcgcaagacccttcctctatataaggaagttcatttcatttggagaggac

SEQ ID NO: 21 - DNA, 435 bp, Arabidopsis thaliana
atggattacagagaatccaccggtgaaagtcagtcaaagtacaaaggaatccgtcgtcggaaatggggcaaatgggtatcagagattagagttccgggaactcgtgaccgtctctggttaggttcattctcaacagcagaaggtgccgccgtagcacacgacgttgctttcttctgtttacaccaacctgattctttagaatctctcaatttccctcatttgcttaatccttcactcgtttccagaacttctccgagatctatccagcaagctgcttctaacgccggcatggccattgacgccggaatcgtccacagtaccagcgtgaactctggatgcggagatacgacgacgtattacgagaatggagctgatcaagtggagccgttgaatatttcagtgtatgattatctgggcggccacgatcacgtttga

SEQ ID NO: 22 - DNA, 1086 bp, Populus trichocarpa
atggctgtggagcttatgatggggtattctggcgatagttttgctacaaaaatgcaagagaatgatgtgagagaagccgcaactgctgggatacaaagcgttgaggaagtcataaaactgctcaaacaaaatcaactggaacagcaacaaaaacaacaatactaccaggagttgtctgcagcctcctcaagttccaatcttggcacggataatatcatggctgttactgatatggccgtgaacaatttcaaaaaggttatttctttactgggtcgtaccacaagaactggccatgctcgatttagaagagctcctgttgcctgccctcctcaacaacgaatgcaagaaccagaaccagaaccgcaacagcaaaaacagcaagttcaagagccagtaccatatgttcgagcaattaattcgcagccaacagagcaaggctctgcttttagagtttatcaaccgaccccaattcatcgtctccctcctttgcctcacaatcagcaacaaaagacactggtggttacgaaaaatggattatcagatcggaatgaaatggctactacgatcaatttctccaattcgccaacaatatctgctcctacttctttcttgtcttctgtaacaggggaaactgatagcttccagcgttctacgctttctgggtttcagtttacccaaccttctgctggtaaaccccctttgtcctcttcttctcttaagagaaagtgtaactccatggatgatgctgctctcaagtgtggctcctcttctagtcgctgccactgctccaagaaaaggaaatcaagaattaaaagggtggttagagttcctgcaattagtagtaagatggctgatatcccacctgatgattattcctggagaaagtatggtcaaaagcccatcaaaggctctcctcatcccaggggatactacaagtgcagtagcgtgagaggatgtccggcacgcaaacacgtggagagagctctagatgactcgatgatgcttgttgtgacctatgaaggggaacacaaccactctcatccaatcgatgaagcacccggtgctcttgtccttgaatcatcttaa

SEQ ID NO: 23 - DNA, 1707 bp, Populus trichocarpa
atggaaagagataagttgtttgtgagcgagggagcgaacacagcagcaaccatttggaattcttgcagttttggaatggaaatacaagccaatgagctgagttgtggtccagagaaacttgtcaattgctttctcaatcccaattgggacaactcattggatcagagcgatccctttgagtctgctttgagctccattgtatcctcacctgttgcatccggtgccaatgcaaacgccaacgccgttcctaatgctggcgttggtggtgacggttttatgattagagaactcattggaagactaggaaacatttgcaattctggagacatttcaccacaatcttttgttaacaataataacaatagcactaacacttcttgctatagtacccctttgaattcccctccaaagctgaatctttcgatgatggattcacaaatgagaggaaatctgccaattcctgggaacagcgtagtaaagcatccaggtttagcaccatttccagctgattttgtagagagggctgcacgattttcttgctttgggagcaacaatcttggaggcctcaataaacaattcggattgaatgaatccgaattgattaataggttgatgccacgagtagaacctggtaagctctcgagagtttcgagtaacaattcaatgaaggtcactgtatcgcaagcaaatgttcaagaaagcaacaagagctcaccccaggatgggagtttgaattctgataaaaaattcagtaggcagtcaaggccttcaacatcagagaatggagattccagggaggaatcttcagtgtctgagcaagtcccaggtgggaaattgagcatgaaatcccagaatgacgccaattccaggaaaagaaaatcaattcccagaggaaaagccaaagaaactccctcttcatctccatctgcttctgatgtcaaggttgcagcagagaatgatgactcgaaggcaaaaagaagcaaatcggatgaaactaatggcagtgacaaggatacagcaaaggaaaaggaagaagaaaatggaaatcagaaacagaacaaaaataattcaaagccgccagagccaccaaaggattatatccatgtcagagccagaaggggtcaggctacagatagccacagtcttgctgaaagagttagaagagagaaaatcagtgaaagaatgaagttcctccaggatcttgttcccggatgcaataaggttactggtaaagcagtgatgcttgacgagattataaactatgtacagtcattgcagcgccaggttgagtttctgtccatgaagctgtcatctgtgaatccgagaatggagttcaacatggaaactctgttgtccaaggatattttccaatcccgtggatccatgcctcatagtctttatccatcagatgcctccacgccggcattcccttatggataccaatcccagcaagggctggccctgcaaaatggcatgccaagcaatgcagaaacccagttctccatgaacccattaaacgctgcgttgcggcgaaacccgagcatgcatctgccaccccttgatggttttggtgatcctgctgttcttcaggcctcagccatgtgggaagacgaccttcaaagtgttgtgcagatgggatatggtcagaatcatcaggagagctttcaaggctcagtgccctcaactcacatgaaaattgagctgtaa

SEQ ID NO: 24 - DNA, 1044 bp, Populus trichocarpa
atggagggggttgaagaagctaaccgggcagctgtggagagctgccatagagttataactttgctatcccaaccccaagatcaggttcaatataggaatttaatggtggaaactggagaggctgtgtttaggttcaagaaagtagtttcccttttaaatactggtttaggtcatgcaagagttcgaaaacttaagaagttaccgacccctttatcccaaagcatccttttagacaacccactgagcagtacaggccacccatccaaaacatcccagtttctccagtccagtagttacctggaaagccaatcaattcaagaattgggctcaattgctaaaaattgtctatctctgggaaccccatccctggaattgagttcaaatgggaaaaaccctcttcagcttggacaacccacgccagcagcgccctatcagttccttcagcaacagcaactgcataggctacagcttcaacagcagcagcaaatgaagcagcaagctgagataatgtttagaaaaaacaatagtgggatgagcttgaatttcgatagttctagctgcactcctacaatgtcatccaccagatcttttatatcgtccttgagtattgacggtaatgtggctaatttggaaggaactgcattccatttaacgggggcggctcgctcctcagatcagagttcacagcaacacaagaggaaatgttccggaaggggagaagatgggagtatgaaatgtggaagcagcgttagatgtcattgctcaaagaagaggaaacatagggtgaagaggtcgatcaaggttcctgctattagcaacaagcttgctgatatccctcctgatgattactcatggagaaagtatgggcaaaagccaatcaagggttctcctcatcctaggggatattacaaatgtagcagtatgagaggttgtcctgcaaggaagcatgtggagaggtgcttggaagatccgtccatgcttattgttacctatgagggtgaacataaccacccaaggattccagcacaatccacaaacacgtaa

SEQ ID NO: 25 - DNA, 906 bp, Populus trichocarpa
atggctgtggatctagttaggtattcaaagatggaagatcagatggctatacaagaagctgcatcagctgggctcgagagcatggagcacttgatctttgcactctctaaccaaactcgacaaagccaccaacttgactgcggagaaatcacaaacttcaccgttgccaagttcaagcaagtcatctccatgttgaaccggaccggtcatgcccgttttcgccgtggaccaacttcttctccttcttcctacccggttcccgtccgacctgtccctcaagaacctcaaaaactgaaccttgattttgttaacagtaagagcccccctaaagctgagtcgaaaaatgacctgtctttgggtagtcagtattcaaaggatagccttagctctggcaccactacctcatccttcgtgtcttctgttacagctgatgggagtgtctctaatgggaaacaaggtggctcttctcttttcggaactcaagctcgatctaccggaaagccacctctctcatcgacccaccgcaagaaatgccacgatcatgccctttccgccagaaagatctcctccggtggcagctgtcattgctccaaaagaaggaaatcaagggttaagaggacaataagggtaccagccgtgagttccaagcttgccgatataccagcagatgagtactcatggagaaaatatggtcaaaagccaatcaagggctcaccatacccaagagggtattacaagtgtagtagtgtgaggggatgtcccgcaaagaagcatgtggagcgtgccgtagatgactcggccatgcttattgtgacttacgagggggagcaccgtcactcacatactccgttgccggaagacgtcacggctagtgctgcaatgcgacacgtgtttcactcaacatga

SEQ ID NO: 26 - DNA, 1802 bp, Populus trichocarpa
gcgagcctgtcaaaacaaaccattgacaccaatcttggatagaataaatgtgggaagaggaaattgaaaaaaagagagaagaaattggcaccgtggactgctaataggtctgcatctgaaacaatggattgcctaccccaattagtttttgttcatcatgtactgtgttctcaaatcaagatcatacttgggaaagtacaattgacggtttggaattaacggtgcagtgttgatctcatgttcttaaaattcactcagtcatttcaaacatctaacatgatcacacctatgaactgtcaacaacgaaaagttgataaaagtaattttgcctttcaattctcttttgaaaatttgccagggaatgctattttgagccgttggcgtttgagaaggttgaaattgcctatcttcaaaagatgctggacccgttttctatttaaaaaaacggttcgaatttagagagaaacggctcttttggagtcacattaatgtatttttagaagttgggtaaaagttaatttttaaaaatattttttatttaaaaatatattaattttttaaaaaacataattaaatcacagtcataaacgcgtccgtagtgagtataatctgcagggcggcattttttataataaaggtaatttaaatcaggtcttctttccggtgacttaacactgattttactccgactccaacttaattccgtagataattatgtaaaataaataaatgacgcttaaagttaagctttgtcccctaaactccttaatttaatttaatttctccttcttcttattaactcgactgagttatcgatactacgtgcaatatattatctccactaatggatattatttatgtagaaccaaaaaataaaaaaataaacaattacttttgatattaattaaattccaatatcaggaattgagtaaatagatattatttacttttgagattatgatttttttttaaatcatcgatgaggtatttaatcaggaaagatttaaagcgaaatccgaagcaaacatctttcaactccctgaaacgattttgttgctgtatttattgttattattataactattcatgaattaaaaaaaaaaaaagtctcttgtgagtcccaaacaaaatatatgtgcccattaagttaaagaaattaaactaaaggacaaaacacacctttgaatttgagtaaatagatattattttttaaaatattttttatttaaaaatacaataaaataaattttttatattttaaaatttatttttgatattactaacaaaataataaaaaaattaatttaaaactaaaaatatttacaataacattattgaaacacaatgtgcatggtgtagaatatgtagatgtagtttaatattacgacagtatttgttttttaaagtgttttttattttaaaatatattaaaataatatatattttattattttaaaatttattttttaaaaaaaataaaaaaaatttaaaataaaaaataaaaaaatttaaattttttgaaagcaaaattaaatctcgtaggcactagaaaacgtcgtaaaatatatttttaactggaatctagcacagcagcagcaacctccctagttctcaaagtgtctttccatttgaaaaaccattaaataaatcgtttctcctcctcctcctcctccctaccatcccaacacacacacaaaaagaagaaaaaattcaaacttcaaactcaagctcagatcccatcctctctcaaacgccaccttttcctccagatccagcctcgatctaccaaatcaccgtcaccg

SEQ ID NO: 27 - DNA, 2000 bp, Populus trichocarpa
gtgttttcccatatgattttttatgatttttttcaaaattatctttgtcgatttttgtttaatattgagttggttaagaattataattataatgaagctaaatcatatgggaaaagcgttgcagattttctcacaaaacactatgaattgctacagtatttctctaaatggttttttattttattttatcggggaaagcattgtagttttcctcacaaaacattatcaattgctacagtgttttttttcataggtattttcattccaaaattatctttgttgatttttttttaatattaagttggtaaagaatttagctttataattctttttgctttttattaacagaaaatctaaatcatgtggtgaaaacactgtgtctttcctcccaaaacactgtgaattgctacagatcattttgttaagtctctaagttttttatcaccaatataactttatttccatcataaaatattaattctatcatacttttaatttttattatttatctaatactgatacataattataacattattaatacttgtgtttataaattcatggcaacatgcgcgcatgccatctcatgataataaaatacaggagttcttaaggtacattggttttgccacttgcatgacgttgggtttctgctcagaacgctggctgacctgttgccaagaatctttgtgagcatgccatggcccaaattgaatataacccgagttatatatatatatatatatatatatgggtttgaccaataaacaatttcttcgcaaatgtttaaaagaattataattatctccttttaggatctctgttatgctagtttgaaaatgtaattgtgattattttttaaaaaaattttatttaaaaatatattaaaataatatttttttttatttttttaaaattatttttgacatcagcacatcaaaatgatttgaaaacattaaaaaaatattaatttgaaataaaaaaataaaaaaatttattttttttttaaaatgcttttacaatacaaaaacaaatcaaatctaaacactaatactttcattaaattggtataagtcacggcaactttcactcaatagatctttcatgtttttatatataaaaaaatttagacactaatactaacttgattttataattaagttatttcttatattaatttcaacttaaaactgttttaattcgtcgtcaatgacttctgttaaaatcatccaacaagaattattattattattattattatttaaaataatgttgtttctgttttaaaaagtataattttggtaaaaaaaatataaaagttttaaaaaattcacataaaagttcttaattatactcttttaatttaaaagtgaaattaaaaaaaaatcatttgacaataaaatcgaaaggtgggtatttttgagatctacttttcaagtttctagcaacggaaaaccgtgaaacttgtgtggcagcaaattcaggcttgacctcgcaggctgctgatgtcagcagagagctcatgcaattagtccacgacaagagccttccgttgctgggcccaacaactttgagcccatcggacatactccgaatattcccacttccagaacattaagactcccacggtcattaaggaaagtgcgctataccttcctcttacgcctctccctcatagataaacaaccagtcaaccacccaagactgaatccaaatgccacaaaatcgcgtgaatttcctttttaaaatcagcggctaatacaacggcttttcaaaattccaatcagcggcttaaaaccaagctaattgtttctttcgttttgcccaagaaaaaaaaaaccgctcacgtgacctaaccccaccacgcacctactcttctttatatgaccctcaattagcagccactctcctcactaaaattatctctgtttaagcttatccctcaaatctcccctcttaattctaaatctctcctctgtgtcccgttactatcaacaaca

SEQ ID NO: 28 - DNA, 2000 bp, Populus trichocarpa
agttcgcgtctcattacaagcgtggggtgaagatgatcaattacatgtaactttggttcttgagagcaagattcttgctggatcaagttgtaaacttttcttcaaacttcaaattagtaatctaagagacaattccacatcaaatagtaattaacaggacatggatcaaatgttaaggaaaaaataattaaaagggttatcctaaacttttaaaggggttgatgcaaattttaaaggaaaaaaatggtcgttggtgccaaactagaggtgcatttagtgcacccttcgcggggggctccaaaatctttcaaacactatcatagaaggcgatgtttggtgattaaatgtccccacacttgtcgtccacttgttagggcatgcaaaaaaattttaaaattattttttaaaatacaaaaatacccctgagttatcttgatattaaaaaactatgatgaaaagacaaaaaaaaaacttgaaaaatagttttgttaatttcaaacccaagtataattaagtaatttaacttcaatagaaaattaaaaaagacataaaatcctctgggtttaagcccttttttttttgttccgggatatttaaataacttaactgttttttttttttaaaagactaatctaccataaaataatttgaaaatgacgttgaagaggatatgtatttttttgtttcgacagtaagaatattataccgagctagcttgtgcgtcaacagaaattcaaatttttttagaatgattttaaaaatatattcttcacattgacatgataaattaaaaataataataattactaatactaagatttagatttaaaaaaaataaaagaactttcttaattaccgaacaatttcataggaggtaatggtttacagtttacaatacggcgatgatttggtttcaaggacagtcaaaatcggaaattgccccctgacgaccccaggggaagaaaacaataattacatgaaaagatgagtggtcaccaccactaccaccaccttgtaaaaatgtatgacgacccaaaacaaaaacgccaactacaccattaacaccacaaaacccattttaggcaactaatccttgcaccaggaagagggagatgtattttcatgcctcttctaaatacaatcatggtaattacattacattaccttacccatccccctctctctgtgcattaccgtaaggttataaagacagctcaatgcaaaaacaaagagagagagggggagaaaacgacttgttattattcactagaatggcattggttacaatcagaaaatcatacaccacacccaataacccaattgagttatagaagagagagagaaagggactctgagagagttgcaggttttatagcagaggtctctgacagtaagagagtatatattttaactttatctatcaaataattctctcttactctctctctctatataggagctagctgcttgttctctttatgtttctctctttcacacttgtatctttttggtactgatgaatactcaatgagtctactgtttttcttagagagatagagagacttgtgtgttgccagaacgatgtgatggaacgatataaagccaagccaagccagactgagagctagtcatgttataactacattacataagccccaaaagcaaaaacttattcaaaaagaaaatcataaccccatttgcataaacccttctctttctctgaaaaccttgtattttcatttcattgtcggcgacttcttctcaatgagagcttaaaagggtttcttctttctccaagttttaagtgacgggaatggttattttggctgcctagagtggttaagtttggaggaggggggtttttgaacgatggttgttctcaagtgagcaaattttggattctcttttttggaagagcagtgaagtgatggcatttcgtttggaacttgtcctttttgctcttcttctctctttggttgttgattctgtgcattctgatg

SEQ ID NO: 29 - DNA, 2500 bp, Populus trichocarpa
aacatcttggatttgtttactcatcaattggccccttatgtgggaactgataaaaaaactatcaatttctaaaacttatttttgacactttcatgtcattgcatgacacacaaccaaaacactcatgggttaagatgcaagataaatctacttgttatcacgaacatttctacccagctagactttcaacaactcacaagttagatgcaacttctcacccaaaccgtattggtaacccaaggtcaaaataagaccttaccacccccaacaagtcttggtaactatgacaacacacttgatcccatcaccatttccactggccgctcccaacgcccatagcccattgcactacccataagagcctgggtagaatgacctccaagtgagtattctgcctccatactcgtcaagtccctccaggggtcgctcgcgctattgtgatacccgtgcacatagccaggactccatattgctcccctaactaccgtaggatggaccttggttaccaatctcgttgtttcatgccaaactttttaggccatactcgtcaagaccatgaatgatgaaattgatgctattgaaaaaaaacaacacttgaaaatcaatgaagcttctaaaaagacaaaaaaccattgatgtaaaatggatttttaaaacaaaattgaaggggaatgataggttgacaagtataaaacatgcttggtaactaaaggtaacaagcaagagtacgatgtcgattactaagaagtttttgttttagttgccgggtatgatacaataatattttttctttggtaactcaaaatccatggtttatgttgaatgtaaaaccaatatttttacatgaagaccttggttataagagagttcttcatcattaaactgattgttcaagaacatcgatataaaggagaaatagttagatattagttgaaatcctattccaagtagaaattcttgatagaaaaggatttgtgtctaaaatccttattgaattagttaattataaatcttattggattatgattgttagaggttgcatcctataaatataaaacttttaccagattttctgtccttctgtagtggttgaaaaatgttgcagggccatgacgcacgctatttttgaaagaaaaatatacaggagaaatagacatgttgaaaacaaagaaaattcgaggcacacgcacttggtttttatagttttgtactgggcacatgggttaaaatctttcaggcctaaccatacttggttttatttatttatttatttatttggctctaatttgtttttacattttacaataaaatcaactgtaaataaatttattcagacattctcttttctagaaaaaataacgtgtcttaatactcgaatatcccttcttaaaactcacatgtacatccaatttatttttattatatgagaaaaaaatagtattatgttccaagcttacacttgaaaaaaaacaacgaaaaggataccgtttgattacgaacgcagcatcggaaaataaaataagaatttcgactttatcctcccggaggggcctttgatcatcattcccggaatcttttaaatatatcacagacccacttccccaccttttgccgtggaagcaggtgctcactccacaccgaatgacccaaagtcgttaaaaaagcaaatggagtctctgttctttttcgcatttatattcaaatccgaaaagaaaaaggtttaattttacaccacgcgctctatatagcgtggcacgtgacaatcgcgttttgttttttttacatcatcttaagtgattttcttttccttttcaatgaaaatatttaccctttcttcatttgtaatttcaagagattatatattgcctgcactttaacatgacgtcaatgaaaccgttaatccctttcaaaataaattccgacatctgtttttttatccaaagcattctgtatgtatcttttaaatttttgaaaaaaatggttttttataccaacagctcccttttttttaatattttatttattctggtcggaactaatttctctgattgaacttcccttttaactttttttttgtaattataaattaactttattaagctaaaaaacaaatattttagaggtaattatgagtacgatagcgttgttatttttaaagtatttttacttataaattcatttaaataatactttttattttttaaaatttatttttgatattaacatatcaaaaataatttataaataaaaaaattaattttaaataaaaaaattaaaattttatcgaaactcacaccagcaccgaacgggccgaagttgctcacttcacctaatgttttatagataaacaaaaagtcacgctagcaattcacagggaacagtcaccaccaatatcatgctgccagatgaataaagcagaaagtcaaaaatggtcacatcgatgacccgcataagaagctttcaatccaaatgaacggtgggtgatggggctgtgagagca

SEQ ID NO: 30 - DNA, 2700 bp, Populus trichocarpa
aacatgcctgtaataataataatttaaaaaaattgatattacggaagttttgctattgtgcgctgaaacggtggtcttaatacaagctacaagcggactcctcgttgacttaggttttgatttatagtattaagtcaagcaatagattaattaggattattattattattagcatgggcttatgtttagagtaattgtgttaagagcaacagggaccacgtacgtgcctgatagtgtcacgcttcccaataacatgaaaccgccgtagccctcaatcactctgactgcaggtggcatatgcaacctttataaaaatcgagagaaaagttgacttgttaaagtcagagatatccatggctgtgattttgcccttcaatacccttaaataacaggcttgttgtatctgctatgttttttttttttttttaaaaaaatggattcacgtcatgtgtgtttaaacaggagagcgcatgattacaggaggaggagtgataatcaacccacaaaactagaaagcagcaaaacgacggaatgtggcgcatttgaagcgctgaaatcgagcgtacaccgttgcctctttttttttttttttgtctatatctcttcctctgtaaaccccattaatttaatgcgcctctcacttcccactctgtagacactgctacctactctctctactctcttagctctgtctttctctgcaaacactgtgctgtcagttgctgttgtggagatatataatggtggtggctgtgatggaggaggtgcaccggagtagctgaccctaggacattccttattatataaaaaaaaaaggaaaatcttgtttttgccctttgtcattcgcgtgccccctttttaagcctagtgtcagtcgtcagatctctctctttctacatgtttaagtttgttagtgtttttctcgaaaaattaattttctttgcagtctcaagtctaatctctcatttctgtctttgctctctcgtattctgttccgttcctgctcgttcctctctctctagctaggcaggcatctttctccctctcctccagggtttgttttagcccttttcaattcccattttatataaattaacagtattacattcgagatgcgtcgaaaaagaagttcggtttcaaccacttgaagaagaatgtacgtgaccatgttcctctttaatatagtttttcttttcctgctatcccttgcttcttccttccaaataagaggtttggttgctggattgtttttttctgtatgtatatatatatatatctctggatctaatgactgcagcttttgctttctcgtttattattagagtagtaaaaaaaccgaagtaacggtaaagattttcacacaaaaattgttttgtcagcccggtaataaagtatagttgcttgttgtgttttttttttttttttttgagattgtgttgtttcgatgaagagtgctattgttaatattttataacattgttgcagtagcttaaacgattatctttttttcagatgcctctgatttgtggctaatatataagttgttttcttagatttttcagaaatattgatatttgaaacacaaccattagatttggaggacgttgatagaaatttggtttttttttttcttaagctgcaggtctatgtatagttttgtattttccgttgtggcttgaaaaaataaataaataaaagttatgatatcaagaacaatggatcatacggttaacaagtttcgctttttgcaccttatttgttggtaattgattatgggatgctcacgaccattattagtattttgtgcagcaaacaaatccacaaagatgcatttgtcataatatgcccttttttttatgctgaagtttatgattgcttgaggaattctggtagatataagtgaagtttcactgaattcttttgggtttacaaatcattgctatacacgtttttgggagttacatatgatatggtaggggaaacaaggatttgatgagattgtgtatttggatgaatttctcaagtattagaccacaccacatgctgtttcgttgctgatgcctatggcccaataccaatggtgaattattggtgctgagcatttctaaaagtggagctacttggtgaattattgcttgacatcatttgctgtttgggctggaattctatcatcataacccagtaaattgctcaatctgttatcggttgtaattgcttacttgtgcctgacttatgacatgataagaaattcatcttgcttattccgtgattgtttgttgccaatgatagaagcaatgtgtttgttgtgtgttttaggattattttattttttattaattctatgtctttttatggatactgctactaaacttgttcaggtgtgtatatatatcatacacatgaaggcgagcttttcattactccgtttgtacattcttgatgcaggttatggcccttgttcgcgggtccaaggttgataattttgttgggatccttatgttaatttctgcagtgcggacctacttatttagatgttatatattcatcttgggctaaaccctgcttttcttttgatgtggaatagtagagtaattatttacatgttttgccaaggtgaaggagattgatgccatgttctgctatgtttcagatacattatgaagagttcaaggcaatggaaagtggtgtctacacctagaa

SEQ ID NO: 31 - DNA, 2500 bp, Populus trichocarpa
ctctataattgtagaaatcttagattattgaacctgaataccatcaacaaacacaataaaccaagaaaaattacaatactagtaaagaacttaaactttttgcgtttgacatataattgttctttccttaaagtgccaaaaatagcccttaaatcctcagaatataactataaatcaggatgtcgttaaaataaaccacaacaaatttgcctataaatggtctcaatttctaactcataaacctcatgaaagtgctgagagtattgcacatatcatatagcataaccatccattcatataaaccatattgtgttttaaaggctatcttttactcatcctcgacttgattttgatataatggtggtcattcttgagatcaatcttggaaaacacctttgaacctgccagttagtcaaacatgtcatctagttatgatattgagtactagtattttattgtgacctgttaatggctcaaccccatactcatatacgtcatgaaccattatttttagggaataagagagctaaaactttacatgagctcatactttcttaaatatactccttttttagcaacttcaccatttgtttcaacaaattttcttcttttttaaggctagtctataagttagtatattcaatagactaaaacttagtactagatcaatatggtgttgtatctttctcatgaaaggtaatttctagggcaactcttttgacatcaaatctagaaattttgttagcataccatgcatttaattgtaaatgtcattaacattgtcctctttcccaactgcatttcaacttgtagtatcaacttctctcaacctcgttcaaccaatttatgaattcctctatttgtaaaattcctactaactcaaggattttgatatgaaatccaaaatccttcaatatgttctctttttgatcaagaggttgtctcctctgattctgcctttggtctttagtgttggctagggacccatggttgttcttctagtcttggtctcccaggtccctcttctctaacctgccgttcaactctgcaatctgcctccgtatgtcctcaatgatgaccttctaaatgtttgtctctaatgaggtaacctcctaatcccctccttgatcatgccacacttcgtaacctcatcctttcatggttattaatagcaaacaacaaataaataagtatccacaagattgtaacacaacaaacaatgaacctgagatcattaggctctgataccaattaatactagcaaaatcacaatagacaacaacaagcataaaaaaaatagaatttttgatgagtgaaaaggctgcagatataagccttaaattcataatttattattctaaaataaagtctaataatatctacctcctaagaggttatataagatatttaaatatgtcagaaaaccctatctctattaggatacaaatcaaaatttgaaaaagaaaaattaacataaaatccaaaataaaataataaatccaaaaaaatcaagaaaaaattacaaaattggcccaaataacatcttctagatctaattttgggagatccattagtttgatgaacgacaaatcatttttttatatgaacatggccgttagaattatctaatcaaatttaaaatcgattcaacgatcagatcttctgttatgatttgttttagttattattttggtctgacataaccaagctttttttttgacctagacttttctcaattatccataaaaacatttattagatcatccatatagtttgtttgggacaaaacctcattcaaatgctcaaaatttcagcttttacaatctcgactacattgtctcattacatatatgtttagatgaagttttattatatatatattttttttttgcatgtacatcattttcaatttaagaaactcctttgtcattgtgattacaatttaattttatatacaaattatgatgatttatttcttttaatttcaaagttttttgttttatatttaaatttttaaatatagtcgaatcgccgatgacaatacataataagtgtactttctcctctcatcttgcaaaaactagccacatcggatataggccacccaatctgataatggggttgggtaagggttaggttttccattgattttaatatttattgaccttttaattatataaacatttgttaaaaaaaatgaagaaatttagttgtactaataataacgaaaatacaaaaataatattggtagcgaagtaatagaggaaaggtaataagaaattaataacgaaaaaaaaaaaaaggacaggcgtgaaagggttctcagataaaatccttcccttccctactgtatttgtctctctctattactccatctctcggtagggcctaaaaagagagaaagatatgcaatatatacaaagagaagcttgagagattttaccttccttttcattttcatggttttctataatgagaagaggattgaatctcttcttct

SEQ ID NO: 32 - DNA, 2101 bp, Populus trichocarpa
gcggtcgggagagagggagaaagggtcatgtcagccaggcagccaaatctttatacttgaattcttgtttaccggaaatattgtatgtaatgaattttatccacaaggaaattttttttatgggaattatagccttttagatgcatgaaagttaccctagagtcatgccctaaagaatttttgttacatcgatcacatgcactgagaatgttttccactgctatcatgtgggaaatgactttcagtccctcactctatggtctatgcctatgaatgtctcttgtctaactgcttccagaaaagaggtggttttttgaggaaaaaatacgtcctccgagctgcatattccaccttaatatcctcacaaaatcagtgcaaattcacaatagatcatgactcatcaccacacgactaggtcaagataagaagttgtggggatgtttttccaaaccaatacaaatgtgtttgaaagttttgaagaaatagcatcgaggataaaaggattttgaaaaatagcacaataaacaaaaaaactacaataaaaatgaggtatttaaacaaaacgtagttgagaattgtgatatttaaatgaagatacctttatactaaatgctatttaaaaaagaaaaaaaaaccagtagtttctgtgatttaaaaaaaaatcgcatgcaagaatcacagattttctagctgtgcttcttttcaaaaaaacgtttttatacgtactagctagtcaaatttttaaaaaagctctgctaatttcttataataaaattgaaggtttcaccacacaattattgaaaacaaatttagtgcataaacgacatatttgaagtcaattttttagcaattactaccagaatcttgtccattagaggaaaaacatgctcagctcagtcgaggtttcctttcaacagtactcaataaactctggtctgtccacactgcccccctaagaaaatcacagctacgaagggcaatcatataagaaaaatttaccatttggcaaatgtttgcgataatgattcatgacaatgataattctgattaatcaagcacatctgctgtttatgtctgatcacaatttctttgcccacccaatcacacgtgctatatggaatcacttattgacagttcaaagtgcatgatgcccgtgattgcagtcagtcgaaatccttctgcaatcctccagtttcactgagaaactaatcataatgcacatgaccagaactattattctctccaaatgttattatacgtgcttatcatcaactaatcagtggtctgtcagataatacataaatatttaggctatggcttgtttacgcagttcatatctccgagtgttatttatagtctcgcttcgcttgaaaaattattaaaaaaaaattatctttttcaattcatacggagttgaaaatgccgcagtaccaaacaaacaaacacggaacaggacatgagaaggggggataaatgggtggggtttggtggtttttatagtttatactatgtgggaaattggagctacagatcccagagaagaggaattggatttggatatggcatgcactactgaaataaatatatattagggttatttatgttttaatttttcaacgttctctaccagttaaaagacgacggcattcaccaatatttatccgtatcttgaaaagcaaagaagttccattttcaagtttagggattggaggaatctttttcatcctctccctccctctctccctctctttactttatactgtaatgaaaaagcttgagagagaaccagagaggccaccgaaaagcatggacaccttatcatgaaagcaagaaaaaaacgaaccgatttgacgggccaacccacacgcataaacacacagttactcactcactaacacacccacacgctcgatcgatcacacatttgtgtcactcactgtgtgttaatttttgggtgtctttccttttgttaaaaatatggaaatcataagtcaacctcccctcatgatttggtcttggtttcttctaagcaccacctcatatcccactttctttagcaccctctatataattaccactccctttcattcagtccttcacc

SEQ ID NO: 33 - DNA, 1801 bp, Eucalyptus grandis
tggtgcgccgggaccatctaatattttctcgggactgaaacggtagaattgtcaactttttctcaacctttatgcgactgtgattggttagccatttaaaaaggataatagaatttaaaagaaaaaagttcaaaagagaaaagagaaaaattggagatttttaaaagaaaaattgcagttgcgatttgttattctctggaaaaaaaatataatttaaacgaaaaaagagtaaaaaagaaaaaaaagaaaaattggggatttttactaatggacggtggattgggagctgattatggaatctacgcgaacgatttattatattaaatattcagaaattcgcatgcgtgggacatctaggccaagtgatttcaagcgcgagatccacacgtgtcagctctagagtaatactgcggtaaaaaagtcaacctttgaaccatcgagctttcgagaggagaaaaaaattattgagcttaatggcgtcgagcaccggacgtgaaccagaagttaaatttcgtcgtataatgatttataacgagggttaatatctttaaaaatcttaaattattattacatgataccttaattccaaactaattttcacctcataaatgatcctaaatcagtgcttccatggcacttttatctcaaattgattctcatatcacaaaaatttccaaaccggtatctaatgtcacattcacttgtattaataattttcatctcactgaaaatatcaaactaagaccctaaccaagtctgccttccagtagtattgtgcacaatatcccattagaaatgacaactataagatagatcgacgtataaaatgctaacgaatagcaaattcgggtcgaggagtgctagttggggaatttttgttgaatgagaagtagttcattaacaaaaaattggatgaaaattgaattgagttaaaggtttaatacctcaaaaaatctaaaactataccaattgtaacacaaatagcgaaaaacttttttcttgtcactaaaaaacctcaaacttacccattgtaacacaatttccaagctttttttgagttataaaaaacccaaaacccatatcaatatgataaatatatcttaaatagaactaaaatagagaatatatatgtcacacatatataggtttaaatttttttgtgataaaaaaatattttatttatgtcatggtaaacttaatttggagctttttgttatatttaccttaagataaatatgcttaattgatatcaacttgtaattttcagtagtaattaattgttataataacatgggaggttagaaagtcgatgacaagacgatagcgagagggtgaggtgaacaggctgaataatgatggtcattagggttgagataattattatagattatgatgattgggcaaaagaaaaacaaaaaagaaaaagacaaaaagacaaaggaggacaaactagccgttccagtcccgcagcgaatccaattaaaattaaagcaaaagcggacggtgggaccgccgcgagcacgacgggtgtgctggacctcttttttattattataaattgtcattattatatttttgtttttccaacggtcagatttttgctccacagtgccgaatgtgaccgtttgagcatgtcattcggccggatataagaaccatctctccgtctttccatcccaattcactcctcaaactcctcctctcttctcttcttcagcatcatcatctagccagcttcgaaagagctttccttgaattactcagatttttgccaagcgaaatcaagggaagaaaaagaaat

SEQ ID NO: 34 - DNA, 600 bp, Populus trichocarpa
ttttaatgcacttgatgacatattttcaagctattaaaatttaaaaaataaccgctatcttcctttccggcaccgtccgagcccacaacactacaattcgttgcctgccacttcatccaaatgtgatgtgaacttaaatgagtagagcccatatgtatgagcttaactaagatcatctggtcaatagccgagcaccacaagggtggtcaggtgcatcttaaaggggcttgaaagagagagtagaagccgaagctcgactcggcgataacctcaaatgaactagtatcacacatccatgtcctcccgaggatgagataaggtcctggagcttcttccacgtggcaaatccattgtggtgcctaacgataaggctagcattccaagaatttccaccctcatgtggatagaatggtgtcatgtcatcacttatcatatccaacggtcacattttgctcattatcaaccacgatagcttgtgtccataggatatgagatagacaagttgaggcattatatatacggtgtggcaggagtacttcaatcttacaatactagcaaaaccacatatagagggtgtaatagctaagtagcctgtaagag

SEQ ID NO: 35 - DNA, 1800 bp, Populus trichocarpa
taaaacttgatctctaataaatttaatattaaaagataaattaaaaaaaaaactaaattaaaaaaatatatcaagttatcaaattaataacttgaattataagattacatgattctatccaaaacaaattaaaataaaatataatgcaaaacataactcttgctttatccattaccatgacatcatatgtgacaattctccattatctagtaaatctaataatgaattataaatttttaaaaaactaaattataaaaaataaaaaaaattaataaattcaatatttcaacaaaccttgttttatgaggatatatatatatatttgttaaatcaaacatgtacaaattcataaaacaaaggacataatcaataagagctagcagggaagaaacggagaggagttgtggtggtagcattgagtgagaaaaaaataataatggtctgttatggtatgagcccacatgctctttacagatggccatgagaagcttctattggccaattgaaagtttgaaacatctagaccatttcctttgttttcccctgaatatgtagcattgggtttcataaatacactggaccggaccatcaaagccttgtctggtggactaaattgcatcatttaaacatttaaagggcctgatgcataattttgactgtgacacttaacaggcctacacggtccaaactcgagggacctgaacatctatggggccttcagctagtttagggtttcattttcgataatggaagctccatcccttttctaataattcaagtttaaagtttctcctaaaagctccactgtgcaattgaagattgagtgtaaaagacgctccaagagtcattttcgatcacattgacatgccaatcgaaagtgttcttttttattattattattaatgtgaatgtctggactaatttgcgcgtattttgattaattctacgagccatgaagttaacgaccatgtaaacttccaatgaccctgaactttatgagattcgaattggtaacttctagaaaacaaacttaaaacctgatcagataagctacacctctcgagattgtgttcttcttctaagcagtgggtgccaaaaaaatcaacccatgcatgcaatctggtatcaatttcttagaaaaaattgattttgaaaaaagaaggttacacataatttaggggcatggttcactttcattctttttaatgcacttgatgacatattttcaagctattaaaatttaaaaaataaccgctatcttcctttccggcaccgtccgagcccacaacactacaattcgttgcctgccacttcatccaaatgtgatgtgaacttaaatgagtagagcccatatgtatgagcttaactaagatcatctggtcaatagccgagcaccacaagggtggtcaggtgcatcttaaaggggcttgaaagagagagtagaagccgaagctcgactcggcgataacctcaaatgaactagtatcacacatccatgtcctcccgaggatgagataaggtcctggagcttcttccacgtggcaaatccattgtggtgcctaacgataaggctagcattccaagaatttccaccctcatgtggatagaatggtgtcatgtcatcacttatcatatccaacggtcacattttgctcattatcaaccacgatagcttgtgtccataggatatgagatagacaagttgaggcattatatatacggtgtggcaggagtacttcaatcttacaatactagcaaaaccacatatagagggtgtaatagctaagtagcctgtaagag

SEQ ID NO: 36 - DNA, 2000 bp, Populus trichocarpa
gtcaaacaaactaaaagcaaggtgacccatgttattttaaaattgaccacaaaaatctcatataaagcgaattaaaaaaataatagaatagtaaagtataaaaaaaggctttaaaaaagcaaaaaaacacggaaacctgtgtccatgtcaacttcgttaatcaaagtcaatctcttaaatctataaatcattaaattctacacctggactaaactaagaaacctaacccgatcaccctgcgacccaagatatgagatgaggattacccgacaaaaaagaaagttgaacaaatcacaaagctcatagcctaataattcaatgtcaaatgataaaaataaaaaaaattctgaaaaggattttaaaaaataccaaactcaaactaagtaaatcgttgaaactagtgaactaggtcataaaaatgagacaaccctgtaaaagaaagaaataatcaaaaagcaaaatcctcaattataaaaaattaaaaaaataaacaataaggaccaaatatgatattaaaaataattgaaaaaaactaattagggacaaaactgaaaacaaaataaatgaagaaaatgatagaaaaggagtaatgaaaaaaataagtaccaaaattttaaaaaaatgaattaaaattttaaaggacaaaatcaaaaaaataaaataaatgcaaaggatgaaaaaacaacaattgaaagaataaggaccagattgtaaataaaaaaattaaattaaatgcagagagggattaaattgaaaaaaataaatttctaaaagcattaaaatcaaagcaaatagaaatcaaaagaatgaggttcgaatccaaaacaaattcaaaatgaaggacaactaaatttttcaaggcttggcatgaaaaccaagaccgagagagaaacaaagggcaagagaaaaaaccccatcgccaccaaaccgctgcccgtcgtggagcacgcgccactccagcggctgcgccacatccttgcatattgattgagatggcgatctgttttattggccatcgtccttggccacacgcaccttcagaatagcatgaaggattctgacacgttgatgcgtgtgtggcatacgttatcatattttactgatttattaatattttaataagaaaaattacaaaaaagagcccaatgacataccattattacaaagaaatcatgatgcaaagattgaaacaccctcggaagctatgctttaaatatggaaagtcaaaggtcaataacgtaatttttctgtacaaaaataatagtcaaaggtcaataacgtaatttttttgtataaaaataatacaaagacaaataaatcccttattgcaaggtcattttgtttgagcacccaagggtataatcattttactgtgtaaattaaaaaaaaatcttagtaggagaccatttttatcagatttcaagggtatataaaaatatattttcactgtgcattataatttagaatgaaatctttgcccctgatgaattctgaaataccatttgaatctcatggacaatattattttaccccagtatcatagataaaaaattataattacactgcttgaatttacggtgattctccttatatgctacagtgttttctttcgcaaggagcccttaacccgagtccctagtcgaactaaaagattatcgccatggccatttaatctacgcttttttttttttttcttatgaacttacaattaatttatttttcaatttttttttggtataaaagaactatttctcgtaaagaatctcgttaaattcgttgggaaccgaagaggttttattttctaaaatctcggagaatccagagacagaaggagtagatctttggtggacattgaactccgactcttcccgggacacataaaccgtatcctgctaggactattacgcttgattccccattctataaatatatcaaactcggtttagaaaaggagctctcagcaaaaagtttcagatcaggaaggcaggggaacctcaacc

SEQ ID NO: 37 - DNA, 2000 bp, Populus trichocarpa
aaaaaaattaattttttttaaaatatttttaaaacaaaaaaataaccagttttaaataaagatgagatggcaagcttttccactagtcacccaaatacggcttcaaagttcaaataggtatacatttttttcctttttttcggtgggactttaaataccgaccacaatttattttaatgttgtcctgaaaccttatgtagattaatatacgtttaatgaaacagatccacatcatgatcaataaataattgccgactcactcaacatagaaaactccacatctctcttcttgatactgttctcatcattgaaggattcgtgtcttgaaaaacagtccattatcatcattaatttgaatgtttttcgtaaattttatctgttagacgtctgctatatatatataatttatatatatatatatatatatatatatatatataattttcttttaaaattacaattaattgttagagacttagaggacgtaaatacctagtgtttaattatcaagtgcaaatgtaaatttgtaatatatcactttcgtgtttccattttcgattatagtaattaaatcagaaattgaagcagaaagaaatatggtttgatcaaattaattagcttctcaagactgagaattaatttcacaagaaccttatcgatactctaaaggaagattgtaactcattgacttggatgctattgccagctcttgaaatggacgtccccgtcacaatcatgacgggattatcgactatatatatatatatatatacctaattctaattctctaaacaaagctaattattatctatacatttgaagtggaaaacacgatttatataaaaacaaaaaccacctcaagtttattttatttttttcaactcctttttattatttgggacctttcaactcctttttattatttgggtccctttttcattcaattttatttattgtatcgttttgcttttcatttaacaattgtagtgcagtttcataaaattgatgctccataaaccatgaaataatgtttgaaattacaaatatgtaaaacaatgtaaggtgaaagaaatattaaaaaaataataatggaaaaacaatatagaaaaaagacaatccactaagagttgcaataattacccataatgtattatttttatttttttgtcgcttgattcttttatttttaatttaatcatttcatattaaatttatttgtgattgaatttgatgttttgttttgattgactctaacatagggctctcacaatattaaaaataaattttgatgttgtgttgaattaaaaattttgagatccaatttgaaattaaaacaaatattcaatttgttttttttaaataacatttttattttagcttcccaactcaatttttaattgtaattaatagatttattattatttattaacatatataattttttatttattctattaaatatatgcatgtataaacttttcagttcgcaataaaaatatttaacattgtggaaaatcaaactagcttgattcatgagaaatgccccccctttttttatcgtttgatacgaggaaaatgacataggagggcattaatcatttccaagttgtagcttactttggtgcaaatgaattattctatcaaaacatgcttatcctcacaagttataagatgttggctttgtgtctttgtttccgtaactaacatttagcagggtttattttagttgtcttatgctcataattaatgtataattattactaatcaaataaaaggcggttggtcggcttccaatcatatagtgctcctccattcatatgggtcccatggtcggtgccggctatgatgcttattgcaaaattagcatcgcagagcgccagtggtgctataatataaaccacgcccatgaaatcaatgcagcccatagaaacacatacaagaacttgagctagctagcagtaattaagcttaattggcccaggactactgatcaagcaaga

SEQ ID NO: 38 - DNA, 2500 bp, Populus trichocarpa
ttttttgactcgataaataataaatataaactcgatttaatttgatgagtactcactatcatctttagccacggtgaatccagcttgccacttgtttgatttaaataaaacagtaacaagattcgttgctccacgtgcaaatgctaaatcgaaccagctagatttcatcgaccttgtaaatccaatgcacgtggctcacccatggcgggaaaacacaactccggtggtgaataataatagcacgggaagaaaagcagtggaaaaaaatggtcactgaagcctatatttcttctttttttcttgctcttcgagcaactaggatattaatttttattaatctttgaaaaaataataataataaatatcttataaagcttaaagaatcgtgaatattgttaaaaaaaatcactataattgatgtaatgcttatctaacccttgaaaaaataacaatgatgttgatactcttattatcatagttttaaaactcggtctagcaggttaatcctgaatccgacagatccggggttaaaatcgagccgagttgagaaaaaaatagagaaagaaaaaacccggtgtgacccggtcaaaaatccggatacaacctgttgacttttgtttttttatttaactaaaaaattgacccggacgacctggtcaaaaccagaacccgaaccttgaaccgggccggattttaaaaaatatggttcttgtattagttttctcctcctttaatatttttaatttcttttagtgataaagattcagacaacataggatgacgattatccttttatatatatatatatatatatatctgacatttttacatgagaaaaataacttaaagtatagggacttaaaaatgccattaaactaacggaaaacagcaggagagtggatcgagagacaagttttattacagtgctcttttcaatcgaattcgtttagaatttcaagctgtgtatcataaaaatttaagattttattttatttaagattaattttttatattattaaatcgttttaatatattaatataaaaatacattattaaaaactaaaaatatattattttaatatatttttaaacaaaaaaacattttaaaaaccacctttacaaccttaccaaaaactcataaaagcaacctcggcgcgtgcacagtctaccgttacagattctgacagtctccgttcgaatacggtcaacgcttttgacgctttccagaaccacacttacatctgcgcgtgtcaagcacatacacggatctgtgagaacttgtaaagcacgcgttttcttgaaaggcgacgttagaaatcggttttggtatggtcatcatatgcttactcgcaggttatctcttttagtttttagatttttatttttatttttctcgggaaatatcggtgacgcccgcccttcgagtggcggttagtttttcctatccccttgatttataatttgtaacttttattatcattgttggatttatcttattataaataaaaaaaataatgatattgataatattataattcaagtttcagtatatttattatattttttatttctctacttttttgtatatttaatatttttaaagtatattattattctaaatatcaacaaattataaaaatcatgttttttaattatgatatatataaactgtgttattttatcaatacttttaaaatatatgttaaaaataaaaaataaccctctttccattaactatccatacgaaagggaaaaaaaaatctatcaaggatttaggatttaattctaaaaacaagttatgaataattatttttttcattttacaacctttgttgtttaattattctttcaaaatatattaacaattataaaaaaaaactaaaaaagaagtgatttttagtgtatttctccacacaaaatattatttattataataatgtttttatttttttatcatttgatatttttttatttagtattttttttaatttcatcatttaatattaaatttattttttattgagttattttattttcatgacatgaattatgagttttgcatattatattaactaactcagtttttttaattaatttttatttttttattttattttttaatattaatttgattaataaaaaatctaaataataataaatttttacttgtataatactatttgctaaaatattatgtttttttcaaataaataaatttaacgaaaatacaagaaaataatagcaaggtaataacggaaagcgcagtgagaaaaagaaaagaaaagaaaagggcaaaaaaagacaggcgtgaagagttctcagataaaaccccttcactcgcttactctatttgtctctctccattacagtagggcctcatagagagagaaagatatgcaatatatgcaaagagaagcttgagagatttttatctccctttttcatttttgatggtgttctataatgagaagaggattaaatctcttcttctctgaagaag

SEQ ID NO: 39 - DNA, 2101 bp, Populus trichocarpa
atgctcaacctttttaattttttaaaaaaaatctctttcactacttttcttgttttatataattcaagaattggttgctatacgaagatccaagttgttgatgataaaaagaaaggaaagaaaagaaatccaagttgtcggttctttaaattgtgcaaggaaagcaagagcagataagcttaaatgttaagaggaaagccaaaggtctgcatgtcgtctgtgtataaacccgtcaagagtttagaatgagttgttcagcaacccaaatccatatgtcaggccaaaaacattgttagctgaaggatcttattgtactacattgcaaatatgtggtcgagagagagaggttcacatcaactcggtcgccaaatctttatcttagaagcctttgtttaccggaaaaaacaaaatatagtgaattttgtccataggtaaaaatcatatggataatatagccagctagatgcatgaaagttacactagagtcatagcctgaagaatttttgttacattagttaatcaaatgtactcgtaatgtttttaacagcttattaatttaacatgttttttaaaatcctttttaaaatttgttttatataaaaagaatattaaattaatatttttcactgttatcacgtggaaaatggctttatccctcattttaaacatgttttttaatatgctttttaaattagttttttattaaaaaaatattaaattgattttttaagatgttttttgatttgttaatataaaaaatatattttaatacatttttatttcacattaatatcccccacaaaatctgtgaaaattaataatggacgactccccaaccaagtcaagacacgaggtctctccacacaattactggaaacaaatttaatgcgtttaggacatgtatttgaagtgcaatcgcttccaagaacgtaaccttgtccataagaggaaaaacatgctcagctcagtcgagattcctataaatagtcaatgaactctggtctgtccacattggcacccttaattactaaaccactagagaaagttacagccacacaagggcaatcatatatatataataattaagaacataaatttaccatttggcaaatgtttttttatagtgattgatgataatccagattaatcaagcacgtctgctgttaatgtctcccaattcatttaccaaatcacacgtgctacgcagaatcacttattgacagtccaaagtgcatgatggccgtgattgcagtcagtgagatccttctgcgatgctctagtttcactcaacaactaattataacgcacagaatcagaattattattcaccccaatgttataatacgtacttatcatcaactaatcagtggtttatgagataatacattatatagttagtgtaataagacacgataaggtactgccatagaattaagaaaaaggggaataagaggtggggttcggaggtttttataatttagagaggttattctacgtgggaaactggagctagctacagctctcgaagaagaggagttggatttggatatggtatgctgctactacattcaaatagatatattgtgattatatatgctttgttttttcaacattctctaccacttcgagacgacggcattcactcgctggcttctctcagtcaccaatatttttccgtatcctgaaaagcaaagaagttccattttcaagttttgggattggaggaatctttttcattctctccctctctactttatactataataacaaaaaaaaaagcttgagagagaaccgaagaggccaccgaaaaacatgggacaccttatcatgaaagcaagaaaaaaaacgacccgattagacgggccaacccacacgcatatacacacagttactcacacacccacacgctcgatcgatcacacatggtctctctccctctgtgttaaatttgtgtgtgcctcgttctttcttttaaaaatggaaatcataagtcaacctcccctaatgatttggtcttgggttcttctaagcaccacctcatatcccactttctttagcatcctctatataattaccactccctatcattcagtccttcgcc

SEQ ID NO: 40 - DNA, 600 bp, Populus trichocarpa
aaatctagtgaatccagccaaacctaattggttaactctaaatttttttattttaaatatgaaacaatattatttttaaaaaatcttattgacccaaattgacattaactttttttttatatatatatatatatgaagtaaactaagctctaaaatcactgtgtcaatggcaagctgccaagaaccacagaagtggtcataaatatcttaaattaagggagctgaaagagagagtggaattaatcgaaaggctgcctcagcaagaaccataaagccataaattaactagcatcacacatccatgacgtcctccatgggatgagataaggtcatcgagcttcttccacgtggaaacctctttgtggtgctaacgatgaggctagcatcaaaagaattcccaccttcatgtggacagaatagtgtaatgtcatcacttatcgtatcgaacggtcaaattccgctcattatcaactccactgatttgtgaccgtaggatacgagggggacaagttgaagcactatatataggaagtgacagtaaagcgagttcagaatatcacatttatagggagcactgcatagcttacaagcttgtaagag

SEQ ID NO: 41 - DNA, 1800 bp, Populus trichocarpa
cattcaaataaataagagattttaggagggaatcatatcagcatccaacctatccatcaattttaatcggatcccagaactacaaattaattttcccaattgaattcctaaaggattggacatttctcaattgagtattccaacaactatatttattggcattttccgttatttcatgcaataaatagcatgaaactattttgaaaacaatttgacatttttctattaaaaagctacaatgatgtcaaatgaaacaagaatttcctaacacgtgagaattttttttataaatttaatcattagaagttcataacacattggagtcgaaaacaaaattcttacaaaatcttcaccatctaagttgtccatagcaaattacattttttacaagagcgatagcgtttgaaaacgcgggataactcgctttctaaaaagttttaatttttgttttttgctaaaaattaaatttttttttatgttttgaattgttttgatacgctgatcttaaaaataatttttttaaaataaaaaaaattattttaatgtatttcaacatgaaaaatactttaaaaagtaatcacaatattctctcaaacaggtccaaaataaaaaaaagaaaaaaaaaaagaagagggagttgctgggctgtttagtaatgtgtaacggaggtgagattataatgggcggaaatggttttagcccgacttctctttagaaatagccatgggcccatggcattcttctttgggctaatttaaattgctagaccattttctttttttttccctaagaaagtactggaccagaccattaagaaccctgtccactccttgtttacttggccattttcaatgcatactgagctggatttgatcgttagaggacctaaagcattgcttacttgtgaccacgtattgctttaaattttgaggttttgagggtgttgttttttaaattattattttttatttagagttgtattaaaataatatttttttatttattaagatttattcttgacatcaaaataataataaaaaatataaaaaaataattttaaataaaaaaaagtaaattttcaatgatctttatttggatcgcaattccaaaccaatactaaaaaccagattgttgagctttcatgaatgttttggttttactttccataatgaaattgctccaactaaaaaaaaaaaggtaaaatctagtgaatccagccaaacctaattggttaactctaaatttttttattttaaatatgaaacaatattatttttaaaaaatcttattgacccaaattgacattaactttttttttatatatatatatatatgaagtaaactaagctctaaaatcactgtgtcaatggcaagctgccaagaaccacagaagtggtcataaatatcttaaattaagggagctgaaagagagagtggaattaatcgaaaggctgcctcagcaagaaccataaagccataaattaactagcatcacacatccatgacgtcctccatgggatgagataaggtcatcgagcttcttccacgtggaaacctctttgtggtgctaacgatgaggctagcatcaaaagaattcccaccttcatgtggacagaatagtgtaatgtcatcacttatcgtatcgaacggtcaaattccgctcattatcaactccactgatttgtgaccgtaggatacgagggggacaagttgaagcactatatataggaagtgacagtaaagcgagttcagaatatcacatttatagggagcactgcatagcttacaagcttgtaagag

SEQ ID NO: 42 - DNA, 2000 bp, Populus trichocarpa
tgggaagggttgtcgggactctcgtgagggtacgacaaaaataataacaaaatgataaaagatggaaacaaaaagcttttaaaaaaacaaaagcaccatggaaacttgtgtccctatcagcttcattaatcggagtcaatctcttaaacttgtaaaccgttaaattctacactcggactaaacttagaaacttaacccgaccaacctacgacctgagatatgaaatggggataactcgacaaaaaaaaaagctaaacaaatcacaaagctcatagcccaataattcaaagtcaaatgaaaaaaattaaataaaaacaaattaataagtcaatgtcaaatgataaaaataaacaaaaaaaaccgaattctaaaaaggattttaaaaaatatcgaactcaaactaggtaaatcattgaaactggtgaactgagtcatgagaacgggacaaccatgtaaaagaaagaaataatcaaaaagaaaaatcctcaatttaaaaaaaaattaaaagataaccaatgaggaccaaatcttgcacaaaaaataattgaaagaaagtaattagggacaaaattgaaaataaaataaatgaagaaaaggaaaaaaaatgagtaatgaaaaaatgaggaccaaaatttgaaaaaaatgaattaaaattgtaaaggacaaaatcaaaaaaataaaataaatgaaaaggatgaaaaaacaacaattaaaagattaaggaccagattgtaaacaaaaaacaaaataaattaaatgcaaagaaggatgaaactgagaaaaataaatttcaagaagcattaaaatcaaagcaaatagaaatctaaagaatgaggaccgaacccaaaacaaattcaaaatggaggacaactaaattttttaagatctagcatgaaaaccaagatctaagagagagaaacgaagggcaggagaaaaaacccattgccgccaccaatcgtggagcacgcgccactccagcagctgcgccacatccttgtgtatcagttgagacggagatcggttttattggccatcgtacttggccacacgcgccttcggaatagcgttgaggaccctgacacactgatgcatgcatgatacacgtcagcatattttactgatttattaatattttaataagtaaaattacaaaaaaaatccaaggacataccattattacaaagaaaccatggtgcaaagactaatatgccctcagaagttaagctttaaatccggaaagtcaaaggtcaacaatgtaaattttagtataaaaataatgcaaagacaaataaacccctccttgcaaggctattttttgtgagcactcagagctataaatgttattttactgtgtaagttaaaaaaaaatacaaaaaaaaactaattattattagattttaagagcaaaatagtattttttaccgtgcattatagtttggaatgcaatctatgcccctgatcaattctaaaataacatttaaatctcattaaaaaatataaagataattattaagaataatgaagagcaaaaccataattacactgcttgaatacgtaattaatcacctcatgatacagcgaaaaactacactgaggccatttaatttttttttgtgagcccttcacccgagtccctagtcgaactaaaagattatcgccatggccatttaatctacgctttttatttattttttcttgagaacttacaattaatttatttttcattttttttttgtataaaagaactatttctcgtaaagaatctcgttaaattcgttgggaaccgaagaggttttattttctaaaatctcggagaatccagagacagaaggagtagatctttggtggacattgaactccgactcttcccgggacacataaaccgtatcctgctaggactattacgcttgattccccattctataaatatatcaaactctgtttagaaaaggagctctcagcaaaaagtttcagatcaggaaggcaggggaacctcaacc

SEQ ID NO: 43 - DNA, 2000 bp, Populus trichocarpa
aatttttttatataattttttatttgattatataataaaaatgatgtttgtaaaatcaaaaaccaactaaatatcagagtgttttattcaagattctgataaacctatgaatatcaaatataaataatttatgtttcccaataaaaaatcaataaaatattaaagaataagattgaaaagaattaagcaagaaaaatcaataaaaatccaattatgaatgatcaaattgaaaaaaaaacaattcaaaaaaataaataaaagaaggcaaaaataaaaagagccaattgtgaaggatcaaattgaaaaaaaaggcccatgagtgcaagcttgaggctgttaaattttttttcttttattgtccacctatggtttttttgaaaaaaaatagcaggcaacttgttgccttctctatccagattttgattgtcggccataggtgttaaacaccataaaaatttatttaaaccataattttggccccaaaacacttgataaacatcttgaagacttaaataaacttgtttatacctttaaataattcaaaaatgataaacaaacaaaaaatcaagtcgaaatcaaaatactttctgagatcagatttacttttttaagaaaactataggtgaaagaacaccttactagaactctttccggcatataaaactcgtacaaaccaatatcgactattttggtagcataattcgttgtcaaccaatattttttctccactagcagaatttaatttaatgactttctctcttccatcttgaactagaaaatggacaaaaaaaatttgttccacaattgagtttttgaaatatttagggaccgagaagttatcatttaaaaagtaagaaggtcaaagtttactttttatccctttttgataacaccacatgtttcctccttgttttacttatcaatctcatttgttttaatcttgtctctcattaacaatttttgataaatcatccacgaaaattgggcattgaaggacacaattgaatagaaaaaaattgaataaacaattatagaattgtgaattgcaacactaaaaaactcatgcattttagagtttttgttaataaataactaatataaaattaatatataaaattaatataatattttaatttttttaaaatgaatcttaaacttaattatcaagtttaatatgatataataattttaataatggtctataattttaatttcaatattactcattcccacttactaaaatagtaaacttaagcaaaagttgtaattagtcatcatgaccgtgaagactcataatatataaaatataataaaaaattactaaaaaaattcaatttaatatatttttaagttaaaaatatttttaaaaaatatctagaagcaaaaccagaaattataccgaacaactcagatgacattgctagctctagaaagagttacccatcacaatcatgatggaattatcaaccatgtaccatatttaaaaaaaaaaaaaaaaacacaccaactctttgaacaaagctaattatttcatatatgataaaacgccctaatttttatcatttgatacggggaaatgacacgtggacatcgatcattaccatattaattattggtgctgaattgatcatatcccatcaaaacatgctttgtttcctttcttaacacacacacataaataacaagtaaattagttgtcttgtgttcataattagtgatgacatattagttattactaatcaaataaaaggcggttggtcggcttccattcttttagggctcttccattcatatgggtcccacggtcggcgccggctatgatgcttactgcaaatttagcatagcaaatcaccagtaggagcgtgtatttaaaccacgcccatgagaccaacgcattgcagcccatcgagaaacacacacaagaactcgagcgagctatattgatagttctaataattaattaagtttaattagtctaataattagtgaaacaagaaaga

SEQ ID NO: 44 - DNA, 1757 bp, Populus trichocarpa
ttcgcaattcaaagcctttttttttttaatgattttgatacatgaaaattaatttaaaaaacattattttaaaaaaaaaaatatttcaccatattactgaaaatacacttattctagttaggctattaatcaaatagattaagtttttaatttgctaaaacttgttaagtttagttaattttttaataatctaaatgacatgataaagtcaaataaaaaggtttaagacctaaattataagtttaacgagttgagttaatttatttcaatccaaaacaatgttatatttttttaaaaattgaaacaatatgattttgaaatatatatatatatatatatatatatatatatatatattttataattttatagtcaaatcaaatttcatccagaaatttaacttctataaaattaattatatttaactaaattaattttcactttatttaatataaaacccgattcaaatcaggttttaaaacaccttaattgaaaatattcaaagattattaactattgtaggaaaaatcattacttttctttgtctcttttatttcacacttggctcgagatttacttgaaataatatgcaacaatttagaatttcatgtggtgggatagatgttttgcaagcttgaagcatgtctttgtgcatatagatttcatgttatagactttagaatttcattttaacagcaatctacctaacaattatttttatataagaagtgatgcccatgtctggattattttttactttttatgtataagaaaatatttttaaaaatattttaattattttctccatttaaactggccaacaattttcatagttggtgggatgctagcaagcacgaaggatggcttgtctgtgactaatgttagcttaatatcttgtaaagatgagattcaaccagcaagaatatatctcatgtttatagacttaattaaataattttctatataatagtaattgaacaaataaagataataatgttattttcatttttcttgtataaaaaagtagcatgtattgattttttatgctgataatcattatgttatttgtccattaacccatctagatattctagacgtgattgagaccctaaccctttttaaattaaatataatcaacaatatattaaagattaaaaaaaaaattgtacggataggtagttaaatatatatatatatatatatatatatatatatatatatatatatatatttcagaaaaatgaagaatattccaaggacattgaagggcatccggtcatggtttcagaagacatcgctggatttcttgctagttaattagctctgaaaaaacttaggaatatcccagaacattaaatttgaccctcagtagaatgattagcatggagaggtaagttacatattgatctctttccttgaggcaacagagagagggacatatttgttttctaatataatttaatttgtatcttcgttatgagcaagagtgtatgaaagcttaaccatacttgttttcagtcataattattttttaaaaaatttatttagttttctaaattagattaattataattccaaatgggtatatcctcaatattccctttctaatttcttgttattctcccatggcttagtgttcatcgagctcgacgtgcattattttttctttatcatattgcttaaaataccaattatataaccatgaaatcctaggcaagaaaattaaccactcccgccaaaagaacgaaaagaaagac

SEQ ID NO: 45-49 - skipped (5 entries)

SEQ ID NO: 50 - protein, 186 aa, Populus trichocarpa
MSGSSGGSSSSSSSRIIDQESGASASQRKFKGARRRKWGKWVSEIRIPGKQERLWLGSYSTPEAAAVAHDIASYCLRGPSSLESLNFPLMLPASVREDMSPKSIQKAASDAGMAIDAQMILNRSLQNEVKVGPENVAINHGPQTQLWEPAAGGGGDSSNRCENWHENNIGTRVGDDLNISIEDYLM

SEQ ID NO: 51 - DNA, 561 bp, Populus trichocarpa
atgagtggtagcagcggcggcagcagcagcagcagcagcagcaggataatagatcaagaaagtggagcaagtgcatctcaaaggaaattcaagggagcaagaaggcgaaaatggggcaagtgggtgtctgaaataaggattcctgggaagcaagaacgactttggttaggttcttattctacacccgaggcagctgcggtggctcatgacatagcttcttattgtttacgtgggccttcttcgttagagagtctgaatttccccctaatgttgcctgcaagtgtaagggaagacatgtcacccaagtccatacagaaagctgcgtcggatgctgggatggcaatcgatgctcagatgatactgaacaggtcgctccaaaacgaggtcaaggttggacctgagaatgttgcgattaatcatgggccacagacacagttatgggaacctgcagcaggtggtggtggtgatagtagtaatcgttgcgagaactggcatgaaaacaatatcggaacgagagtaggggacgatttaaacatctccattgaagattatctcatgtag

SEQ ID NO: 52 - protein, 168 aa, Populus trichocarpa
MSGSSSSRTDQESGASAARKKFKGVRRRKWGKWVSEIRIPGKQDRLWLGSYSTPEAAAVAHDIASYCLRGPSSIESLNFPLMLPASVREDMSPKSIQKAASDAGMAIDAQMILNRVPENEVKFWTASGGVNHGLEIELCEPAGGDHGGNWHGNNTGMREGDISIEDYL

SEQ ID NO: 53 - DNA, 507 bp, Populus trichocarpa
atgagcggtagtagcagcagcagaacagatcaagaaagtggagcaagtgcagctcggaagaaattcaagggagtgaggaggcggaaatggggcaagtgggtgtctgaaataaggattcctggcaagcaagatcgactttggttaggttcttattcaacacccgaggcagctgcggtggctcatgacatagcctcttattgtttacgcggaccttcttcgatagagagtctcaatttccctctaatgttgcctgcaagtgtaagggaagacatgtcacctaagtccatacagaaagctgcttcagatgctggcatggcaattgatgctcaaatgatactgaacagggtaccagaaaatgaggtcaagttctggactgcaagtggtggggttaatcatgggctggagatagagttatgcgaacctgcaggtggcgatcatggtggtaattggcatggaaacaatactggaatgagagaaggggacatctccattgaagattatctctag

SEQ ID NO: 54 - protein, 155 aa, Eucalyptus grandis
MSSSSSEEPRNAKYAGVRRRKWGKWVSEIRVPGTQERLWLGSYTSPEGAAVAHDVASYCLRGPSCLDKLNFPSLLPPSARPGVSPRSAQRAASDAGMAVDARYIARRSDEEADRTSPGHRPEVGWECAQGNEASSGTRGGRGGGDGLSISVDDYL

SEQ ID NO: 55 - DNA, 468 bp, Eucalyptus grandis
atgagcagctcgtcgtccgaggagcccaggaacgccaagtacgccggggtccgccggaggaagtggggcaagtgggtgtcggagatccgggtccccggcacgcaggagcggctctggctcggctcctacacctcccccgagggcgccgccgtcgcccacgacgtcgcctcctactgcctccgcgggccctcctgcctcgacaagctcaacttcccctcgctgctgccgcccagcgcgcggcccggcgtgtcgccgaggtcggcgcagagggccgcctcggacgccggcatggcggtcgacgcgcggtacatcgccaggaggtcggacgaggaagcggacaggacgagccccggccaccgaccagaggtcggttgggagtgtgcgcaagggaatgaggcttcttccgggacgcggggagggagaggaggaggtgatggtttgagcatttcggtggatgactacctgtga

SEQ ID NO: 56 - protein, 388 aa, Populus trichocarpa
MPLAFERGKVNQSIERKRDSVLDGVKDMAVELMMGYSGDSFATKMQENDVREAATAGIQSVEEVIKLLKQNQLEQQQKQQYYQELSAASSSSNLGTDNIMAVTDMAVNNFKKVISLLGRTTRTGHARFRRAPVACPPQQQIQEPEPGPQQQKQQVQEPVPYVRAINSQPTEQGSAFRVYQPTPIHRLPPLPHNQQQKTLLVTKNGLSDRNEMATTINFANSPTISAPSFLSSLTGETDSFQCSKSSGFQFTQPSAGKPPLSSSSLKRKCNSMDDAALKCGSSSSRCHCSKKSRKSRIKRVVRVPAISSKMADIPPDDYSWRKYGQKPIKGSPHPRGYYKCSSVRGCPARKHVERALDDSMMLIVTYEGEHNHSHPIDEAPGALVLESS

SEQ ID NO: 57 - DNA, 1167 bp, Populus trichocarpa
atgcctttggcatttgagagaggaaaggtcaatcaatccatagagagaaagagagattcagtcttggatggtgtaaaagacatggctgtggagcttatgatggggtattctggtgatagttttgctacaaaaatgcaagagaatgatgtgagagaagccgcaactgctgggatacaaagcgttgaggaagtcataaaactgctcaaacaaaatcaactggaacagcaacaaaaacaacaatactaccaagagttgtctgcagcctcttcaagttccaatcttggcacggataatatcatggctgttactgatatggccgtgaacaatttcaaaaaggttatttctttactgggtcgcaccacaagaactggccatgctcgatttagaagagctcctgttgcctgccctcctcaacaacaaatacaagaaccagaaccaggaccgcaacagcaaaaacagcaagttcaagagccagtaccatatgttcgagcaattaattcgcagccaacagagcaaggctctgcttttagagtttatcaaccgaccccaattcatcgtctccctcctttgcctcacaatcagcaacaaaagacactgctggttacgaaaaatggattatcagatcggaatgaaatggctactacgatcaatttcgctaattcgccaacaatatctgctccttctttcttgtcttctttaacaggggaaactgatagcttccagtgttctaagtcttctgggtttcagtttacccaaccttctgctggtaaacctcctttgtcctcttcttctcttaagagaaagtgcaactccatggatgatgctgctctcaagtgtggctcttcttctagtcgctgccactgctccaagaaaagcaggaaatcaagaattaaaagggtggttagagttcctgcaattagtagtaagatggcagatatcccacctgatgattattcctggagaaagtatggccaaaagcccatcaaaggctctcctcatcccaggggatactacaagtgcagtagcgtgagaggatgtccggcacgcaaacacgtggagagagctctagatgactcgatgatgcttattgtgacctatgaaggggaacacaaccactctcatccaatcgatgaagcacctggtgctcttgtccttgaatcatcttaa

SEQ ID NO: 58 - protein, 358 aa, Populus trichocarpa
MAVELMMGYSGDCFATKMQENAVREAAASGIQSVEEVIKLLKQNQLEQQHYQELSAASSSSNLGTDNIMTVTDMAVNNFKKVISLLGRTTRTGHARFRRAPDTPPTQQQIREEPESQQEKRQVQEPGPSVRAINSQPTEQASAFRVYQPTPIHRLPPLPHNQQQKSPLLVTKKGLSDRNEIPTTINFSNSPSISSATSFMSSLTGETDGFQRSMPSRFHFTQPSAGKPPLSSSSLKRKCNSMDDAALKCGSSSGRCHCSKKSRKSRAKRVVRVPAISNKMADIPPDDYSWRKYGQKPIKGSPHPRGYYKCSSVRGCPARKHVERALDDSMMLIVTYEGEHNHSHPFDDAPAALVPESS

SEQ ID NO: 59 - DNA, 1077 bp, Populus trichocarpa
atggctgtggagcttatgatggggtattctggtgattgttttgctacaaaaatgcaagagaatgccgtgagggaagcggcagcttctgggatacaaagcgtcgaggaagtcataaaattgctcaaacaaaatcaacttgaacagcaacactaccaagagttatctgcagcctcttcaagttccaatcttggcacggataatatcatgactgttactgatatggcggtgaacaacttcaaaaaggtcatctctttactgggtcgcaccacaagaactggccacgctcgatttagaagagctcctgataccccccctactcaacaacaaatacgagaagaaccagaatcgcaacaagaaaaacggcaagttcaagagcctggaccatctgttcgagcaattaattcgcagccaacagagcaagcctctgcttttagagtttatcaaccgaccccaattcatcgtctccctcctttacctcacaatcagcagcaaaagagccctcttctggttacaaaaaaagggttgtcagatcggaatgaaattcctaccacaatcaatttctctaattcgccatcaatttcttctgccacttctttcatgtcttctcttacaggggaaactgatggcttccagcgttctatgccttctaggtttcattttacccaaccttctgctggtaaaccccctttgtcctcttcttctcttaagagaaagtgcaactccatggatgatgctgctctcaagtgtggctcttcttctggtcgctgccattgctccaagaaaagcagaaaatcaagggctaaaagagtggtcagagttcctgcaattagcaataagatggctgatattccacctgatgattattcctggagaaagtatggtcaaaagcccatcaaaggctctcctcatccaaggggatattacaagtgcagcagcgtgagaggatgtccagcacgcaaacatgtggagagagctctagatgactccatgatgcttattgtgacctatgaaggggaacacaatcactctcatccattcgatgatgcacctgctgctctcgtccctgaatcatcttaa

SEQ ID NO: 60 - protein, 437 aa, Eucalyptus grandis
MPRGGKARGQIYLYVLRPLSSRLLPLLLIDPPRARLLLHMCSFSSRSRERGMAVELMMGYGSGGDGGVGFAVKKEETALREAASAGIQSVENLIKMLSSSPSSPSGGGVGGGRRAGQDSPSPSSSSSGGPSPAVDIEAATDAAVNKFRKVISLLDRARTGHARFRRAPVADPLPENREAFTPVRPAENPVGSARLQSAEPVSAFKVYCPTPIQRLPPLPHNHHHHHNHNHHHHHHQVQQNPIPVVPKVERKESATPTTINFSTSPPISAANSSFLSSLTGETDSVQRSFSSAGFQMTHHLSQVSSADKPPLSYSLKRKCSSMDDAALKCGSSSGKCHCSKKRKSRLKRVVRVPAVSSKMADIPPDDFSWRKYGQKPIKGSPHPRGYYKCSSVRGCPARKHVERALDDPGMLIVTYEGEHNHSQSVADVKAPLVLESS

SEQ ID NO: 61 - DNA, 1314 bp, Eucalyptus grandis
atgccaagaggaggaaaggcgagggggcagatctatctctatgtcctgcgacccctttcctctcgtcttcttccccttcttcttatagacccccccagggctcggcttcttcttcatatgtgttccttctctagccgctccagggagagaggtatggccgtggagctgatgatgggttacgggagcggcggcgacggcggcgttggcttcgcggtgaagaaggaggagaccgccctccgggaggccgcctccgccggcatacagagcgtcgagaatctcatcaagatgctgtcttcctcgccttcctccccctccggcggcggcgtgggcggcgggcggcgggccgggcaggactcgccgtcgccgtcgtcgtcctcttccgggggcccgagccccgccgtggacatcgaggccgccacggacgccgccgtcaacaagttcaggaaggtcatctcgctgctcgacagggcgaggaccggccacgcccgcttcaggagagcccctgtcgccgaccccctccctgagaaccgggaagcgtttactccggtccgaccggcggagaacccggtcgggagcgcccggttgcagagcgccgagccggtctcggctttcaaggtctactgcccgacgccgatccagcggctgccgcccctgcctcacaaccaccaccaccaccacaaccacaaccaccaccaccaccaccaccaggtccaacagaaccccatcccggtggttccgaaggtggagagaaaggagtccgcgacgccgacgactataaatttctccacctcgccgccgatctcggctgcgaactcctcgttcctgtcctcactgaccggggagacggacagcgtgcagagatccttctcctctgcagggtttcagatgacgcaccatctatcgcaggtttcgtcggcggacaagcctcccttgtcgtactcactgaagaggaagtgcagttccatggacgacgcggctctgaagtgcgggtcgtcctccggcaagtgccattgctcgaagaagaggaaatcgagattgaagagagtggttagagtcccagcggtcagttcgaaaatggcggacatcccaccagatgatttctcatggaggaagtatggacagaagcccatcaaaggctcccctcatccaaggggctattacaagtgcagcagcgtaagaggatgcccggcgaggaagcacgtggagcgggccctggacgacccgggcatgctcatcgtgacctacgagggcgaacacaaccactcccagtccgtcgccgacgtgaaggcgccgctggtcctggaatcttcctag

SEQ ID NO: 62 - protein, 353 aa, Arabidopsis thaliana
MTVELMMSSYSGGGGGGDGFPAIAAAAKMEDTALREAASAGIHGVEEFLKLIGQSQQPTEKSQTEITAVTDVAVNSFKKVISLLGRSRTGHARFRRAPASTQTPFKQTPVVEEEVEVEEKKPETSSVLTKQKTEQYHGGGSAFRVYCPTPIHRRPPLSHNNNNNQNQTKNGSSSSSPPMLANGAPSTINFAPSPPVSATNSFMSSHRCDTDSTHMSSGFEFTNPSQLSGSRGKPPLSSASLKRRCNSSPSSRCHCSKKRKSRVKRVIRVPAVSSKMADIPSDEFSWRKYGQKPIKGSPHPRGYYKCSSVRGCPARKHVERALDDAMMLIVTYEGDHNHALVLETTTMNHDKTL

SEQ ID NO: 63 - DNA, 1062 bp, Arabidopsis thaliana
atgactgttgagctgatgatgagcagctacagcggcggcggaggaggaggtgatggttttcctgcaatcgccgcggcggcgaaaatggaagataccgctttgagagaagctgcttctgcagggattcacggtgtggaggagtttcttaaactgatcggtcaaagtcaacaaccaacggagaagagtcagacggagataaccgcggtgactgacgtcgccgttaacagcttcaagaaggtcatttctctactcggtagatctagaaccggacacgctagattcagacgagctcccgcgtcaacgcaaacgccgtttaagcaaacgccggtggttgaggaggaggtggaggtggaggagaagaagccagaaacaagctccgtgttaacaaaacagaaaacagagcaatatcacggtggtggatctgcgtttagagtttattgtccaacaccaattcatcgtcgtcctcctctatcacacaataacaacaacaatcagaatcaaacaaagaacggttcgtcttcttcatctcctccgatgctcgcaaacggagcaccgtcaacgataaactttgcgccgtcaccaccagtctcagcgacgaactcattcatgtcttctcatagatgtgacaccgatagtactcacatgtcatcaggattcgagttcactaacccatctcagctctctggttcgagaggtaaacctcctttatcatcagcttcgttgaagagaagatgtaattcatctccctcaagccgttgccattgctccaagaaaaggaaatcaagagtaaaaagagtgattagagttccagcagtaagtagcaaaatggctgatataccatcagatgagttttcatggagaaaatatggtcaaaaaccaatcaaaggctctcctcatcctcggggatattacaagtgcagcagtgtaagaggttgtccggcgcgtaagcatgtggagcgtgcactagatgatgcgatgatgctaatcgtgacgtacgaaggagaccacaaccatgctttggttctcgagacgacgacgatgaatcatgacaaaactctttag

SEQ ID NO: 64 - protein, 572 aa, Populus trichocarpa
MERDKLFVSEGANTAATIWNSCSFGMEMQANELSCGPEKLANCFLNPNWDNSLDQSDPFESALSSIVSSPVASGANANANAIPNAGVGGDSLMIRELIGRLGNICNSGDISLQSFVNNNNNSTNTSCYSTPMNSPPKLNLSMMDSQMRGNLPIPGNSVVKHPGLAPFPADFVERAARYSCFGSNNPGGINKQFGLNESELINRLMPRVEPGKLSRVSSNNSMKVTVSQANVQESNKSSPQDGSLNSEKKFSRQSRPTTSENGDSREESSLSEQVPGGKLSMKSQNDANSRKRKSIPRGKAKETPSSSPSASDVKVAAENDESKAKRSKSDETNGSDKDTAKEKEEENGNQKQNKNNSKPPEPPKDYIHVRARRGQATDSHSLAERVRREKISERMKFLQDLVPGCNKVTGKAVMLDEIINYVQSLQRQVEFLSMKLSSVNPRMEINMETLLSKDIFQSRGSMPHSLYPLDASTPVFPYGYQSQQGLALQNGMPSNAETQFSMNPLNAALRRNPSMHLPHLDGFGDPAALQLEFYSSGLSHVGRRPSKCCADGIWSESSGELSRLSALNSHEN

SEQ ID NO: 65 - DNA, 1719 bp, Populus trichocarpa
atggaaagagataagttgtttgtgagcgagggagccaacacagcagcaaccatttggaattcttgcagttttggaatggaaatgcaagccaatgagctgagttgcggtccagagaaacttgccaattgctttctcaatcccaattgggacaactcattggatcagagcgatccctttgagtctgctttgagctccattgtctcatcacctgttgcatccggtgccaacgcaaacgccaacgccattcctaatgctggcgttggtggtgacagtcttatgattagagaacttattggaagactaggaaacatttgcaattctggagacatttcactacaatcttttgttaacaataataacaatagcactaacacttcttgctatagtaccccaatgaattcccctccaaagctgaatctctcgatgatggattcacaaatgagaggaaatctgccaattcctggaaacagcgtagtaaagcatccaggtttagcaccatttccagctgattttgtagagagggctgcacgatattcttgctttggtagcaacaatcctggaggcatcaataaacaattcggattgaatgaatccgaattgattaataggttgatgccacgagtagaacctggtaagctctcgagagtttcgagtaacaattcaatgaaggtcactgtatcgcaagcaaatgttcaagaaagcaacaagagctcaccccaggatgggagtttgaattctgaaaagaaattcagtaggcagtcaaggcctacaacatcagagaatggagattccagggaagaatcttcattgtctgagcaggtcccaggtgggaaattgagcatgaaatcccagaatgacgccaattccaggaaaagaaaatcaattcccagaggaaaagccaaagaaactccctcttcatctccatctgcttctgatgtcaaggttgcagcagagaatgatgaatcgaaggcaaaaagaagcaaatcggatgaaactaatggcagtgacaaggatacagcaaaggaaaaggaagaagaaaatggaaatcagaaacagaacaaaaataattcaaagccgccagagccaccaaaggattatatccatgtcagagccagaaggggtcaggctacagatagccacagtcttgctgaaagagttagaagagagaaaatcagtgaaagaatgaagttcctccaggatcttgttcccggatgcaataaggttactgggaaagcagtgatgcttgacgagattataaactatgtacagtcattgcagcgccaggttgagtttctgtcaatgaagttgtcatctgtgaatccgaggatggagatcaacatggaaactttgttgtccaaggatattttccaatcccgtggatctatgccacatagtctttatccattagatgcctccacgccggtattcccttatggttaccaatcccagcaagggttagccctgcaaaatggcatgccaagcaatgccgaaacccagttctctatgaacccattaaatgctgcgttgcggcgaaacccgagcatgcatttgccacaccttgatggtttcggtgatcctgctgctcttcagctagaattttattcttcaggcctcagccatgtgggaagacgaccttcaaagtgttgtgcagatgggatatggtcagaatcatcaggagagctttcaaggctcagtgccctcaactcacatgaaaattga

SEQ ID NO: 66 - protein, 567 aa, Populus trichocarpa
MEKDKLFMSEGASTAAPIWNSCSFGMEMQTDELNCSSGQLANCFLNPNWDNLLDQSDPFESALSSIVSSPVASSVNANVISNAGVGGDSVLIRELIGRLGNICNSGEMSPQSYINNNNNSTNTSCYSTPLNSPPKLSISMMDSQMRGNLPILGNSLVNHPSLAPFPADPGFVERAARYSCFGSNNLGGLNGQFGLNESELINRMMPRVEPGKLSRVSSNNSMKVAGSQANVQESNKSSPQDGNLNSDKKFSRLSRPSTPENGDSREESSVSEQIPGGELSMKSQTDANSRKRKSIPRGKAKETPSPSPSASDVKVAAENDESSAKKSKSEDTNGSDKDSAKAMEEENGNHKQKKDNSNPPEPPKDYIHVRARRGQATDSHSLAERVRREKISERMKFLQDLVPGCNKVTGKAVMLDEIINYVQSLQRQVEFLSMKMATVNPKMEINMETFLSKDIFQSRGSMPHGLYPLDSSTPAFPYGYQSQQGLALQDGMSRNAESQFSMNPLNAALRRSSSMQLPALDGFGDASHQASAMWQDDLQSVVQMGYGQNQQQDFQGSVPPTQMKIEL

SEQ ID NO: 67 - DNA, 1704 bp, Populus trichocarpa
atggaaaaagacaagttgtttatgagcgagggagccagcacagcagctcccatttggaattcttgcagttttggaatggaaatgcaaaccgatgagctgaattgcagttcagggcaacttgccaattgctttctcaatcccaattgggacaacttattggatcagagcgatccctttgagtctgctttgagctccattgtctcatctccagtggcatccagtgtcaatgccaacgttatttctaatgctggcgttggtggtgacagtgttttgatcagagaacttattggaagactaggaaacatttgcaattccggcgagatgtctccacaatcctacattaacaacaataacaacagcaccaacacttcttgttatagtaccccattgaattcccctccaaagctgagtatttcaatgatggattcacagatgagaggaaatctgccaattcttggaaacagcttagtaaaccatccaagtttagcaccatttcctgctgaccctggatttgtagagagggctgctcgatattcttgctttggaagcaacaatcttggaggcctaaatggacaattcggattgaatgaatcagaattgatcaataggatgatgccccgagtagaacctggtaagctgtcgagagtttcgagtaacaattcaatgaaggtcgctggatcgcaagcaaatgttcaagaaagcaataagagctcaccccaggatgggaatttgaattctgataagaaattcagtcggttgtcaagaccttcaacaccagagaatggagattccagggaggaatcttcagtgtccgagcagatcccgggtggggaattgagcatgaaatcccagactgatgccaattccaggaaaagaaaatcaattcccagaggaaaagccaaagaaactccctctccctctccctctgcttctgatgtcaaggttgcagcagagaatgatgaatcgagtgcaaaaaaaagcaaatcagaggacactaatgggagtgacaaggattcagcaaaggccatggaagaagaaaatggaaatcacaaacagaaaaaagacaattcaaacccgccagagccaccaaaggactatatccatgtcagagccagaaggggtcaggctacagatagccacagtcttgctgaaagagttaggagagaaaaaatcagcgaaagaatgaagtttcttcaggatcttgttcctggatgcaataaggttactgggaaagcagtgatgcttgatgagattataaactatgtgcagtcattacagcgccaggttgagtttctgtcaatgaagatggcaactgtgaacccgaagatggaaattaacatggaaactttcttgtccaaggatattttccaatcccgtggatccatgccacatggtctttatccattagattcctccacgccggcattcccttatggttaccaatcccagcaagggttagccctacaagatggcatgtccaggaatgcagaatcccagttctctatgaacccattaaatgctgcattgcggcgaagctcgagtatgcagttgcctgcccttgatggctttggtgatgcttctcatcaggcctcagcaatgtggcaagatgatcttcaaagtgttgtgcagatgggatatggtcagaatcagcagcaggactttcaaggctcagtgccaccaactcagatgaaaattgagctatga

SEQ ID NO: 68 - protein, 531 aa, Eucalyptus grandis
MEGSSTPLTQNSSTFGIGIHPNDQLPNCFLVAGWEDSLDQGDPFESALSSIVSSPVAPHAGEGEAGMIRELIGRLGSICDSGQASPGSYNHSTTNTPCYSTPLNSPPELSLSMADQLAHGGFPAPGSHFPGHPSFVSVMADPGFAERAARLSCFGPRNVNAANLNGGLGLNASEFLGKQANKLDSGRFCRVPSSQSLRANVGSQICAQGNERSFLQPGVSISTPENGEMGESREGSSISEQVTHGEMRANGQIDVNSRKRKPILKAKGRNSAVSPQSAKDSEVPMENEEPITKKIKPAETDGNEKDAAKGDQKQSKENSKMAEPQKDYIHVRARRGQATDSHSLAERVRREKISLRMKALQDLVPNCNKVTGKAMMLDEIINYVQSLQRQVELLSMKLSTLNPTVDFNLEAFLSKDILHPQGPLPNSLYPVDSSGSMLYGYQPPQGLMPMPSVVSSNMDAQFPVNFLNSGIHRDASLNLPLCVDNYGEASAPAPALWEDDLQSVVQMGLGQIEPQRVEQGSLATSQMKVEL

SEQ ID NO: 69 - DNA, 1596 bp, Eucalyptus grandis
atggaaggaagctccactccattgactcagaattcatccacctttggcattggcattcaccccaacgaccagctccccaactgcttcctcgtcgccggctgggaggactccctggatcagggcgatccctttgagtccgccctgagctccattgtgtcgtccccggtcgcgccccacgctggcgagggcgaggcgggcatgatccgggagctaatcgggaggctcggcagcatctgcgattccggccaggcctccccggggtcctacaaccacagcaccaccaacactccctgttacagcacccctctgaattcgccgcccgagctcagcctctcgatggcagatcagctcgcccacgggggcttcccggcccccggcagccattttccgggccacccgagtttcgtgtcggtcatggcggatcccgggttcgccgagagggcggcgaggctctcttgcttcggccctaggaatgtgaatgccgccaatctaaacggtggcctcgggttgaatgcatcggaattcctggggaaacaggcgaataagctcgattcggggagattttgcagggttccaagcagtcagtcactgagggctaatgtcggatctcaaatctgtgcacaagggaatgagagaagcttcctccagccaggggtctctatttcgacccctgaaaatggagaaatgggggaatcccgcgaggggtcttcgatctccgagcaggtcacgcatggggagatgcgtgccaatggacaaatcgacgtgaattcaagaaagaggaaaccgatcctgaaagcaaaagggcgaaactcggctgtttctccacaatctgctaaagattctgaggttcccatggagaatgaagaaccgataaccaagaaaatcaaacccgccgagactgacggcaatgagaaagatgcagcaaagggggaccagaaacagagcaaggagaattcgaagatggcggagccgcagaaggactatatccatgtgagagcaagaaggggtcaggccactgacagccatagccttgctgaaagagtcaggagagagaagataagtctgaggatgaaggctctccaggatctcgtgcctaactgcaacaaggtcactgggaaagctatgatgctcgatgagatcattaactacgtccagtccttgcaacgtcaggttgagcttctctccatgaagctgtcgactctgaaccccacagtggatttcaatctggaagctttcctgtcaaaagatatcttgcaccctcaaggacccttaccgaattctctctatccagttgattcgtcggggtccatgttgtatggttatcagcccccgcaaggactaatgccgatgccaagcgtcgtttccagcaatatggatgcccaatttccagtgaactttttgaattccggaattcacagagatgccagcttgaacttgcctctttgtgtggacaattacggcgaagcttctgctccggccccagctctatgggaggatgacctccaaagtgtagtccaaatgggtctcggccagattgagccccagagagtagaacaaggctccctggcgacttctcagatgaaagttgagttgtag

SEQ ID NO: 70 - protein, 498 aa, Arabidopsis thaliana
MDNELFMNTEFPPPPEMATHFEHQQSSSSAMMLNWALMDPNPHQDSSFLWEKSTEQQQQQSIFDSALSSLVSSPTPSNSNFSGGGGDGFLIRELIGKLGNIGNNNNNSGEIYGTPMSRSASCYATPMSSPPPPTNSNSQMMMNRTTPLTEFSADPGFAERAARFSCFGSRSFNGRTNTNLPINNGNNMVNNSGKLTRVSSTPALKALVSPEVTPGGEFSRKRKSVPKGKSKENPISTASPSPSFSKTAEKNGGKGGSKSSEEKGGKRRREEEDDEEEEGEGEGNKSNNTKPPEPPKDYIHVRARRGQATDSHSLAERVRREKIGERMKLLQDLVPGCNKVTGKALMLDEIINYVQSLQRQVEFLSMKLSSVNDTRLDFNVDALVSKDVMIPSSNNRLHEEGLQSKSSSHHHQQQLNIYNNNSQLLPNISSNNMMLQSPMNSLETSTLARSFTHLPTLTQFTDSISQYQMFSEEDLQSIVGMGVAENPNNESQHMKIEL

SEQ ID NO: 71 - DNA, 1497 bp, Arabidopsis thaliana
atggacaacgagctgtttatgaacacagagtttccaccaccgccggagatggcgacgcatttcgaacaccaacagtcttcttcatcggccatgatgcttaattgggctttaatggatccaaatccgcatcaagattcttcctttttatgggaaaagtcaacggaacaacaacaacaacaaagcatctttgactctgctttaagctcattagtctcatcaccgacgccgtcaaattccaacttctccggcggtggcggtgacggttttctcatcagagaactcatcggaaagcttggaaacatcggtaataataataacaactccggtgagatctacggaactccgatgtctcgctccgcctcatgttacgcaactccgatgagctctccaccgccaccgacgaattcgaattctcagatgatgatgaacagaacgacgccgttgacggaattctcagcagatccgggttttgcggagagagcagctagattctcttgttttggtagtcggagctttaacggaagaaccaatacaaatcttccgattaacaacggtaataacatggtcaacaactccgggaagctgacacgtgtctccagcacaccagctcttaaggctcttgtttcaccggaagtcacacccggcggcgaattttcccggaagagaaaatctgtgcctaaaggaaaatccaaagaaaaccccatttctacagcttctccatctcctagtttctcaaagacggcggaaaagaatggtggaaaaggaggaagtaaaagttcagaagaaaaaggaggaaaaaggagaagagaagaagaagatgatgaagaagaagaaggagaaggtgaagggaacaaaagcaataacacaaaaccacctgagcctcctaaagattacattcatgttcgagctcgacgaggccaagcaaccgatagtcacagcctcgccgaacgagttcggagggagaaaattggtgaaaggatgaagcttcttcaagatcttgtgcctggatgcaataaggttactggaaaagcactgatgcttgatgaaattataaactacgtacaatcattgcaaagacaagttgagttcttgtcaatgaagttatcatcagtgaacgacaccaggctggattttaacgtggacgctcttgtgtcaaaggatgttatgattccatcaagtaacaaccgattgcatgaagaaggactccaatcaaagtcttcaagtcatcatcatcaacaacaacttaatatttataacaataattcacaattacttcccaatatttcttccaataacatgatgctccagtctcctatgaactctttggaaacctctaccttagccagaagcttcactcacttaccaacacttacccaatttactgactcaatttctcagtatcaaatgtttagcgaagaagatttacaaagcatagtaggaatgggagtggcagaaaaccccaacaatgaatctcaacacatgaaaattgagctttga

SEQ ID NO: 72 - protein, 456 aa, Arabidopsis thaliana
MENELFMNAGVSHPPVMTSPSSSSAMLKWVSMETQPVDPSLSRNLFWEKSTEQSIFDSALSSLVSSPTPSNSNFSVGGVGGENVIMRELIGKLGNIGDIYGITASNGNSCYATPMSSPPPGSMMETKTTTPMAELSGDPGFAERAARFSCFGSRSFNSRTNSPFPINNEPPITTNEKMPRVSSSPVFKPLASHVPAGESSGELSRKRKTKSKQNSPSAVSSSKEIEEKEDSDPKRCKKSEENGDKTKSIDPYKDYIHVRARRGQATDSHSLAERVRREKISERMKLLQDLVPGCNKVTGKALMLDEIINYVQSLQRQVEFLSMKLSSVNTRLDFNMDALLSKDIFPSSNNLMHHQQVLQLDSSAETLLGDHHNKNLQLNPDISSNNVINPLETSETRSFISHLPTLAHFTDSISQYSTFSEDDLHSIIHMGFAQNRLQELNQGSSNQVPSHMKAEL

SEQ ID NO: 73 - DNA, 1371 bp, Arabidopsis thaliana
atggagaacgagctgtttatgaatgcaggagtttcgcatccgccggtgatgacgtcaccgtcttcttcgtcggcgatgcttaagtgggtttcaatggagactcagccagtggatccaagtctcagtcgcaatctgttttgggaaaagtcaacggaacagagcatttttgattcggctctgagctcactcgtctcttctcctacgccgtcaaattcaaacttttcggttggcggagtaggtggagaaaatgtcattatgagagagctcatcgggaaactgggtaatatcggcgatatctatggaattacggcgagcaatggaaactcgtgttacgcaactccgatgagctctccaccgcctggaagtatgatggagacgaaaacgacgacgccgatggcagaactgtccggcgacccgggattcgctgagagagcggcgaggttctcgtgttttggtagccggagttttaacagcagaacaaactcgccgtttccgattaataacgaaccacccatcacaaccaatgagaaaatgccacgtgtatcaagcagcccagtttttaagcctcttgcgtctcatgttcccgccggcgaatcgtccggtgaactttcccggaaaagaaaaactaaatccaagcagaattctccttctgcagtttcatcatcaaaggagattgaagagaaggaagattctgatccaaagagatgcaaaaaatcagaagaaaatggagacaaaactaaatcaattgatccttacaaagattacattcatgttagagctcgacgaggccaagccaccgatagtcacagtctcgccgaacgagttcgaagagagaaaataagcgaaagaatgaagctgcttcaagatcttgtccctggatgcaacaaggttactggaaaagcactgatgttggatgaaattataaactatgtccaatcattgcaacgacaagttgagttcttgtcgatgaagttatcgtcagtgaacaccaggctggactttaacatggacgctctcttgtctaaggatatatttccttcaagcaacaatctaatgcatcatcaacaagtacttcaattagattcttcagcagaaacgttattgggtgatcatcacaacaaaaatttgcaattgaaccctgatatttcttctaataacgtaataaaccctttggaaacttctgaaactagaagcttcatttctcacttaccaacacttgctcatttcactgactctatttctcagtattcaacattttccgaagatgatttacatagcattattcatatgggttttgcgcaaaaccgtctccaagaattgaaccaaggttcatcaaaccaagtaccatcgcacatgaaagctgaactttga

SEQ ID NO: 74 - protein, 301 aa, Populus trichocarpa
MAVDLVRYSKMEDQMAIQEAASAGLESMEHLIFAFSNQTRQSHQLDCGEITNFTVAKFKQVISMLNRTGHARFRRGPTSSPSSYPVPVRPVPQEPQKLNLDFVNSNSPPKAESKNDLSLGSQYSKDSLSSGTTTSSFVSSVTADGSVSNGKQGGSSLFGTQARSTGKPPLSSTHRKKCHDHALSARKISSGGSCHCSKRRKSRVKRTIRVPAVSSKIADIPADEYSWRKYGQKPIKGSPYPRGYYKCSSVRGCPARKHVERAVDDSAMLIVTYEGEHRHSHTPLPGDVTASAAMRHVFHST

SEQ ID NO: 75 - DNA, 906 bp, Populus trichocarpa
atggctgtggatctagttaggtattcaaagatggaagatcagatggctatacaagaagctgcatcagctgggctcgagagcatggagcacttgatctttgcattctctaaccaaactcgacaaagccaccaacttgactgcggagaaatcacaaacttcaccgttgctaagttcaagcaagtcatctccatgttgaaccggaccggtcatgcccgttttcgccgtggaccaacttcttctccttcttcctacccggttcccgtccgacctgtccctcaagagcctcaaaaactgaaccttgattttgttaacagtaatagcccccctaaagctgagtcgaaaaatgacctgtctttgggtagtcagtattcaaaggatagccttagctctggcaccactacctcatccttcgtgtcttctgttacagctgatgggagtgtctctaatgggaaacaaggtggctcttctcttttcggaactcaagcgcgatctaccggaaaaccacctctctcatcgacccaccgcaagaaatgccacgatcatgccctctccgccagaaagatctcctccggtggaagctgtcattgctccaaaagaaggaaatcaagggttaagaggacaataagggtaccagccgtgagttccaagattgccgatataccagcagatgagtactcatggagaaaatatggtcaaaagccaatcaagggctcaccatacccaagagggtattacaagtgtagcagtgttagaggatgtccagcaaggaagcatgtggagcgtgccgtagatgactcggccatgcttatcgtgacttacgagggggagcaccgtcactcacatactccgttgccgggagacgtcaccgcgagtgctgcaatgcgacacgtgtttcactcaacatga

SEQ ID NO: 76 - protein, 300 aa, Populus trichocarpa
MAVDLVGYSKMEDQMAIQEAASAGIKSMEHLIFALSNQTQQSHQLDCREITSFTVAKFKQVISILNRTGHARFRRGPTSSNPVSVRPVVQEPQKLNLDFFKSNNTFKSETKNDLSFGSQYSKDCFSSGTTTSSFLSSVTADGSVSDGKQGGSSSLFGTHPRPTGKPPLSSIHRKKCHDHTLSTSKISSSGGSCHCSKRRKSRVKRTIRVPAISSKVADIPADEFSWRKYGQKPIKGSPYPRGYYKCSSVRGCPARKHVERAVDDPAMLIVTYEGEHRHSHAPLPENVTANAAMRHVFQST

SEQ ID NO: 77 - DNA, 903 bp, Populus trichocarpa
atggctgttgatctagttgggtactcaaagatggaagatcagatggctattcaagaagctgcatcagctgggattaagagcatggagcacttgatctttgcactctctaaccaaacccaacaaagtcaccaacttgactgcagagaaatcactagcttcaccgttgctaagttcaagcaagtcatctccatcctgaaccggaccggtcatgcccgtttccgccgtggacccacttcttccaacccggtttccgtccgacctgtcgtccaagaacctcaaaaactaaatcttgatttctttaagagtaacaatacctttaaatctgagaccaaaaacgacttgtcattcggcagtcagtattccaaggattgttttagctctggcacgactacttcgtccttcctgtcttctgttacagctgatgggagtgtctctgatgggaaacaaggtggctcgtcttctcttttcggaactcatcctcgacctaccggaaaaccacctctctcatctatccatcgcaagaaatgccatgatcataccctctccaccagcaagatctcctcctccggtggcagctgccattgctccaaaagaaggaaatcaagggtgaagaggacaataagagtcccagcaataagttccaaagttgctgatataccagcagatgagttctcatggagaaaatatggtcaaaagccaatcaagggttcaccttacccaagagggtactacaagtgtagtagtgtgaggggatgtccagcaaggaagcacgtggagcgtgccgtagatgatccggccatgcttattgtaacatacgaaggggagcaccgtcactcacatgctcccctaccagaaaatgtcacagccaacgctgccatgcgacacgtgttccagtcaacatga

SEQ ID NO: 78 - protein, 343 aa, Eucalyptus grandis
MAIELHLGFSKMEDHTAIQEAASQGLKTMEHLIGVLSRQNLHHPGAVDCTDLTDRTVSKFRKVISLLDRTGHARFRRAPLPSSSSSSSKSAPVASPVPPAVQSRSQPLAPTPIQAPTSSQPSPASFLHAQPKQSLTLDFTRPSILGPNSKGVSEIEFAKDSFSVSSNSSFMSSAITGDGSVSNGKLGTSMFIAPASGPASSAGKPPISSVPYKKRCHEHDPSDNISGKHSGSGSGKCHCSKRRKNRVKKVTRVPAISNKIADIPADEFSWRKYGQKPIKGSPFPRGYYKCSTMRGCPARKHVERAPDDPTMLIVTYEGEHRHSQSASQEIVPAGAMNLVFKST

SEQ ID NO: 79 - DNA, 1032 bp, Eucalyptus grandis
atggcgatcgagctgcatcttggcttctccaagatggaggatcacacggcgatacaggaggccgcgtctcaggggctgaagaccatggagcacctgatcggcgtcctctcccgccagaacctccaccaccccggcgccgtcgactgcaccgacctcaccgaccggaccgtctccaagttcaggaaggtcatctccctcctggaccgcaccggccacgcccgcttccggcgggccccgctcccctcctcctcctcttcctcctccaagtctgcccccgtcgcttcccctgtccccccggcggttcagtctcggagccagcctctagcgccgacgcccatccaggccccgacgagctcgcagccgtctccggccagcttcctccacgcgcagcccaagcagagcttgaccctcgacttcacccggccgagcatcctgggccccaactccaaaggcgtttccgagatcgagttcgcgaaggacagcttcagcgtgtcgtccaactcttccttcatgtcttcggcgatcaccggcgacggaagcgtttcgaacgggaagctggggacgtcgatgttcatagctccggcgtccggcccggcttcgtccgccggaaagccaccgatctcgagcgtgccgtacaagaagcggtgccacgagcacgacccctccgataacatctccggcaagcactccggctccggcagcggcaagtgccactgctccaaaagaaggaaaaaccgagtgaagaaggtgacgagagtgccggcgatcagcaacaagatcgcggacatcccggccgacgagttctcgtggaggaagtacggacagaagccgatcaaagggtctcccttcccacgaggttactacaagtgcagtacaatgagagggtgccccgcgaggaaacacgtggagagggcccccgacgatccaacgatgctgatcgtgacgtacgagggggagcatcgtcactcccagtccgcgtcgcaggagattgtgcccgccggtgcgatgaacctggtattcaagtcaacctga

SEQ ID NO: 80 - protein, 325 aa, Arabidopsis thaliana
MAVDLMRFPKIDDQTAIQEAASQGLQSMEHLIRVLSNRPEQQHNVDCSEITDFTVSKFKTVISLLNRTGHARFRRGPVHSTSSAASQKLQSQIVKNTQPEAPIVRTTTNHPQIVPPPSSVTLDFSKPSIFGTKAKSAELEFSKENFSVSLNSSFMSSAITGDGSVSNGKIFLASAPLQPVNSSGKPPLAGHPYRKRCLEHEHSESFSGKVSGSAYGKCHCKKSRKNRMKRTVRVPAISAKIADIPPDEYSWRKYGQKPIKGSPHPRGYYKCSTFRGCPARKHVERALDDPAMLIVTYEGEHRHNQSAMQENISSSGINDLVFASA

SEQ ID NO: 81 - DNA, 978 bp, Arabidopsis thaliana
atggccgtcgatctaatgcgtttccctaagatagatgatcaaacggctattcaggaagctgcatcgcaaggtttacaaagtatggaacatctgatccgtgtcctctctaaccgtcccgaacaacaacacaacgttgactgctccgagatcactgacttcaccgtttctaaattcaaaaccgtcatttctctccttaaccgtactggtcacgctcggttcagacgcggaccggttcactccacttcctctgccgcatctcagaaactacagagtcagatcgttaaaaatactcaacctgaggctccgatagtgagaacaactacgaatcaccctcaaatcgttcctccaccgtctagtgtaacactcgatttctctaaaccaagcatcttcggcaccaaagctaagagcgccgagctggaattctccaaagaaaacttcagtgtttctttaaactcctcattcatgtcgtcggcgataaccggagacggcagcgtctccaatggaaaaatcttccttgcttctgctccgttgcagcctgttaactcttccggaaaaccaccgttggctggtcatccttacagaaagagatgtctcgagcatgagcactcagagagtttctccggaaaagtctccggctccgcctacggaaagtgccattgcaagaaaagcaggaaaaatcggatgaagagaaccgtgagagtaccggcgataagtgcaaagatcgccgatattccaccggacgaatattcgtggaggaagtacggacaaaaaccgatcaagggctcaccacacccacgtggttactacaagtgcagtacattcagaggatgtccagcgaggaaacacgtggaacgagcattagatgatccagcgatgcttattgtgacatacgaaggagagcaccgtcataaccaatccgcgatgcaggagaatatttcttcttcaggcattaatgatttagtgtttgcctcggcttga

SEQ ID NO: 82 - protein, 321 aa, Arabidopsis thaliana
MTVDIMRLPKMEDQTAIQEAASQGLKSMEHLIRVLSNRPEERNVDCSEITDFTVSKFKKVISLLNRSGHARFRRGPVHSPPSSSVPPPVKVTTPAPTQISAPAPVSFVQANQQSVTLDFTRPSVFGAKTKSSEVVEFAKESFSVSSNSSFMSSAITGDGSVSKGSSIFLAPAPAVPVTSSGKPPLSGLPYRKRCFEHDHSEGFSGKISGSGNGKCHCKKSRKNRMKRTVRVPAVSAKIADIPPDEYSWRKYGQKPIKGSPHPRGYYKCSTFRGCPARKHVERALDDSTMLIVTYEGEHRHHQSTMQEHVTPSVSGLVFGSA

SEQ ID NO: 83 - DNA, 966 bp, Arabidopsis thaliana
atgaccgttgatattatgcgtttacctaagatggaagatcaaacggctatacaagaagctgcatcacaaggcttaaaaagcatggaacacttgattcgtgtcctctctaaccgtcccgaagaacgtaacgttgattgctctgagatcactgatttcacagtttctaagttcaagaaagttatctctcttcttaaccgttccggtcacgcccggtttagacgtggtccggttcattcccctccttcctcctccgttcctccaccggtgaaagtgacaactccggctcccactcagatctctgctccagcaccggttagcttcgttcaggcaaatcaacaaagcgtgacgttagatttcactagaccgagcgtttttggcgctaaaaccaagagctcggaggttgttgagtttgctaaagagagctttagcgtatcttctaactcttctttcatgtcttctgcgatcaccggtgatggaagtgtctctaaaggctcttcgatctttcttgctccggctccagcggtgccagtgacttcctccgggaaaccgccgctttctggtcttccttacaggaagagatgctttgaacatgaccactctgaaggcttttccggcaagatctctggctccggcaacggcaagtgccattgcaagaaaagccgaaaaaatcggatgaagagaaccgtgagagtaccggcggtaagtgcaaagatcgccgatataccaccagacgaatattcatggagaaagtatggacaaaaaccgatcaaaggctcaccacatccacggggttattacaagtgtagtacatttagaggatgtccagcgaggaaacacgtggaaagagctttggatgattcaacgatgttgattgtgacgtacgaaggagagcaccgtcatcaccagtccacgatgcaggagcatgtaactcctagcgtgagtggtttggtgtttggttcggcttga

SEQ ID NO: 84 - protein, 347 aa, Populus trichocarpa
MEGVEEANRAAVESCHRVISLLSQPQDQVQYRNLMVETGEAVFRFKKVVSLLNTGLGHARVRKLKKLPTPLSQSILLDNPLSSTDHPSKTPQFLQSSSYLESQPIQELGSIAKNCLSLGTPSLELSSNGKNPLQLGQPTPAAHYQFLQQQQLHRLQLQQQQQMKQQAEMMFRKSNSGISLNFDSSSCTPTMSSTRSFISSLSIDGNVANLEGSAFHLTGAARSSDQSSQQHKRKCSGRGEDGSMKCGSSVRCHCSKKRKHRVKRSIKVPAISNKLADIPPDDYSWRKYGQKPIKGSPHPRGYYKCSSMRGCPARKHVERCLEDPSMLIVTYEGEHNHPRIPAQSTNT

SEQ ID NO: 85 - DNA, 1044 bp, Populus trichocarpa
atggagggggttgaagaagctaaccgggcagctgtggagagctgccatagagttataagtttgctatcccaaccccaagatcaggttcaatataggaatttaatggtggaaactggagaggctgtgtttaggttcaagaaagtagtttcccttttaaatactggtttaggtcatgcaagagttcgaaaacttaagaagttaccgacccctttatcccaaagcatcctcttagacaacccactgagcagtacagaccacccatccaaaacaccccagtttctccagtccagtagttacctggaaagccaaccaattcaagaattgggctcaattgctaaaaattgtctatctttgggaaccccatccctggaattgagttcaaatgggaaaaaccctcttcagcttggccaacccacgccagcagcgcactatcagttccttcagcaacagcaactgcataggctacagcttcaacagcagcagcaaatgaagcagcaagctgagatgatgtttagaaaaagcaatagtgggattagcttgaatttcgatagttctagctgcactcctacaatgtcatctaccagatcttttatatcgtccttgagtattgatggtaatgtggctaatttggaaggaagtgcattccatttaacgggggcggctcgctcctcagatcagagttcacagcaacacaagaggaaatgttctggaaggggagaagatggaagtatgaaatgtggaagcagcgttagatgtcattgctcaaagaagaggaaacatagggtgaagaggtcgatcaaggttcctgctattagcaacaagcttgctgatatccctcctgatgattactcatggagaaagtatgggcaaaagccaatcaagggttctcctcatcctaggggatattacaaatgtagcagtatgagaggttgtcctgcaaggaagcatgtggagaggtgcttggaagatccgtccatgcttattgttacctatgaaggtgaacataaccacccaaggattccagcacaatccacaaacacgtaa

SEQ ID NO: 86 - protein, 351 aa, Populus trichocarpa
MEGVEEANRAAVESCHRVISLLSQPQDQVQYRNLMVETGEAVFRFKKVVSLLNTGLGHARVRKLKKLPTPLSQSILLDNSLNRTGHSSKTPQFLQSSSYLESHPIQELGSSAKNCLSLGTPSLELSSTGKNPLQLGQPTSAANYQFLQLQQQQLHRLQLQQQQQQQMKQQAEMMFRKSNSGISLNFDSSSCTPTLSSTRSFISSLSIDGSVANLEGSAFHLMGPARSSDQSSQQHKRKCSGRGEDGSVKCGSSGRCHCSKKRKHRVKRSIKVPAISNKLADIPPDDYSWRKYGQKPIKGSPHPRGYYKCSSMRGCPARKHVERCLEDPSMLIVTYEGEHNHPRIPAQSANT

SEQ ID NO: 87 - DNA, 1056 bp, Populus trichocarpa
atggagggggttgaagaagctaacagagcagctgtggagagctgccatagagttataagtttgttgtctcaacctcaagatcaggttcaatataggaatttaatggtggaaactggcgaggctgtgtttaggttcaagaaagttgtttctcttttaaatactggtttaggtcatgcaagagttcggaaacttaagaagttaccgacccctttatcccaaagcatccttttagataactcacttaatagaacaggccactcatccaaaacacctcagtttctccagtctagcagttacctggaaagccatccgattcaagaattgggctcaagtgctaagaactgtctttctctgggaaccccatctttggaattgagttcaaccgggaaaaaccctcttcagcttgggcaacccacttcagcagctaattatcagttccttcagcttcaacagcagcagctgcacaggctacagcttcagcagcagcagcagcagcaaatgaagcagcaagctgagatgatgtttagaaaaagcaatagtggaattagcttgaattttgatagttctagctgcacacctacactgtcatccaccagatcttttatatcttccttgagtatagatggtagtgtggctaatttggaaggaagtgcattccatttaatggggccggctcgctcctcggatcagagttcacagcaacacaagaggaaatgttctgggaggggagaagatggaagtgtgaaatgtggaagcagtggtagatgtcattgctcgaagaagaggaaacatagggtaaagaggtcgatcaaggtacctgctattagcaacaagcttgctgatatcccccctgatgattattcctggagaaagtatggacaaaagcccatcaagggctctcctcatcccaggggatattacaagtgtagcagtatgagaggttgtcctgcaaggaagcatgtggagaggtgcttggaagatccgtccatgcttattgttacctatgaaggtgaacataaccacccgaggattccagcacaatctgcaaacacataa

SEQ ID NO: 88 - protein, 343 aa, Eucalyptus grandis
MEEVEEANRAAVESSHRVLSLLSQPQDQVQCRNLMLETGDAVFRFKRVVSLLNTCLGHARVRKLKKLPTPLPQKALLDNPIVRTDQSSKSLQLLPPNYPENAIQELNTHHKASLSLGNPNLELSSNGKSPLHLAQQAPSAHYHFLQQQQQQQKLQFQQQMKHQAEMMYHRSNSGISLNFDSSSCTPTMSSTRSFISSLSIDGSVANLDANAFHLIGAARSSDQNSQHKRKCSGRGEDGSMKCGSSSRCHCSKKRKHRVKRSIKVPAISNKLADIPPDDYSWRKYGQKPIKGSPHPRGYYKCSSMRGCPARKHVERCLEDPSMLIVTYEGDHNHPRVPSQSANT

SEQ ID NO: 89 - DNA, 1032 bp, Eucalyptus grandis
atggaggaggttgaagaagcgaacagagcagctgtggagagctcccacagggttctgagcctcttgtcgcagccgcaagatcaggttcagtgtagaaatctgatgcttgagactggtgatgctgtattcaggttcaagagagtggtttctcttctcaatacttgcttgggtcatgctagagttaggaagttaaagaaactaccgacccctttgccccaaaaggccctcttggacaaccctattgttagaactgaccaatcttcaaagagtctccaactcctccctcctaattaccctgaaaatgcaattcaggaactcaatacacatcacaaagcctctctttctttaggtaacccgaacttggagttgagctccaatggcaaaagccctcttcatttagcccagcaagcgccatcagcacactatcactttctccagcagcagcagcagcagcagaagttacagttccagcaacaaatgaaacaccaagctgagatgatgtaccataggagcaatagtggcataagcttgaatttcgatagctctagctgcacgcccaccatgtcgtctacgaggtctttcatttcttcactgagtatagatgggagcgtggctaacttggatgcgaatgctttccatttgatcggggcggctcgctcatctgatcagaactcgcagcataagaggaagtgctctggcagaggagaggatgggagcatgaaatgcggtagcagtagtagatgtcattgctctaagaagaggaaacatagggtgaagaggtcgattaaggtacctgctataagcaacaagcttgcggatattcctcccgatgattattcgtggaggaagtacgggcagaagccaatcaagggttctcctcatcctaggggatactacaaatgtagcagcatgagaggttgccctgcaaggaagcatgtggaaaggtgcttggaggacccgtctatgctcattgtcacctacgaaggtgaccataaccaccccagggtgccatcacaatctgccaatacatga

SEQ ID NO: 90 - protein, 380 aa, Arabidopsis thaliana
MEEIEGTNRAAVESCHRVLNLLHRSQQQDHVGFEKNLVSETREAVIRFKRVGSLLSSSVGHARFRRAKKLQSHVSQSLLLDPCQQRTTEVPSSSSQKTPVLRSGFQELSLRQPSDSLTLGTRSFSLNSNAKAPLLQLNQQTMPPSNYPTLFPVQQQQQQQQQQQQQEQQQQQQQQQQQFHERLQAHHLHQQQQLQKHQAELMLRKCNGGISLSFDNSSCTPTMSSTRSFVSSLSIDGSVANIEGKNSFHFGVPSSTDQNSLHSKRKCPLKGDEHGSLKCGSSSRCHCAKKRKHRVRRSIRVPAISNKVADIPPDDYSWRKYGQKPIKGSPYPRGYYKCSSMRGCPARKHVERCLEDPAMLIVTYEAEHNHPKLPSQAITT

SEQ ID NO: 91 - DNA, 1143 bp, Arabidopsis thaliana
atggaggagatagaaggaacaaacagagcagctgttgagagttgtcatagagttcttaatcttttacatagatcacagcaacaagatcatgttggttttgaaaagaatttagtatctgaaactagagaagctgtgattaggttcaagagagttgggagtttgttaagcagtagtgttggtcatgctaggtttagaagagctaagaaacttcagagtcatgtctctcaaagtctcttacttgatccatgtcaacaaaggacaacagaagttccatcatcatcttctcagaaaacaccggtactccggtctggtttccaggaattgagcttgagacaaccttcagattcactcactttagggactcgctcttttagtttaaactcaaatgctaaagctcctctccttcagcttaatcagcagacaatgcctccttcgaattatcctactttgtttccagtacaacaacaacaacaacaacaacaacaacaacaacagcaggagcagcagcagcagcagcagcagcaacagcaacagtttcatgaacggttacaagctcaccatcttcatcagcaacagcagctacagaaacatcaagctgagcttatgcttaggaaatgcaatggtgggataagtttgagtttcgataactctagttgtactccaactatgtcatccactaggtcctttgtttcttcacttagcatagatggtagtgttgctaatatagagggaaagaactccttccattttggggttcctagttcaactgatcagaattcactacattctaagaggaaatgccccttgaaaggagatgaacatggaagcttaaaatgcgggagctctagccgatgccactgcgctaagaagaggaaacatcgggttaggagatcgattagagtaccggctataagtaacaaggttgcagatatccctcctgatgattattcatggcgaaaatatggtcagaagcccatcaagggctctccttatcccagaggatattacaaatgtagtagcatgagaggttgtccagcgaggaagcatgttgagagatgtttggaagatccggcaatgcttattgttacttatgaagcagagcataaccacccgaaattgccatctcaagctataacaacttaa

SEQ ID NO: 92-99 - skipped (8 entries)

SEQ ID NO: 100 - protein, 178 aa, Zea mays
MRRAEPVGEQADAERRMSGYKGVRRRRWGKWVSEIRVPGSRERLWLGSYATPEAAAVAHDTAVYFLRGGGGAGDVAALNFPERAAAAYGAGGRLSPRSVQRVASDAGMAADAQLVAAREDTRALRAGIGGGASARPRDRDAGDACAGRAHNASLHSTGAGREQPVSGEISVDDMDILL

SEQ ID NO: 101 - DNA, 537 bp, Zea mays
atgaggcgcgcggagccggtcggcgagcaggcggacgcggagcggcgcatgagcgggtacaagggcgtgcggcggcgccggtgggggaagtgggtgtcggagatccgggtgcccggctcgcgggagcgcctgtggctcggctcctacgccacgcccgaggccgccgccgtcgcgcacgacacggccgtctacttcctccgcggcggcggcggcgcgggcgacgtcgcggcgctcaacttccccgagcgcgcggcggccgcgtacggcgcagggggccgcctgtcgccccggtccgtgcagcgcgtggcgtccgacgccggcatggccgccgacgcgcagctcgtcgcggcgcgggaggacacccgcgcgcttcgcgccggcattggcggtggcgccagcgcgcgcccgcgcgatcgggatgctggtgacgcctgcgcgggccgtgcgcacaacgctagccttcacagtacgggcgccggaagggagcagcctgtctccggggagattagcgtggatgacatggatattttgctgtag

SEQ ID NO: 102 - protein, 186 aa, Zea mays
MSRAATNSGAERRCRYRGVRRRAWGKWVSEIRVPGTRERLWLGSYAAPEAAAVAHDAAACLLRGCAGRRLNFPGRAACYYACGGQQPLSPRSVQRVASDAGMAADAQIVDARAALASPPPVVQPAALAGIIGGAAREGGGGVRGPACAPAPPSNGAGSSSTYWSTPSSEPPLVYGDISVDDIEILI

SEQ ID NO: 103 - DNA, 561 bp, Zea mays
atgagccgcgcagcgaccaacagcggcgcggagcggcggtgccggtacaggggcgtgcggcggcgggcctgggggaagtgggtgtcggagatccgggtgccgggcacgcgggagcggctgtggctgggatcctacgcggcgcccgaggccgccgccgtcgcgcacgacgccgccgcgtgcctcctccgcggctgcgcgggccgccgcctcaacttcccgggccgcgccgcctgctactacgcctgcggcgggcagcagccgctgtcgccgcgctccgtgcagcgcgtcgcgtccgacgccggcatggccgccgacgcgcagatcgtcgacgcgcgggcggccctcgcctcgccgccgcccgttgtccagcccgccgctctcgctggcattattggcggcgccgcgcgagaaggcggcggaggcgtgcgaggccccgcgtgcgcgccggcgccgccaagcaacggcgctggcagcagcagtacgtattggtccacgccgagcagtgagccgccgcttgtttacggggacattagcgtagacgacatagagatcttgatttga

SEQ ID NO: 104 - protein, 316 aa, Zea mays
MAVDLMGCYAPRRANDQLAIQEAAAAGLRSLELLVSSLSTQAAAPHRAAAHQLQKPPSQPPIGEIADQAVSRFRKVISILDRTGHARFRRGPVVEAPPPVPPPAVSAPALPVAHVVAPVGAAQPQSLTLDFTKPNLAVSGGATSVTSTSFFSSVTAGEGSVSKGRSLVSSGKPPLSGHKRKPCAGAHSEATTNGSRCHCSKRRKNRVKRTIRVPAISAKIADIPPDEYSWRKYGQKPIKGSPYPRGYYKCSTVRGCPARKHVERATDDPAMLVVTYEGEHRHTPGAPAPAPSPLAAASPVPASAAAAVSAGNNGLV

SEQ ID NO: 105 - DNA, 951 bp, Zea mays
atggccgtggacctgatggggtgctacgccccgcgccgcgccaacgaccagctcgccatccaggaggcggcggcggcggggctccgcagcctggagctcctcgtgtcgtcgctgtccacgcaggccgccgcgccgcacagggccgcggctcaccagctgcagaagccgccttcgcagccgccgatcggcgagatcgccgaccaggccgtctccaggttccgcaaggtcatctccatcctggaccgcaccggccacgcccgcttccggcgcgggcccgtggtcgaggcgccgccaccggtgcctcctccggccgtctccgctcccgctctccccgtggcgcacgtggtggctcccgtcggcgcggcgcagccccagagcctgaccctggacttcacgaagccgaacctggccgtgtcgggcggcgccacgtccgtcacctccacgtccttcttctcctcggtcacggccggcgagggcagcgtgtccaagggccgcagcctggtgtcctccggcaagccgccgctgtccggccacaagcggaagccctgcgccggcgcgcactccgaggccaccaccaacggcagccgctgccactgctccaagagaaggaaaaaccgcgtgaagaggaccatcagagtgccggcgatcagcgccaagatcgcggacatcccgccggacgagtactcgtggaggaagtacggccagaagcccatcaagggctccccctacccacggggctactacaagtgcagcaccgtgcgcgggtgcccggcgaggaagcacgtggagcgcgccaccgacgacccggccatgctggtggtgacgtacgagggcgagcaccgccacacgccgggcgcgcccgcgcccgcgcccagccccctggcggccgcgtcgccggtgcccgcctccgccgccgccgccgtctccgccggcaacaacgggcttgtctag

SEQ ID NO: 106 - protein, 331 aa, Zea mays
MTTLDLMGGYGRVDEQVAIQEAATAGLRGMERLILQLSQAGTGERSLSPPAVQAQRQQQKQLEQIQQQVDCRELTDMTVSKFKKVISILNRTGHARFRRGPVAARSQSQSQGPASPEPAQSAPAPAARPLTLDFTKSVSGYSRDSGFSVSGASSSFLSSVTTGDGSVSNGRAGGSSFLMFPPAPGAASCAKPPPAGAAQKRKCHDHAHSENVAGGKYGANGGRCHCSKRRKHRVKRTIRVPAISPKVADIPADEYSWRKYGQKPIKGSPYPRGYYKCSTVRGCPARKHVERDPADPSMLIVTYEGEHRHSPASGQDPPPPSLAPLPELPSH

SEQ ID NO: 107 - DNA, 996 bp, Zea mays
atgacgaccctcgatctgatgggagggtacgggcgggtggacgagcaggtggccatccaggaggccgccacggcggggctgcgcgggatggagcgtctcatcttgcagctctcccaggctggcaccggggagcggtcgttgtccccaccggcggtacaggcgcagcgccagcagcagaagcagctggagcagatccagcagcaggttgactgccgggagctcacggacatgacggtgtccaagttcaagaaggtgatctccatcctgaaccgcacggggcacgcgcggttccggcgtggccccgtggcggcgcggtcgcagtcgcagtcgcagggacctgcctcccccgagcccgcgcaatcggcgccggctcccgccgcgaggcccctgacgctggacttcaccaagtcggtgtccggttacagcagggactccgggttcagcgtgtccggcgcgagctcgtcgttcctgtcgtcggtgacgaccggggacgggagcgtgtcgaacgggcgcgcgggaggctcgtcgttcctcatgttcccaccggcgcccggcgcggccagctgcgcgaagccgccgcccgccggtgcggcgcagaagcgcaagtgccacgaccacgcgcactcggagaacgtcgccggcggcaagtacggggctaacggcgggcgctgccactgctcgaagcgcaggaagcaccgtgtgaagcgcacgatccgcgtgccggcgatcagccccaaagtggcggacatccccgccgacgagtactcgtggcgcaagtacggccagaaacccatcaaggggtcgccctacccacgcggctactacaagtgcagcacggtgcgcggctgccccgcccggaagcatgtggagcgcgaccccgccgacccgtcgatgctgatcgtcacctacgagggcgagcaccgccacagccccgcctccggccaggacccgccgccgccgtcgctcgcgccgctgccggagctgcccagccattga

SEQ ID NO: 108 - protein, 350 aa, Zea mays
MDSDYIASLLMGSSAPALSFAALDAGFLDTLRGGGGGGLFGVPAEAGCGGGSPEGSSVSDPAWARARDYGNARKRKAPPTGSAGGKEACLSKVAEAKGPDGKRCRVVGASDSPVKPKEEEEEAAASDALVEVKAQKKGKGKSSKPAVEPPKDYVHVRARRGQATDSHSLAERVRREKISQRMKFLQDLVPGCNKVVGKALMLDEIINYVQSLQQQVEFLSMKLATVNPELDFSNLSTLLHKDMYQQPCGGPSASSVFPLESAGAAFPFCEQADLFHSFGSGGSGSGSGMEDQCSLSLLLDTALPHAASPQFAFQKQQRDLWEDGLQHALPTPTTGSEQRQEEDGLLVPDL

SEQ ID NO: 109 - DNA, 1053 bp, Zea mays
atggacagcgactacattgccagcctgctcatgggctcatccgcccctgcactcagcttcgccgcgctggacgccgggttcctcgacacgctacgcggcggcggcggcgggggcctcttcggggtgcccgcggaggcagggtgtggcggcgggtctccggaggggtcgtcggtgtccgacccagcgtgggcgcgcgctagggactacggcaatgccaggaaacgcaaggcgccgcccacggggtccgccggtggcaaggaggcctgcttgagcaaggttgcggaggccaagggtccggacgggaagaggtgcagagtagtgggtgccagcgacagtccggtgaagccgaaggaagaggaggaggaggcggcggcgagcgacgccttggttgaagtcaaagcgcagaagaagggcaaggggaagagctcgaagccggcagtcgaaccgcccaaagactacgtccatgtccgggcgcggcgggggcaggcgactgacagccacagccttgcagagagggttagaagagagaagattagccagaggatgaaatttctacaggacctagtgccaggatgcaacaaggtggtcggcaaggcactcatgctcgatgagatcataaactacgtccagtcgctgcagcagcaagttgagttcctgtccatgaagctcgccactgtgaacccagagcttgatttcagcaacctatcgacactcctgcacaaagacatgtaccaacagccatgtggtggcccttcggcaagttcggtctttccactggaaagcgccggcgcagcttttccattctgcgagcaggcggatcttttccacagctttggctcgggtggtagcggtagcggtagtggtatggaggatcagtgctctctaagcctgctgctagacacggctctgccccacgcggccagcccacagtttgcttttcaaaagcagcaaagggacttgtgggaggatggcctacagcatgctttgcctacccctactaccggtagcgagcaaaggcaggaggaggatgggcttttagtacccgacctttga

SEQ ID NO: 110 - protein, 460 aa, Zea mays
MDCGPPDQLPPSSAPACFLNLNWDQSMAAATAGDHLDLVSSPASNSTAADGLALHGISPQPQYGGTPLSSPRKLNLSMMGQFHHYPPMGHLDQFLADPGFAARAARLSGFDGRPGGSGYGGAVPGQFGLPDAGPIGGALRELELGNGRDESSVSDPASASAEMALKAPSDGNAKKRKASGKGKGKDGPGSTAATKEESSGKRCKSAEESNGAEENSGKGKAAAQSNSDNGGKKQGKDGASKPPEPPKDYIHVRARRGEATDSHSLAERVRREKISQRMKLLQDLVPGCNKVVGKAVMLDEIINYVQSLQRQVEFLSMKLATVNPQLDFNNLPNLLPKDMHQSCGPLQNSHFPLETSGAPLPYLNQGNPLIGCGLPNGMDNSQSSMHPLDPAFCRPMSSQQHPFLNGVSDAASKVGTFWQDDLQSVVHMDMGQQSQQEMAPTSSNSYNDGSLQTVHMKMEL

SEQ ID NO: 111 - DNA, 1383 bp, Zea mays
atggactgcgggccgcccgaccagctgccgccgtcgtcggcgccggcgtgcttcctcaacctcaactgggaccagtccatggccgccgccacggctggcgaccacctcgacctggtctcctccccggcgtccaactcgacggcggctgacggcctcgctctccacgggatctcgccgcagccgcagtacggaggcactccgctcagctcgccccgcaagctgaacctctccatgatgggccagttccaccactacccgccgatgggccatctagaccagttcctcgccgacccaggcttcgccgcgcgcgcggcgaggctctccggcttcgacggccgccccggtgggagtggctacggcggcgccgtcccgggacagtttggcctccccgacgccggccccatcggcggcgcattgagggagctggagctcgggaacggccgggacgagtcatcggtgtccgatccggcgtccgccagcgccgagatggcgctcaaggcgccttccgatggcaatgcgaagaaacggaaggctagcgggaaggggaaaggcaaggacggccccgggtccaccgccgccaccaaggaggagtccagtgggaaacggtgcaaatcggcggaggagagcaatggcgcggaggagaactccggcaagggtaaggccgccgcgcagagcaacagcgacaacggtgggaagaagcaggggaaggacggcgcgtccaagcctccggagccgcccaaggactacatccacgtccgggcgaggcgcggcgaggcgacagacagccacagcctcgctgagagggtgagaagggagaagatcagccagcggatgaagcttctgcaggatctcgtcccgggctgcaacaaggtggtcggcaaggcggtgatgctggatgaaatcataaactacgtgcagtccttgcaacggcaagtcgagttcctgtccatgaaactggccaccgtgaatccccagctggacttcaacaacctgcctaacctccttcctaaagatatgcaccagtcctgcggcccgctgcagaactcgcatttcccgctggagacctcaggcgcgccgctgccatacctcaaccaggggaaccctctaataggctgcggcctacccaacggcatggacaacagccagagctccatgcacccgctcgacccggcgttttgccggccgatgagctcgcagcagcaccctttcctcaacggtgtcagcgacgcagcgtccaaggtcgggactttctggcaagatgaccttcagagcgtagtccacatggatatggggcagcagagccagcaggagatggctcccacctcctccaacagctacaacgacggttcgttgcaaacagtgcacatgaaaatggagctttga

SEQ ID NO: 112 - protein, 404 aa, Zea mays
MKEGRPGAGDYIASLLSSSPRLDFGGEEEEDCLDRFCGDPGFAARAARLSSFSGQRFAVTAGLFGLPPPLPAASGGGEFAGSREASSVSDPASAMKDANAKKRKAPAAAAAKGKGREPSAQAQAGEPKGPDAKRCCKAEGGEGEEGSPVKLPKPEQAGSDSSVEDGGAQNQKPPPPVKGKNAKPVEPPRDYVHVRARRGQATDSHSLAERVRRERISQRMKVLQDLVPGCNKVIGKALMLDEIINYVQSLQRQVEFLSMKLATVNPLDLSNLPTLLQKDMFQACGASASSVFSLESCSPGFPFGGQGDVFQSFVPNGLENPCGGLNPLDLALSQATGGQFGFQDGTAGTNLQQRNYWEEEEEDLQSVFHIDDNGQSQEHGASASAQSFHGQLQPQEGHMKMEFF

SEQ ID NO: 113 - DNA, 1215 bp, Zea mays
atgaaagagggcagacccggcgccggcgactacattgccagcctgctaagctcgtcgccgaggctcgacttcggcggggaggaggaggaggactgcctggacaggttctgcggcgacccggggttcgcggctcgcgcggcgcggctgtccagcttcagcgggcagcgcttcgccgtcaccgcgggcctcttcgggctgcccccgccgctgcccgccgcgagcggcggcggcgagttcgccgggtcccgggaggcgtcgtcggtgtcggacccggcgtcggcgatgaaggacgccaatgccaagaagcggaaggcgcccgcggcggcggcggccaagggcaaaggcagggagccatctgcgcaggcacaggcaggggagccgaagggtccggacgccaagaggtgctgcaaggcggagggaggcgagggggaggaggggagccccgtgaagctgcccaagccggagcaggccggcagcgacagctccgtcgaggacggcggcgcgcagaaccagaagccgccgccgccggtgaagggaaagaatgccaagccggtggagcctcccagggactacgtccatgtccgggccaggagagggcaggctaccgacagccacagcctcgcagagagggtgagaagggagaggatcagccagaggatgaaggtccttcaggacctggtgccaggatgcaacaaggtgatcggcaaggcgctgatgctcgacgagatcataaactacgtgcagtcgctgcaacggcaggtcgagttcctctccatgaagctcgcaaccgtcaacccactggacctgagcaacctgcccacgctcctacaaaaagatatgttccaggcctgcggcgcttcggcgagctcggtcttctcgctggagagctgcagcccggggttcccgttcggcgggcaaggggacgtgttccagtccttcgtcccgaacggcctggagaacccgtgcggcggcctgaacccgctggacctggctctgtcccaggctaccggcgggcagttcggtttccaggacggaacggccggcacaaacctgcagcaaaggaactactgggaggaggaggaggaggacctgcagagcgtgttccacatcgacgacaacgggcagagccaggagcacggggcctcagcttcagcacaaagcttccatggtcagcttcaaccacaagagggccacatgaagatggagttcttctga

SEQ ID NO: 114 - protein, 397 aa, Zea mays
MEGMEEANRTAVESCHRVLALLSNPHGQLVPSKELVAATGEAVAKFGSLTAKLSNSNGDGLLQGHARVRKVKKPLHIFDSNLFLESSAVAAAAAPAKTPSPSPILGLQLFPRYHQFEGSSSKDPVRIPTQFPKRLLLEKPTAGMEGSTSQSPPIVQMVQPVSVAPPAGTPTPALPPAHLHFIQQQQSYQRFQLMQQMKIQSEMMKRSNLGDQGGSLSGGGGGGRKGVNLKFDSSNCTASSSRSFLSSLSMEGSLASLDGSRTSRPFQLLSGSQTASTPELGLVQRRRCAGREDGTGRCATGSRCHCSKKRKLRIRRSIKVPAISNKVADIPADEFSWRKYGQKPIKGSPHPRGYYKCSSVRGCPARKHVERCVDDPSMLIVTYEGDHNHNRVLAQPA

SEQ ID NO: 115 - DNA, 1194 bp, Zea mays
atggaggggatggaggaggccaacaggacggcagtggagagctgccaccgggtgctggcgctcctctccaacccgcacggccagctcgtccccagcaaggagctcgtggccgccaccggggaggccgtcgccaagttcggctcactgacggccaagctctccaactccaacggcgatggcctactgcagggccacgctagggtcaggaaggtcaagaagcccctgcacatcttcgacagcaacctcttcctcgagagctctgcggtggccgccgccgctgctccggccaagacgcccagcccgagcccgatccttggcctccagctgttcccgaggtaccaccagtttgagggctcgtcgtctaaggatcctgtcaggatccctacccagttccccaagaggttgctgctagagaagccgactgccggtatggaggggtcgacgtcgcagtcccctccgatcgtccagatggtccagccggtgtccgttgcgccccccgcagggacgcccaccccggcattgccccccgctcaccttcatttcatccagcagcagcaaagctaccagaggtttcagctcatgcagcagatgaagatccagagcgagatgatgaagaggagcaatcttggtgatcagggtggtagcttaagtggcggcggcggcggcggtcgtaagggtgtgaatctcaagtttgacagctctaattgcacggcgtcatcgtctcgctcgttcctttcgtctctgagcatggaagggagtcttgcgagtttggatggaagccggaccagcaggccgttccagctacttagtggctctcagacagctagcacgccggagctgggcctggtgcaaaggagaaggtgcgctggcagggaggatgggactggtcggtgtgcaaccgggagccggtgccattgttcaaagaaaaggaagctaaggataaggaggtccatcaaagtccctgcaataagcaacaaggttgcagacatcccagctgatgaattctcatggaggaagtatgggcagaagccaattaagggatccccacatcctaggggttattacaagtgtagcagtgtgagaggctgccccgcgaggaagcatgtcgagaggtgcgtggacgacccctcgatgctgattgttacctatgaaggtgaccacaaccacaaccgagttctagcccagccagcctga

SEQ ID NO: 116 - protein, 374 aa, Zea mays
MEEVEVANRAAVESCHRVLALLSQQRDPALLKSVASETAEACAKFRKVAALLGSGVGHARGRFSRRVRPLGLVGHKSPVGSGGNNPVEMLPSAAAVTSPSPSTSYPPQMRARLNGVPDPRGLDMACSSSSKSGGVGGGGAHPFGGAPKLVQPLSVQFQIGNVAHRYPFHQQPPSRQKLQAAEMFRRSSSGTISLKFDSPIPSGGGGAAGTVSFVSSLSMDGSVGVASLDGKRPFHLVGTPVAASDTAADAHRAPKRRCTCRGGEEDGRGNKCGTSGRCHCSKRRKLRIKRSIKVPAISNKVADIPPDEYSWRKYGQKPIKGSPHPRGYYKCSSVRGCPARKHVERCVDDPAMLIVTYEGEHGHTQLPAQPSTQT

SEQ ID NO: 117 - DNA, 1125 bp, Zea mays
atggaggaggtggaggtggccaaccgggccgcggtggagagctgccaccgtgtgctggccctgctctcgcagcagcgggacccggccctgctcaagagtgtagcgtcagagacggccgaagcctgcgccaagttcaggaaggtagccgccctcctcggcagcggtgtcggccacgctagaggcaggttctccagacgagtccggcctctggggctcgttggccacaagagccccgtggggagcggcggcaacaacccggtggagatgctgcccagcgccgccgccgttacgtccccgtctccgtcaaccagctacccgccgcaaatgcgcgctcggctgaacggcgtgccagacccacgagggctggacatggcctgctccagcagcagcaagagcggcggcgttggcggaggcggcgctcatccattcggcggagcgccgaagctggtgcagccgctgtccgtgcagttccagatcgggaacgtcgcgcacaggtacccgttccaccagcagccgccgtcgcggcagaagctgcaggccgccgagatgttcaggaggagcagcagcgggacgatcagcctcaagttcgatagcccaatccctagcggtggcggtggcgccgctggcaccgtgtcgttcgtgtcgtccttgagcatggacgggagcgtgggcgtggcaagcttggacgggaagcggccgttccatctggtcggcaccccggtggcggcgagcgacacggcggcagacgcccaccgcgcgcccaaacgccggtgcacgtgtagaggaggcgaggaggatgggagaggcaacaagtgcggcacctccggcaggtgccattgctcaaagagaaggaagctgcggatcaagaggtcgatcaaagtgccagccatcagcaacaaggtcgccgacatacctcccgacgagtactcgtggcgcaagtacgggcagaagccgatcaagggctccccgcacccgaggggctactacaagtgcagcagcgtcaggggctgcccggcgaggaagcacgtcgagcggtgcgtggacgacccagcgatgctgatcgtgacgtacgaaggcgagcacggccacacccagctgccggcgcagccttccacccagacgtag

SEQ ID NO: 118 - protein, 367 aa, Zea mays
MEEVEVANMAAVESCHRVLALLSQQQDPALLKSVASETAEACAKFRKVAALLGSASGGGGCGHARGRFSRRVRPLGLVNQKSPLGIATGSGNPLEMMPSTAAAAGSPSPPQSTSYAQMRARLSSAPESSRGLDLACSSSRCSPHPFGAPKLVQPLSVQFQIGSVAHRYPFHQQQSRQKLQAEMFRRSNSGISLKFDSPSPSGGAAGTMSSARSFMSSLSIDRSMASLDGKRPFHLVGTPVASDPADAHRAPKRRCTGRGEDGRGKCATTGRCHCSKRRKLRIKRSIRVPAISNKIADIPPDEYSWRKYGQKPIKGSPHPRGYYKCSSVRGCPARKHVERCVDDPAMLIVTYEGEHSHTQLPAQPAQT

SEQ ID NO: 119 - DNA, 1104 bp, Zea mays
atggaggaggtggaggtggccaacatggccgcggtggagagctgccaccgggtgctggctctgctctcgcagcagcaggacccagccctgctcaagagcgtagcttcagagacggctgaagcctgcgccaagttcaggaaggtagcggccctcctcggcagtgccagtggcggaggtggctgtggccatgctagaggcaggttctccagacgagtccggcctctggggctcgtcaaccagaagagccccttggggatcgccaccggcagcggcaacccgctggagatgatgcccagcacagctgctgctgctgggtctccatctccacctcagtcgactagctatgcgcaaatgcgcgctcggcttagcagtgcgccagagtcctcacgagggctggatttggcctgctccagcagcaggtgtagccctcatccatttggagcccccaagctggtccagccactgtctgtgcagttccagattgggagtgttgcgcataggtacccgttccaccagcagcagtcgaggcagaagctgcaggccgagatgttcaggaggagcaacagtgggatcagcctcaagttcgatagccctagccccagcggtggtgctgctggcaccatgtcgtctgcgagatcattcatgtcgtcgttgagtatagacaggagcatggcgagcttggatgggaagcggccgttccatttggtaggcaccccggtggcgagcgacccagcagatgcgcaccgtgcgcccaaacggcgatgcacgggtagaggggaggatggaagaggcaagtgtgccaccactggcagatgccattgctcaaagagaaggaaactgcggattaagaggtcgattagagtgccagccattagcaacaaaatcgctgatatccctcctgatgagtactcgtggcgcaagtacgggcagaagccaattaagggttccccacacccgaggggttactacaaatgcagcagcgtcaggggctgcccagcaaggaagcacgtcgagcgatgtgtagacgacccggcgatgctaatcgtgacatacgaaggcgagcacagccacacccagctgccagcacagcctgcccagacctag

SEQ ID NO: 120 - protein, 369 aa, Zea mays
MEEVEEANREAVESCRRVLALLSHPHDPAQVRSIALGTDEACTKFRKVVSLLSNGEVGTGEAGPSGTSASASHPRAKLVSRRQNPGFLTQKGFLDSNTPVVVLNSAAHPSPTSAQVHPRAGALDTEGVHPLGVGGPPKLVQPLSAHFQFGNVSSRYQQLPSHHHRHQQQEKLQAAEMFKRSNSGINLKFESASGTGTMSSARSFLSSLSMDGSVVASLDGKLPSSSSSFRLIGAPAMSDPANAAQQAPRRRCTGRGKDGTGKCALAGRCHCSKRSKKLRVKRSIKVPAVSNKIADIPPDEYSWRKYGQKPIKGSPHPRGYYKCSSVRGCPARKHVERCVDDSAMLIVTYEGEHNHTGMPAQSAAAAAQV

SEQ ID NO: 121 - DNA, 1110 bp, Zea mays
atggaggaagtggaggaggcgaacagggaagccgtggagagctgccgcagggtgctagccttgctctcccatccgcatgaccccgcgcaggtcaggagcatagctctggggacggacgaagcatgcaccaagtttaggaaggtggtctccctgctcagcaatggagaagtaggaacaggagaagccggaccatcaggcacaagcgcaagcgcaagccatcctagagctaagcttgttagcagaagacagaatccagggttcttgactcagaaaggcttcctggacagtaacaccccggtcgtggtgctgaacagcgccgcccatccttctccgacctccgcgcaggtgcatccaagagccggagcattggatacggagggcgtgcaccccctcggagttggaggacctcccaagctggtccagcctttgtccgcgcattttcagttcggcaatgtgtcgtcgaggtatcagcagttaccgagtcatcatcatcgtcatcagcagcaggagaagctgcaggccgccgagatgttcaagagaagcaacagcgggataaacctgaagttcgagagcgccagcggcacgggtacaatgtcgtcggcgaggtccttcctgtcgtctctgagcatggatggcagcgtggtggctagcctggatggcaagctgccgtcgtcgtcgtcatcgttccgtttgatcggtgcgcctgcaatgagcgatccggcgaacgccgcgcagcaggccccgaggcggcggtgcacgggccgcgggaaggacgggactggcaagtgcgctttggcgggcaggtgccattgttcaaagagaagtaagaagttgcgggtgaagaggtcgattaaggttcctgccgttagtaacaagatcgctgatatacctccggatgagtactcgtggaggaagtatgggcagaagccgatcaagggttcccctcatcctaggggctactacaaatgcagcagtgtgaggggctgtccagctaggaagcacgtggaacggtgtgtggatgattcggcgatgctcatcgtgacatacgagggcgagcacaaccacaccggaatgccagctcagtcagcagcagcagcagcacaggtgtag

SEQ ID NO: 122 - protein, 354 aa, Zea mays
MEEVEEANREAVESCHRVLALLSQPHDPAQARSIALGTDEACARFRKVVSLLSNGGAGLGEAGPSCGSASASRPRAKLVSRRQNPGFLTQKGFLDSNTPVVVLNSAHPSTTSAQVYPRTGALVDAQSVHPLGVGGPPKLVQPLSAHFQFGSVPARYQFPNQQQQKLHAEMFKRSNSGVNLKFESASGTAGTMSSARSFLSSLSMDGSVASLDAKSSSFHLIGGPAMSDPLNAQQPPRRRCTGRGEDGTGKCAVTGRCHCSKRSRKLRVKRSIKVPAISNKIADIPPDEYSWRKYGQKPIKGSPHPRGYYKCSSVRGCPARKHVERCVDDSAMLIVTYEGEHNHTRMPTTQSAQV

SEQ ID NO: 123 - DNA, 1065 bp, Zea mays
atggaggaagtggaggaagcgaacagggaagccgtggagagctgccacagggtgctcgccttgctctcccagccgcatgaccccgcgcaggccaggagcatagctctgggcacggacgaagcatgtgccaggttcaggaaggtggtctctctactgagcaatggaggagcggggctaggagaagccgggccgtcatgcggaagcgcaagcgcaagccgtcctagagctaagcttgttagcagaagacagaatccagggttcttgacccagaaaggcttcctggacagcaacaccccggtcgtggtgttgaacagcgcccatccttctactacctccgcgcaggtgtaccctagaactggagctctcgtcgatgcacagagcgtgcaccccctcggagtcggaggacctcccaagctggtccagcccttgtccgcgcactttcagttcggcagtgtgccggctcggtatcagttcccgaatcagcagcagcagaagttgcacgccgagatgttcaagagaagcaacagcggggttaacctgaagttcgagagcgccagtggcactgctgggacgatgtcgtcggcgaggtccttcttgtcgtctctgagcatggacggtagcgtggctagcctggacgccaagtcatcgtcgttccatttgatcggtggacctgcgatgagcgatccgctgaacgcgcagcagcccccgaggaggcggtgcacgggccgtggggaggatgggaccggcaagtgcgctgttacagggaggtgccactgttcgaagagaagtaggaagttgcgggtgaagaggtcgattaaggttcctgccattagtaacaagattgccgatatacctccggatgaatactcgtggaggaagtatgggcagaagccaattaagggttcccctcatcctaggggttactacaaatgcagtagcgtgaggggctgcccagccaggaagcatgtggaacggtgcgtagatgattcggcgatgctcatcgtgacatatgagggcgagcacaaccacaccagaatgccaacaactcagtcagcacaggtgtaa

SEQ ID NO: 124 - protein, 395 aa, Zea mays
MEAMEEANRTAVESCHRVLALLSNPHGQLVPSRELVATTGEAVARFGSLAAKLSSSNGNGLQGHARVRKTKKPLPIFYSNLFLESSSAVAAAATVAKTPSPSPTTGLQLFPRYHQMEGSSCKDPVRIPAQFPKRLLLENLAAGLEGSSPPAPPVRMVQPVSVAPPAGMPTPALPAAHLHFIQQQQSYQRFQLMQQMKIQSEMVKRSNLGEQGGSLSGGGGGGKGVNLKFDSSNCTASSSRSFLSSLSMEGSLASLDGSRASRPFQLVSGSQTSSTPELGLVQRRRCAGKEDGSGQCATGSRCHCSKKRKLRIRRSIKVPAVSNKVADIPADEFSWRKYGQKPIKGSPHPRGYYKCSSVRGCPARKHVERCVDDPSMLIVTYEGDHNHSRVLAQPA

SEQ ID NO: 125 - DNA, 1188 bp, Zea mays
atggaggcgatggaggaggccaacaggacggcagtggagagctgccaccgggtgctggcgctcctctccaacccgcacggccagctcgtccccagcagggagctcgtggccaccaccggggaggccgtagccaggttcggctccctggcggccaagctctccagctccaacggcaatggcctgcagggccacgctagggtcaggaagaccaagaagcccctgcccatcttctacagcaacctcttcctcgagagcagctctgcggtggccgccgccgcgactgtggccaagacgcccagtccgagcccgaccactggcctccagctgttcccgaggtaccaccagatggagggctcgtcgtgtaaggatcctgtcaggatccctgcgcagttccccaagaggttgctgctggagaacctggctgccggtctggaggggtcgtcgccgcctgcccctccggtccggatggtgcagccggtgtccgttgcgcctcccgcagggatgcccaccccggcattgcccgccgcacacctccatttcatccagcagcagcagagctaccagaggtttcagctcatgcagcagatgaagattcagagcgagatggttaagaggagcaatcttggtgagcagggtggtagcttaagtggcggcgggggcggtggtaagggtgtgaacctcaagtttgacagctccaattgcacggcgtcatcgtctcgctcgttcctttcgtctctgagcatggaaggaagtcttgcgagcttggatggaagccgggccagcaggccgttccagctagttagtggctctcagacatctagcacaccggagctgggcctggtgcaaaggagaaggtgtgctgggaaggaggatgggagtggtcagtgcgcaaccgggagccggtgccattgttcaaagaaaaggaagctaaggataaggaggtccatcaaagtccctgcagtaagcaacaaggttgcagacatcccagctgatgagttctcgtggaggaagtatgggcagaagccaatcaagggatccccacatcctaggggttactacaagtgtagcagcgtgagaggctgccccgcgaggaagcacgtcgagaggtgcgtggacgacccttcgatgctgatcgttacctacgagggtgaccacaaccacagccgagttctagcccagccagcctga

SEQ ID NO: 126 - protein, 331 aa, Zea mays; identical to SEQ ID NO: 106

SEQ ID NO: 127 - DNA, 996 bp, Zea mays; identical to SEQ ID NO: 107

SEQ ID NO: 128 - protein, 316 aa, Zea mays; identical to SEQ ID NO: 104

SEQ ID NO: 129 - DNA, 951 bp, Zea mays; identical to SEQ ID NO: 105

SEQ ID NO: 130 - protein, 298 aa, Zea mays
MAVDLMGCYAPRRANDQLAIQEAAAAGLRNLELLVTSLSTQAAAPHRAADQPFGEIAGQAVSKFRKVISILDRTGHARFRRGPVEPPPPTPPPPPVVPGPAPLAAVSVAQPPQSLTLDFTKPNLAVSAATSVTSTSFFSSVTAGEGSVSKGRSLMSSGKPPLSGHKRKPCAGAHSEATTNGSRCHCSKRRKNRVKRTIRVPAISSKVADIPSDEYSWRKYGQKPIKGSPYPRGYYKCSTVRGCPARKHVERATDDPAMLVVTYEGEHRHTPGAVQGPSPLATASPVPVAVSAGNGLVV

SEQ ID NO: 131 - DNA, 897 bp, Zea mays
atggccgtggacctgatgggctgctacgccccgcgccgcgccaacgaccagctcgccatccaggaggcggcggcggccgggctccgcaacctggagctgctggtgacgtccctgtccacgcaggccgccgcgccgcacagagccgctgatcagccgttcggcgagatcgccggccaggccgtctccaagttccgcaaggtcatctccatcctcgaccgcacggggcacgcccgcttccgccgcgggcccgtcgagccgccgccgccgacgccgccgccgcctcctgtcgtccccggtcctgcccccctggcggccgtcagcgtggcgcagccgccgcagagcctgacgctggacttcacgaagccgaacctggccgtgtcggccgccacgtccgtcacctccacgtccttcttctcgtcggtcacggccggcgagggcagcgtctccaagggccggagcctcatgtcctccgggaagccgccgctgtccggccacaagcggaagccctgcgccggcgcccactccgaggccaccaccaacggcagccgttgccactgctccaagagaaggaagaaccgcgtgaagaggaccatcagagtgccggcgatcagctcgaaggtcgccgacatcccttcggacgagtactcgtggaggaagtacggccagaagcccatcaagggctccccttacccacggggctactacaagtgcagcactgtgcggggatgcccggcgaggaagcacgtggagcgggccaccgacgacccggccatgctggtggtgacgtacgagggcgagcaccgccacacgccgggcgcggtccaggggccgagccccctggcgaccgcgtcgccggtgcccgtcgccgtctccgccggcaacgggctcgttgtctag